European Patent Specification EP 3 922 722 B1, published June 28, 2023. Title: SELECTIVE ANTISENSE COMPOUNDS AND USES THEREOF. Applicant: Ionis Pharmaceuticals, Inc. The sequence listing filed with the application follows.

SEQUENCE LISTING (95 sequences)

SEQ ID NO: 1 - DNA, 202001 bp, Homo sapiens
gcccagcaggtgtcagcctcattttaccccgcccctattcaagatgaagttgttctggttccaacgcctctgacatattagctgcatcattttacatttcttttttttttttccttttaaatggggtcttgctctgtcacccaggctggagtgctgtggtatgatctcggctcactgcaatctccacctccgaggttccagcgattctcttgcctcagcctcccgagtagctgggactacaggcacccaccatcatactgggctaatttttgtgtttttagtagagatggggtttccccatgttgcccaggctgatctcaaactcctgggcttaagcaatacagccgcgttggcctcccaaagtgttgggattacaagcatgagctaccccacccagctcattttacatttccacttgttaaactgaaaactggcccgagaaagcttctgtactgccatccttgcgtccttgcagatgaatcgtaacctagcatagtaggtaggcagactgaaaacctaacttagcagtaggcttctgtaacaacagctgtgtctcagccagttcctgcagccagacttcaaccactcacaggccgcaaactgttcaaactgtgttcggagaaggcgaattcatctggctgttaacgtgcctcacttctgctttctgtggccactttcccttttctgtccataaatttgctttgaccacacagcatccctagagtctccctgaatctgctgtgattctgggacctgcaccatttgtgaattgttttttttttccttgatcagctaaactctgttcaattcaatttgttggaagtttttaacataccaatggtgcaccaaggttccaatttctccacttcctcataaataagtcattttaaatggcttttcagtattccaatatttggaagtattaatgtttctaccaattttctatttttggacattgaggttgtttcattttttttttctttttttgagacagagtctcgctccgtcacccaggctggagtgcagtggcctgatcccggcccactgcaacctccacctccctcctcagcctcctgagtagctgggattacaggtgcatgcaccaccacacccagctaatttttgtatttttagtagagatggggtttcaccatgttggtcaggctggtctcaaactcctgacctcaggtggtccacctgccttggcctcccaaaatgctgggattacaggcctgagccactgcgcctggcctcatcttcttgatattaatgttgctttaacatctttgtccctgtgttttttgtttttttttttgagacggagtctcattcattctgtcacccaggctggagttcagtggcgtgatctcagctcactgcaacctctgtctcctgggttccagtgattctcctgcgtcggtctcctgagtagctgtgttcctgggtctttcgatggttatttaatacttccctacagtaatgccctgtgcgtacatgctaagtgtgatgaaatggttggcacagttaaatcttttgaaagacattgccaagtcactcttcagaaaagtgataggaggtcatagcaattttaagaagtcctcatttctacatttccttactaatctcggttggtgtctcttcaatctttcctcacacttttcttgggtttttcctgaatcatgagtctactacatttacacattttaaagcatctttagaaacaggatctcattttgttgcccaggctagagtttggtggcatgattatagctcctcatactcctgggctcaagtgatccttccacctctgaaaccccaaaatttgagaaaggtctcatttaatttagaaagtttattttgccaaggttgagggtgcacacctgtgatgatatacgagttaaaaagaaattatttaggcagatactgagggtaagaaagtcctcggtaaggttttcttttcaatgaaaagcagcccccaagcattttcttttctaacaaagagcagcctgtaaaatcgagctgcagacatacacaagcaagctggaagcttgcacaggtgaatgctggcagctgtgccaataagaaaaggctacctggggccaggcagatccaacatggcggctccatcttccctttccttgtcaaccatgtgcacagtaaggagcaggcaacatagtgtcccccgagtagagaccaatttgcataataaaaggtgagggtagggtgggcagcttctttgcatgctatgtaaacattatgcctggtccaaccaatctttgggccctgtgtaaattagacaccacctcctcaagcctgtctataaaaccctgtccattctgccgcaggctggaagacccactggggcacccctctctctctataggagacagctattcatttttctctttctttcacctattaaagctccactcttaaccccactccgtgtgtatctatgttcttgatttccttggcatgaggcaatgaaccttgggtattaccccagaaccttgggtattatgccacttcagtgacacagcctcaggaaatcctgatgacatgttcccaagatggtcggggcacagcttggttttatacattttagggagacatgagacgtcaattcatatatgtaagaagtacattggttccgtccagaaaggcggggacaacttgaggcagggagagagcttctaggtcacaggtagacaaatggttgcattcttttgaatctccgataagcctttccaaaggaggcaatcagaatatgcgtctattgactgggcgcagtggctcatgcctgtaatgccagcactttgggaggcggaggtgggtggatcacctgaggtcaggagtttgagagcagcccggccaacatggtgaaaccctgtctctactaaaaatacaaaaaattagctgggcgtggtggcgggcgcctgtaatcccagctactcgggaggctgaggcaggagaatagcttgaacccagaaggaagaggttgcagtgagctgagatggtgccattgcactccagcctgggcaacaagagtgaaactccatctcagaaaaaaaaaaaaaaggcctgggcaaagtggctcacgcctgtaatcccagcactttgggaagccgaggcgggcaggtcacaaagtcaggagattgagaccatcctggctaacatgatgaaaccccatctctactaaaaaatacaaaaaactagctgggtgtggtggcgagcacctgtagtcccagctactcggcaggctgaggcaggagaatggcgtgaaccggggaggcggagcttgcagtgagccgagatcacaccactgcactccagcccggacgacagggcaagactctatctcaaattaaaaaaaaaaaaaaaaaaaaaaaaaaagagagagagaatatgcatctatctcagtgagcagaaggatgactttgaatggaatgggagcagttcctagcttgaacttcccctttagcttcagtgatttgggggctcaaggtatgttcctttcacatacctcagcctcccaagtagctgggaccacaagtgcatgccaccacacgtggctaatgttttattttttttgtaggaatagggtctcactatgtgtccaggctggtctaaaacccctgagctcaaatggtcctcccgcctcagcctcccgaaatgctgggattacaggcatgagccagcatgcccggcctagtctacatttttataaattgctaattcaaagttccctctccaaaacctcatggttttccctgttctcatcccctgcaccctcccttcccctggagtactcacctggccttggaggtctggtgtgagcccggacttcgattctaggcacagcatgtgatgagcgcccccaggtcaaacacctcccctctgcggcctgtgcttcaccgccttgacagtgagaaaggtctcccttcggctcattctcgaagtctcaaacttcacttctcctgtgcgctgattctgaattcagcccccgtccaaggtcctggcccctttctcttctgcttggcgtgttgttcatcaccactgtgcactgctgagggtaagtgcggttctctggacctctgctttatcattagaacagactcttgcggtttcccacgacattcctttcacttctcacttggaagatgagccgtgaggaaatcctgtgttgtgtggtatgtgggctgtgcttctgcttgacttgagggccaagcagcattgcaagccatggttttaaataagaaagaacatttctaaccttcatcttctagtaaggaaacaagtgggctttagagttcttgctcaggaaagacctatgtcccagtccaaccggaccttttactaaagagatcttcctgatcctcctccccaggccaggggaggggtcctccctggggttggagcctttagtagggggtcggagacacgacgtagccttcatgacattcatagtctagttacacgatccctgtaagggtcagttgaagtaagtgctacaaaggaagggaggtgctcagtggagagggctctcttttatgtattatatttctttcatggggagggatatggatcagggatcagcagaggtgtttcagtcccgagggaaagaaagtcagcgtggcttgggagttgggagcagcaagacagtggctcaagatatcttaagactagtggagtacaccttgcatgttaaaagccttgctcagggctgcctggttcttgtaggacgacagagatggcctagctctgcatactgcacccccaggggctcagaacagtgcaaatgtcagtctatctgtcagtggcagagccagccttggagcaggggtgcaaggaggtctctgcactggccaggcatgcagaacattctgttcagtagcactggacagaaggccccatctagatgagacagagctggtggggcaggacaaagactcctggcagctcaaacggcctggcagatgcttggagagagggggcttcttgagacagcaccatttctgggaagagagtcacctgggagggatgaggccacgctccggcttggaggtgaagagaggggctgctgcaagaaagaattagagacatgccagcctttgctgtgttgcccaggctggtcatgaactcttggcctcaagcaatcttcccacctcagcctccccaagcgctgggattatagacatgagcccccatgctggccaataaaagatgattttatggaggggatggtggtgaaggttgtgggtggtatgaaatagtaagaaatatatattggtctgcacccagttcctgccacagagctcctaaaatcctgagaacttcctgggtgagcatcttttgttctaatgaggtgactcttggtggctcctggataggagtgaatcaccagaaagatcaagccagagttagaagcagaaagtgctggctataacacaggaaagctgtaacacaaataataaagtttttttttttttttttgagatggagcctcactctgttgcccaggctggagtgcaatggtgcaatctcagctcactacaagctctgcctcccaggttcaagtgattctcctgcctcagcctcctgagcagttgggactacaggtgtgtgccaccacatctggctaatttttgtatttttagcagagacggggtttcaccatattaaccaggctggcctcaaactccttaccttgtgatccgcctgcctcagcctcccaaagtgctgggattacaggcatgagccaccgtgcctggccaaaagacattgttcttaaaagaatcaactaactaaccaaataaataaaaatctaacctaattaagaaactaaaaatacacaaaaattaatttcaaggggagaaaaatcatgtaaagagagaaagataatgaatactttgcagaaatttatgaacataaacataaaacttggatgaaatgcatttctaggaaaacataatttatcaaaactaaccacaagtaaaatagaagcctaaataggatattttcaagagaagaagtaaagttgtcaaagtgctacccttcaaaaaaacaccaggctcaaacaatctgacatgggaatgttagcacaccttagagagcaaataaaactttgaatgggcttgaaatattccagactctagaaaaacaaaacttcccaattctttttataaagcaagtataaattgataccaaaatcttataaagaccttatacaaaacttcataccaatctcttttatgaatacaaaacccttaataaagtattaccagacagaacccaacaatacataaaaatgtcacatcataacatagtggggtttatttcaataatgcatggatggttcaatacaaggaaattcagtaacacaatataatagatcatgtgaatatacccaaagaaaaaatagattattttcatagatgctgtaaaggcatttgaccaaattcaacacctactttttaggtggtcaataaaataaattagttactccttctttagcatgataaaatatatttatcagcccagaaggcatcattttacccgataagggcacacgctggagggaataatgttaaaattaggaataagaggatagctagtttctttcttcttttttttttttgagacggagtcttgctctgttgccaggctggagtgcagtggtgcaatgttggctcactgcacgccccccgcctcccaggttcaagcgattctcctgcctcagcctcccgagtagctgggactacaggcgcgcaccaccatgcccggctaatttttttttgtattttagtagagatggggtttcaccatgttggtcaggctggtcttgaactcccaacctcacgtactgggattaccggtgtgagccaccacgccagcccaactactttcaacattatccttaatactgatgcttattgacttactatggggttacctctagataaatccataataagttgaaaatataagtaaaaaatgcccttaatacacctaacctaccaaacatcatagctgagcccagcctgccttagctatgctcagacactgacgtcagcctacaattggcaaaatcacacagcagcacagtctactgcagagcatctgctgtttgcccttgtgactgcgtggctgcctgggagcttcccagcttcacaagacagtattacgtagcacatcactagcctggggaaagatcaaagttgaaaatttgaagtgtggtttccattgaatgtgtactgcttttgcaccatcatcaagtcaaaaaattttagttgaaccagcctaagtttgggaccatctttattttcaggaggaacttccatgtacattgatgacggacgatagaatccgtttctatcatcctaatgaacataatgaataaatccagacaaacataaacattaacagagtaagcagctttcggggctggaagccagaagagggtgggagcgcagagagagaggccaaacaccagggctgcttctgctttgcgggtatttgctgatctggacaaggtatctggaaggctgagctaagcctcctttttttttgaggtggcgtctcactctgttgccaggctggagtgcaatggtgcgatctcagctcactgcaacctccacctccctggttcaagcgattctcctgcctcagcctcccgagtagctgggattacaggctcccgccactacacccagctgatttttgtaattttagtagagacggggtttcaccatgttggccaggatggtctcgatctcttgacgtcatgatctgtccacctcggcctcccaaagtgctgggattataggcgtgacccaccgtgccccgtctgagctaagcctcttgagcataggggactaaaaatgaaatctagcgcatgccaagtttagggtcccaggcaattcctttccactttggggtccactttggggtccaccccacccaagaagaaggatgacttggaagtaaaccagctctgaaatatggatggtcctctgggaccataccaatcccttcatatcaaccacatccagttcctcaaaactggaacttggattaagatggcctaggacttctagtgtcccaggagcctggcattgcaaacaaaaatcctctccggaagaagataataccttaagcttcaaatgactctctaataaatttcaaatacaatgtccagcacacaaacacaaattaccaggaacgtgatatgaggcctgatggatgggaattagcagaaacttcaggcatgagaaacataccctcagaggcctagaatctatctagtgtctagataatggagatatgaaatacagacacttaaacaactatgtttcccatgttcaaagaggaaatttgcaaaacttgaaagtgttggcaggaaatcagaaactataaaatgtgacaacagcatactttagagtcagtataaattacggtcccgaaaactgcagaattccagaacttaatggtaaagcaagggtttaacagcagaatagaaatagccagagagaactaggaagtaagtcagatgacactacccagaataaggcactgagaggccaaggaatggaaaatgcagaagaaaggatatggtgagaggatctaatatacatttatttggagtaccagggagagagagaaggagaagaacagaagccgtgtttcaaggacggtgactgagaggcttcgaaactgatgaaagccatcagttcacaaattcaaagcccagtgaattccaaggagaaaaaaagaaatccatactgtgaaagcaagtccagacaatgacaaacaccatcaacaatacacaggacaggcataagatgcatttaatggggacactcagaggcagagggttatcagaaggaggcacttctctcccaagttctcatcatcccagggccagggacagctggtcacaccttagggagttcactaggagagggatctggcttcttgtcattctgggtatttgtagggaaattggaagggaaccgagagcacctagccaatcgcatagcaatgggagatttcaggctgtggggaatgtctttgctggtgaaaagaacatcctgaccttagaaatctttcaccgagggggatctgcgttccagaacttctggagctggtataggtaaggctttgagctttcctactgagccagcctgttgctaggttaccaaaggggacctcgagggccatctggccaacaagcagacttgtctctccttacacccccagacgtatcactgcaaaactacagaaaaccaaagacagagaaaatcttaaaagcagccagatttaaaaaatggcatattagtttcaaagcagcagccatgaaattgacagctgatgtctcaacagcaagaatgaaaagtggaagacaggccaggtgtggtggctcaggcctgtaatcccagcactttgggaggccgaggcgggtggatcacgaggtcaggagaccaagaccatcctggctaacatggtgaaaccccgtctctactaaaaatacaaaaaaattagtcgggcatggtggtgggtgcctgtagtcccagctactcgggaggctgaggcaggagaatggcgtgaacccgggaggcggagcttgcagtgagccgagattgtgccactgcactccagcctgggtgacagagcaagactctgtctcaaaaaaaaaaaaaaaaaaaaaaaaaaaagggtgacgaagcttcaatctcctgaaaggaagcaactgccgcctttgattcgatacccaccaaaatccgtgaagaaggaaggcaaaataaaaacacttcctgattgaactggaaagatttccgcaatagaagacccactgtccaaggaattctaaaggatgctttccaggcagaagaaaatgaccccagaggaagatcagagattcaggaaagaaatggagagtgataaaaatggaaaattcgggggccaatttaaacaaaagctgactgctctacaactgttgtgtctctatcttttgtaacatatatgtgtgtgtagcttttttttttttttttgtcaagatggattctcactctgtcgcccaggctacagtgaaatggcacggtctcggctcactgcaacctctgccccttgggctcaaatgattctcttgcctcagcctcctgagtagctgagattacaggtgcctggcacaatgcctggctaatttttgtatttttactagagatgggatttctccatgttggccaggctggtcttgaacacctgacctcaggtgatccacctgcctgggcctcccaaagtgctaggattacaggcgcgagccactgcatctggcctatgtgtgtgtttatatggaattaaaacacatggcaataataccctccaaattgggagaaaccaaaaatagcatttaaatgttgtaagctccctgcataatcaagaagagaatagatttacgttagattttgatacctggaggatgaatgttgtaatttctagggtgaccatgaaaagaggagacaacggtgtatgtttttttttttttgagatggagtctcactttgtcacccaggctggagtgttgtggtgtgatcttggctcactgcaacctcctcctcttgggttcaggccatcctcccacctaggcctccagagtaggtgggatcacaggcacctgccaccacacctggctaatttttttttttttttaaatatttagtagagatggggtttcaccatgttggccaggctggtcttgaactcctgacctcaggcgatctgcctacctctgcctctcaaagtgctgggattacaggtgtgagccatcgcgcccggccaacagtgatcactttcaaactaacagaggttcaaaaataaaatcagacttaaccaaaaaccaggtaacagagctggtaggatatacagaaagactgacctcacgtatatcaacgattacagttaatattaatgaaggaaatgctctagtttaaaaacgagggttgtcaaagaccccacataagaagctccttaccagcggtgcacctagaacctaaggaaacaggacagatgaaggaggacgcgcccccgccgctgtcctgcgcctcagccatcctatgagacgggaaaggtttctgtctgcagctgggcccgtgctctttaccagctcctggctttcttctctggaaggttcctgcctgttttgccctcacacctgctcctctctcagccctctcaggggtggggctggaggccaccaaagagcctcctctgctctccagttgctcgactgctcctcatttccccctggggtctgcgtcagggtttccttcttttccagccccaccccgcgtgcatcccacctggtctcgggtcggggctgctcccgcttactgccccctgcccaggctggtgtgcaccccctctggctgctttcaaggcctcttctctcttctcggcaggacaggcacaggcaggtggccaggtgtcatgcttagctccccgcccagtgagattctttcatttaacaatcttcccctgaatagttcatgttcattgctgaaaatttgaaaaatatggaaaagcacaaagattaagatataaaccgccctcaattcccctgcccagagagagtcactgctatgacttggtgactaggaaccttatttctctctcgctcttttttttttttttgagacagagtcttgctctgtcacccaggctggagtgcagtggctcgatctcagctcactgcaacctccgcctcctgggttcaagcgattctcctgcctcagcctcttgagtagctgggattacaggcacctgccaccatgcccggctaatttttgtatttttagttgagagagggtttcatcttgttggtcaggcggacttgaactcctgacctcaggtgatcagcccacctcggcctcccaaagtgctgggattacaggtgtgagccactgcgccttcatctctcttctgtgtatgtgtacgctgttttttctttagaatgggggacgttatcaggctctacatggtgtgtagtcggctagcatgttgtaagcctttccctgtgtcacaagtgctcatctggaacaggattctaatgactgcctgtggctatgttgggattcctttaactcagctccttctgcccagcatctatcttttttccatcttttgtcctaagtgttgctataataaatcattgatcacacatgcctgactgtttgcataggataaattacgggaaatgtttttgctgttcagggactgtgcccatttttaggcctcagagacaccatgccagactgcccagtattgatctttactctttttagatgatgccaaacttttctgtgaactttaaaaacctgtgtcttgacagtccatttctgtaagtctttcacattagatttcctgtcaggatgatagtcaattctaggcagatgatgttttctcagccatggctgaagcagttgtgatttgttgtggccatgtaaagtcccgatgatccattgcctccctggatgggttggaataatttggtttgggagcatataacagaatgacctggagtcacagcagctcagacggaagtgtatttctcccttacagatgaaagaattccaggccaggctggaatgacaactgcacacagtcatctgggccccctccttccagctcccatcaccccaggatgtggcttttatgcagatgatccaaaatggctgctcaagtcccagccaacacatcccattccagggagcaggaaaaaggtgtgtctttcccttcattttatgtgattcctttctagaagtactactcattacttctgcttgcatctccctggctagcacttacttagttatatggccatagctagctgaaggaaggacagggactgtcatacactagctaagaggcaaactgcttagataaaaaggtctctaaagaaggtcagagcggctgctagggtgcaactctattacttattgttatgggacgaactgtgtccctcattcaggttgatgtcctaagccccagaacctcagaatgggattgtatttggagacaggttctttaaggaggtaaggaggctaaaatgagatcattagggtgggccataatccgactgatgtcttacaagaagagattaggacacggacatgctcagagggacggccacgtgaggacaccaagaaaggcagctgtctgcaagtcaaggacagggctcaggggaaaccaaccttgccaacaccttcatctcggacttctagcctctaggaccatgagaagatacatttctgttgtttaagctgcccggtctgtggtactttgttatggcagcccaagtaaacaaatacagtcatctgctgctggaacaaatcaccccagcactgtggcttggcagcacacatgtctagtcatagagttatatgtagttacgtgtagagccatatgtatcgtcacacgttctgtgggtcaggaatttggacccagcttaaccagctccacttctcgccagggttcagtcaaataccagctgcctcccacctgagagctcagccggggaagggtccctttccaatctcacgtggtgttggcaggatccagttcctcatggcctgctggactgagaacctcagttctcactgcctgttggccagaggccgcctttatgtcctcgccatgtgggcctctccaacatggcagctgacttcatcagagcatccatgccaagaaggcaacagagagggccagggagactgaagtcatacccttttgcgacctagtcatggggtgacattccatcacctttgcccattggttagaagcaggccaccaggtacagcccaagctcacggggaggggtcatacaagggtgtcaataccaggaggtgaggggtgctggggccatcttatgagtctgcccactgaggtaactaacaaccttgaggcctgacacagtggacaaaggcccttattaacagcagagaactgggaactttatttatttatttatttttgagacagagtctcactcttgtcacccaggctggagtgcaatggcatgatcttggctcactgcaacctccacctcccaggttcaagcaattctgcctcagcctccggaatagctgggactacaggcatgcaccactacacccggctaatttttgtatttttagtagagacagggtttcgccatgttggccaggctggtctcgaactcctgacctctggtgatctgcctgccttggcctcccaaagtgctgggattacaggcgtgagccaccgcacctcgctggaacttaatttttttagagacagtgtcgctctatcacccaagctggagtgcagtggtgcaatcctagctcacttgcagcctcaaattcctgggttcaggtgatcctcccacatcagcctcccaagaactgggaactaacagctgtttctctgctgtccttctcaagaaaagggaggctactgctaccccactggggacaatgctgggtttccctttaggacaggctctgagacaaggcggaggtgctgtttgtggccacagagcaggggactctgggttgcaggtgtggcctggctaaagtaggctttactgggctcctctctgcctgcatcaccccccggctgggcggttgtctctgaggccaaccttactccctgctgggcaggctggacagctgccctctccgtttgcccctctaccacccaaaaggcaggaggctctggagaccaggaccctgcccgccacggcctgtgtcccaggcgtgagggggtgccccacagacctctgctgagctgctgctgaatgacgccccttgggggtcctgccggaaggtcagagcaggggtgcactcccataaagaaacgcccccaggtcgggactcattcctgtgggcggcatcttgtggccatagctgcttctcgctgcactaatcacagtgcctctgtgggcagcaggcgctgaccacccaggcctgccccagaccctctcctcccttccggggcgctgcgctgggaccgatggggggcgccaggcctgtggacaccgccctgcaggggcctctccagctcactgggggtggggtgggggtcacacttggggtcctcaggtcgtgccgaccacgcgcattctctgcgctctgcgcaggagctcgcccaccctctccccgtgcagagagccccgcagctggctccccgcagggctgtccgggtgagtatggctctggccacgggccagtgtggcgggagggcaaaccccaaggccacctcggctcagagtccacggccggctgtcgccccgctccaggcgtcggcgggggatcctttccgcatgggcctgcgcccgcgctcggcgccccctccacggccccgccccgtccatggccccgtccttcatgggcgagcccctccatggccctgcccctccgcgccccacccctccctcgccccacctctcaccttcctgccccgcccccagcctccccacccctcaccggccagtcccctcccctatcccgctccgcccctcagccgccccgcccctcagccggcctgcctaatgtccccgtccccagcatcgccccgccccgcccccgtctcgccccgcccctcaggcggcctccctgctgtgccccgccccggcctcgccacgcccctacctcaccacgccccccgcatcgccacgccccccgcatcgccacgcctcccttaccatgcagtcccgccccgtcccttcctcgtcccgcctcgccgcgacacttcacacacagcttcgcctcaccccattacagtctcaccacgccccgtcccctctccgttgagccccgcgccttcgcccgggtggggcgctgcgctgtcagcggccttgctgtgtgaggcagaacctgcgggggcaggggcgggctggttccctggccagccattggcagagtccgcaggctagggctgtcaatcatgctggccggcgtggccccgcctccgccggcgcggccccgcctccgccggcgcagcgtctgggacgcaaggcgccgtgggggctgccgggacgggtccaagatggacggccgctcaggttctgcttttacctgcggcccagagccccattcattgccccggtgctgagcggcgccgcgagtcggcccgaggcctccggggactgccgtgccgggcgggagaccgccatggcgaccctggaaaagctgatgaaggccttcgagtccctcaagtccttccagcagcagcagcagcagcagcagcagcagcagcagcagcagcagcagcagcagcagcaacagccgccaccgccgccgccgccgccgccgcctcctcagcttcctcagccgccgccgcaggcacagccgctgctgcctcagccgcagccgcccccgccgccgcccccgccgccacccggcccggctgtggctgaggagccgctgcaccgaccgtgagtttgggcccgctgcagctccctgtcccggcgggtcccaggctacggcggggatggcggtaaccctgcagcctgcgggccggcgacacgaacccccggccccgcagagacagagtgacccagcaacccagagcccatgagggacacccgccccctcctggggcgaggccttcccccacttcagccccgctccctcacttgggtcttcccttgtcctctcgcgaggggaggcagagccttgttggggcctgtcctgaattcaccgaggggagtcacggcctcagccctctcgcccttcgcaggatgcgaagagttggggcgagaacttgtttctttttatttgcgagaaaccagggcgggggttcttttaactgcgttgtgaagagaacttggaggagccgagatttgctcagtgccacttccctcttctagtctgagagggaagagggctgggggcgcgggacacttcgagaggaggcggggtttggagctggagagatgtgggggcagtggatgacataatgcttttaggacgcctcggcgggagtggcggggcagggggggggcggggagtgagggcgcgtccaatgggagatttcttttcctagtggcacttaaaacagcctgagatttgaggctcttcctacattgtcaggacatttcatttagttcatgatcacggtggtagtaacacgattttaagcaccacctaagagatctgctcatctaagcctaagttggtctgcaggcgtttgaatgagttgtggttgccaagtaaagtggtgaacttacgtggtgattaatgaaattatcttaaatattaggaagagttgattgaagttttttgcctatgtgtgttgggaataaaaccaacacgttgctgatggggaggttaattgccgagggatgaatgaggtgtacattttaccagtattccagtcaggcttgccagaatacggggggtccgcagactccgtgggcatctcagatgtgccagtgaaagggtttctgtttgcttcattgctgacagcttgttactttttggaagctaggggtttctgttgcttgttcttggggagaatttttgaaacaggaaaagagagaccattaaaacatctagcggaaccccaggactttccctggaagtctgtgtgtcgagtgtacagtaggagttaggaagtactctggtgcagttcaggcctttctcttacctctcagtattctatttccgatctggatgtgtcccagatggcatttggtaagaatatctctgttaagactgattaatttttagtaatatttcttgttctttgtttctgttatgatccttgtctcgtcttcaaagtttaattagaaaatgattcggagagcagtgttagcttatttgttggaataaaatttaggaataaattattctaaaggatggaaaaactttttggatatttggagaaattttaaaacaatttggcttatctcttcagtaagtaatttctcatccagaaatttactgtagtgcttttctaggaggtaggtgtcataaaagttcacacattgcatgtatcttgtgtaaacactaaacagggctcctgatgggaaggaagacctttctgctgggctgcttcagacacttgatcattctaaaaatatgccttctctttcttatgctgatttgacagaacctgcatttgcttatcttcaaaatatgggtatcaagaaatttcctttgctgccttgacaaaggagatagattttgtttcattactttaaggtaatatatgattaccttatttaaaaaatttaatcaggactggcaaggtggcttacacctttaatccgagcactttgggaggcctaggtggacgaatcacctgaggtcaggagtttgagaccagcctggctaacatggtgaaaccctgtctctactaaaaatacaaaaattagctggtcatggtggcacgtgcctgtaatccaagctacctgggaggctgaggcaggaaaatcgcttgaacccgggaggcagagtctgcagtgagttgagatcacgccactgcactccagcctgggtgacagagcgagactctatctcaaaaaaaattttttttaatgtattatttttgcataagtaatacattgacatgatacaaattctgtaattacaaaagggcaataattaaaatatcttccttccacccctttcctctgagtacctaactttgtccccaagaacaagcactatttcagttcctcatgtatcctgccagatataacctgttcatattgtaagatagatttaaaatgctctaaaaacaaaagtagtttagaataatatatatctatatattttttgagatgtagtctcacattgtcacccaggctggagtgcagtgatacaatctcggctcactgcagtctctgcctcccaggttcaaatgcttctcctgcctcagccttctgagtagctgggattacaggcgcccaccaccatgtccagctaatttttgtatttttagtagagatggggtttcaccatgttggccaggctggtcttgaactcctgaccttgtgatctgtccacctcggcctcccaaagtgctgggattacaggtgtgagccaccatgcctggctagaataataacttttaaaggttcttagcatgctctgaaatcaactgcattaggtttatttatagttttatagttattttaaataaaatgcatatttgtcatatttctctgtattttgctgttgagaaaggaggtattcactaattttgagtaacaaacactgctcacaaagtttggattttggcagttctgttcacgtgcttcagccaaaaaatcctcttctcaaagtaagattgatgaaagcaatttagaaagtatctgttctgtttttatggctcttgctctttggtgtggaactgtggtgtcacgccatgcatgggcctcagtttatgagtgtttgtgctctgctcagcatacaggatgcaggagttccttatggggctggctgcaggctcagcaaatctagcatgcttgggagggtcctcacagtaattaggaggcaattaatacttgcttctggcagtttcttattctccttcagattcctatctggtgtttccctgactttattcattcatcagtaaatatttactaaacatgtactatgtgcctggcactgttataggtgcagggctcagcagtgagcagacaaagctctgccctcgtgaagctttcattctaatgaaggacatagacagtaagcaagatagataagtaaaatatacagtacgttaatacgtggaggaacttcaaagcagggaaggggatagggaaatgtcagggttaatcgagtgttaacttatttttatttttaaaaaaattgttaagggctttccagcaaaacccagaaagcctgctagacaaattccaaaagagctgtagcactaagtgttgacatttttattttattttgttttgttttgttttttttgagacagttcttgctctatcagccaggctggagtgcactagtgtgatcttggctcactgcaacctctgcctcttgggttcaagtgattctcatgcctcagcctcctgtttagctgggattatagacatgcactgccatgcctgggtaattttttttttttcccccgagacggagtcttgctctgtcgcccaggctggagtgcagtggcgcgatctcagctcactgcaagctccgcttcccgagttcacgccattctcctgcctcagtctcccaagtagctgggactacaggcgcctgccaccacgtccagctaatttttttgtatttttaatagagacggggtttcaccgtgttagccaggatgatcttgatctcctgacctcgtcatccgccgaccttgtgatccgcccacctcggcctcccaaagtgctgggattacaggcatgagccactgtgcccggccacgcctgggtaatttttgtatttttagtagagatggggttttgccatgatgagcaggctggtctcgaactcccggcctcatgtgatctgcctgccttggcctcccaaagtgctaggattacaggcatgagccaccatacctggccagtgttgatattttaaatacggtgttcagggaaggtccactgagaagacagctttttttttttttttttttggggttggggggcaaggtcttgctctttaacccaggctggaatgcagtatcactatcgtagctcacttcagccttgaactcctgggctcaagtgatcctcccacctcaacctcacaatgtgttgggactataggtgtgagccatcacacctggccagatgatggcttttgagtaaagacctcaagcgagttaagagtctagtgtaagggtgtatgaagtagtggtattccagatggggggaacaggtccaaaatcttcctgtttcaggaatagcaaggatgtcattttagttgggtgaattgagtgagggggacatttgtagtaagaagtaaggtccaagaggtcaagggagtgccatatcagaccaatactacttgccttgtagatggaataaagatattggcatttatgtgagtgagatgggatgtcactggaggattagagcagaggagtagcatgatctgaatttcaatcttaagtgaactctggctgacaacagagtgaaggggaacaccggcaaaagcagaaaccagttaggaagccactgcagtgctcagataagcatggtgggttctgtcagggtaccggctgtcggctgtgggcagtgtgaggaatgactgactggattttgaatgcggaaccaactgcacttgttgaactctgctaagtataacaatttagcagtagcttgcgttatcaggtttgtattcagctgcaagtaacagaaaatcctgctgcaatagcttaaactggtaacaagcaagagcttatcagaagacaaaaataagtctggggaaattcaacaataagttaaggaacccaggctctttcttttttttttttttgaaacggagtttcgctcttgtcacccgggctggagtgcaatgatgtgatctcagctcactaaaacctctacctcctgggttcaagtgattcttctgcctcagcctcccaagtaactgggattacaggcgtataccaccatgcccagctaatttttgtgtttttagtagagatggggtttcaccatgttggccaggctggtctcgaacttctgacctcaggtgatccactcgcctcagcctgccaaagtgctgggattacaggtttgggccactgcacccggtcagaacccaggctctttcttatacttaccttgcaaacccttgttctcattttttccctttgtatttttattgttgaattgtaatagttctttatatattctggatactggattcttatcagatagatgatttgtaaaaactctcccttcctttggattgtctttttactttcttgatagtgtcttttgaagtgtaaaagtttttaattttgatgaagtcgagtttatctattttgtctttggttgctgtgcttcaagtgtcatatctaagaaatcattgtctaatccaaagtcaaaaaggtttactcctatgttttcttctaagaattttagagttttacatttaagtctgatccattttgagttaatttttatatatggttcaggtagaagtccaactttattcttttccatgtggttattcagttgtcccagcactgtttgttgaagagactattctttccccatggaattatcttagtacccttgttgaaaattaatcgtccttaattgtataaatttatttctagactgtcagttctacctgttggtctttatgtcgatcctgtgccagtaccatacagtcttgattactgaagtttgtgtcacagtttaaattcatgaaatgtgagttctccaactttgttccttttcaagattgatttggccatgctgggtcccttgcatttccgtacgaattgtaggatcagcttgtcagtttcaacaaagaagccaagtaggattctgagagggattgtgttgaatctgtagatcaacttggggagtattcgcatcttaacaatattgtcttccacctatgaacatgggcaaactttgtgtaaatggtcagattgtaagtatttcgggctgtgtgggcacagtgtctctgtcacagctacgcggctctgccattgtagcatgaaagtagccataagcaatatgtatgagtgtctgtgttccaatagaattttattaatgacaaggaagtttgaatttcatataattttcacctgtcatgagatagtatttgattattttggtcaaccatttaaaaatgtaaaaacatttcttagcttgtgaactagccaaaaatatgcaggttatagttttcccactcctaggttaaaatatgataggaccacatttggaaagcatttctttttttttttttttttttttttttgagacggagtttcactcttgttgcccaggctggagtgcagtggcgcgatctcggctcactgcaacctctgcctcccaggttcaagacattctcctgcacggcctccctagtagctgggattacaggcatgcgccaccacacccagctaattttgtatttttagtagagacggggtttctccatgttggtcaggctggtcttgaactcctgacctcaggtgatccacccgcctcagcctcccaaagtgctgggattacagggtgtgagccaccacaccctgctggaaagcatttcttttttggctgtttttgttttttttttaaactagttttgaaaattataaaagttacacatatacattataaaaatatcttcaagcagcacagatgaaaaacaaagcccttcttgcaagtctgtcatctttgtctaacttcctaagaacaaaagtgtttcttgtgtcttcttcccagattttaatatgcatatacaagcatttaaatgtgtcattttttgtttgcttgactgagatcacattacatatgtatttttttacttaacaatgtgtcatagatattgttccatagcagtacctgtaattcttattaattgctatgtaatattttagaatttctttttaaaagaggacttttggagatgtaaaggcaaaggtctcacatttttgtggctgtagaatgtgctggtgacatattctctctaccttgagaagtccccatccccatcacctccatttcctgtaaataagtcaaccacttgataaactacctttgaatggatccacactcaaaacatttagtcttattcagacaacaaggaggaaaaataaaataccttataaagcactgtttaatattgtattaaattggatcaatttgggggctagaatgtatgttagagacatgatatgtccataggtccttgctatcacagtgaggtctcagggacagtcgtttggtatcatttgggatctcataagcagactctctctgcttgacctgacaaatcagagtctgtgttttaacaggttcagtgagtgacttacatgcacattggagtttgggaagctccactgtaggtgcttagaccttacctttgttgttgctaataacaatgcaagcatttgggaggaagacctgtgttgctcatatgtgtccaggtgtagctgaggtggccttgcttatctgctgtagggccgttgagcatttctgtagctgtgatgagtgagctgaggtgagcctgcggagagctcccagccattggtagtgggactcgcttagatgaactggaaggaccctttcatctgagcagccactatggagaaaaacaaccgaatgaggggagagacaatgtgcaattttatttagggcacaaaggagagctgtggttagaaggtgacatttgagtggaaagggggcaagccatgtgtatagcgggagaagagaggtccaggcagagttaacagaaggcagaaatgctttccatgtttgagaaccagtaaggaggccagtggctgaagtaaggtgaagggcagaaataaggatgaggctgcgagagatgagaggttagagacgagcgtcttgtgcaccaagataagcttgtgtggtcaaaacaagtagtttaatttatgtttttaaaagatcattttggctgggcacaatggttcatgcctgtaataccagtagtttgagacggtgtggtgggaggattgcctgaggccagacgaccagcatagccaacatagcagcacctataaggtctctacaaaaaactttaaaaaattagctgggcatagtggtgtgtgcctgtagtcccagctactcaggaggctgaggaggctggaggattgcttgagtccaggagtttgaggctgcagtgagctatgattatgccactacactacaacctgggcaagagagtgagaccctgtctctaaatatacacacacacacacacacacacacacacacacacacacacacacacacacacacacatatatatgtatatatatgcatttagatgaaaagatcactttgacaataccacatgctggtgaggatttagaaaaactaggtcacttattgctggtgggaatataatatagtacggccactctggaaaacagtttggcagtttgtcataaaactgaacataccgttagtatacagcccagcagcaactacaatcctgggcattaatcctagagaaatgaaaccttaatgttcacataaaaacctatactcaagtatgcatagcagctttacccataatatctaagaactggaatcagctcagatgtccttcaacaggtgaatggttaaactactcagtaataaaaaggaatgagctactgatagcatgcaacagtttaggtgaagttatgctaatgaaaaaagccaatcccaaaaggttatacatactgtatgattctatgtttttttgcaatggcacagttttagggatggagaatagattagtggttgcctggggttagagatggggtagtagagtaggttagtggtggcagaggagagaaaagagagggaggtgaatgtggttataaaaggacaacacaggggaatacttgtaatggaaatgctttgtctttttttttttttttttttttttggcgacagagtcttgctctgttgcccaggctggagtgcagtggcatgatcttttctcactgcaacctctgcctcctgggttcaagtgatacttgtgtctcagtctcccatgttcagagtgaaacaaaccagaggtaatgttcatccaaataatccaacacacatgacattaaaacatcaagatcaggtcggacgtggtggctcatgcctgtaatcccagcacttttgggaggccaaggtgggcagatcacttgaggtcaggagttcgagaccagccgggccaacatgatgaaaccccatcttgactaaaaatacaaaaattagccgggcatggtggtgtgcacctgtagtcccagctacttgggaggctgaggcaagagaactgcttgaacccgaggggcagaggttgcagtgagctgagagtgcgccattgcacttcagcctgtgtgacagagtaagactccatctccaaaaaaaaaaaaccaagatcaattaaaatacagcattactgggccgggtgtggtggctcacacctgtaatcccagcactttgggaggccgagatgggcagatcacgaggtcaggagatccagaccatcccggctaacacggtgaaaccccgtctctactaaaaaatacaaaaaattagccgggtatagtggtgggtgcctgtagtcccagctacttgggaggctgaagcaggagaatggtgtgaacccgggaggcagagctggcagtgagctgagatcgcgccactgcactccagcctgggcgacagagcaagactccgtctcgggggaaaaaaaaaaataaataaatagaatgctgtagtgtccttgagtttacatgcccctccttacgcttgtgtgcccgtgcagattgcttgattacacaattagaggaggctggcggaggattgttttaatttttttttttttgagacagtctggctctgttccccaggctagagtgcaatggcgcaatcttggtgcactgcaacctctgcctcctgggttcaagcagttcttctgccgcagcctcccgagtagctgggattataggcgcccgccaccacgcccaactattttttgtatttttagtagagcagcgtttcaccatgctggccaggctggtctcgaactcctgacctcagatgatctgctgccccagcctcccaaagtgctgggattacaggcgtgagccacacctggccgtttgttttaattttgaaggtgaagtgaaagtgactacatttaccaaaagtgattgaaaagccaggactgttcttaccctgtttttccagttcttgctcagagcaaggtggtttctttttcacttaatcaccatacttacttttcatgtagaacaagtcagtttgagttatcagttcatcatcttaactaaattccatgggggaaggaattagttttagtttcttaaacttccaggtttgcttattggacaaaatgagatagcaaggcagtgtttttaagttagattttttatttctttggtaatacaattttctcagaaacttagtagtcttttagtttagttgtttttagttggtcctatgttttggatcacccctctctactttattttgatagtgccaactgtgaagacatctgaagccataggtttggatgggaaggaggcatctttagcctgatcatcttcgccaggctgtttatctccttttgcttggctgagaagtcttaataggaggcttattcccagctatttggggacatagaagcagttagccattgcttatattttactgaggtctgtgtggtatgttgattgtagtcagttaacgattttgagaactgaaggcagcctggtatatatagagtaggtattagactgtgtttcttctaattgaatttcccatctcttgtaatctatgccatcatcttctgtactgctgagaaagaaagaaagtttctaatcaaactataccactggttgtaagatgcagtttggctttagtgatgttaacacatgattcaaacgtgaaattgattgagtattggtgaaatacagaggagatttaaagccagaagacctgggtttaaatgctggctgtatgacttcatatctgtgtgatcttgggcatgtcatggttggcacttcaatttcttctctctataatgggggaagtgaggccagtcatggtggctcatacctataatcccagtgctttgggaggccaagatgggaagatcgcttgaggccaggagtttgagcaattgggcaacatcgtgaggccccgtctctacaaaatattttgaaaaaattagccaggcccagtggtgcgtgcctgtggtccgcgccactcaggaggctgagacgggaggatcctttcagcctaggagtttaaggctaaagtgagccatgattgtgctatcgtactccagcctgggcagcagagcaagatcctgactctaaaaaaaagtaaaataaagtaaaatgggggaaatgaactgctttagtaacatcatctgttttttctgtgagcagcgtagcttgacagccattggtgaactcgtgccctgtgcttccctgtccagatccccattctgcccgcaacatggagtataacggtttattcatagtagtcgagaaacactcactgaatgaatgaatgaggtgtagaactaagtggagtgggtaattcaacacatattaatttccttcttttttttatttttagaaagaaagaactttcagctaccaagaaagaccgtgtgaatcattgtctgacaatatgtgaaaacatagtggcacagtctgtcaggtaattgcactttgaactgtctagagaaaataagaactttgtatattttcagtcttaatgggctagaatattctttgtgtcccagctattttaaatggattcagaaatccatttaagatgaagaaggacccttttcccatatttctggctatatacaaggatatccagacactgaaatgaataatgttccctttttgtaatcttttatgcaaaaattaaaaccattatggtaattgaacaacatgtttatgtttagttaacacccttagcaactatagttattttaaaaccatctatggtttgatatttttgcatttgttgcaatagtaggaacagcacaagacagttcagtttgtctctcttatttgctttttcttggcagtttgctgtcctattgtacctctgctcctagcagtggctggagcccactcctctgtgcttcgggattagtggggatcgtggggcattgactgtaggtcagctttccttgcttgatctttctcactgggatgaactagcagcaccttcttttgtagctgctttgcttttgactatctttctgaccgttgttcctagtagctgtagatggtaaatatatttaggcctgtttccaatggctcagtaggagacatattcacctatgatatctgaattctgttacccacatgggcatgcgtgaaatagttgccttgccttactttcccttggaataaataattcatgttattctcctggtagaagctagaaaaagcctttatagtcagtcagaaaaaaatttttagacaaataatcttgattttagtactgacaaaaacgtgtggtgattctttttttaatttttttttgagacggagtttcactcttgttgcccaggctggagtgcaatggcgtgatctcggctcactgcaacctctgcctcctgggttcaagtgattctcctgcctcagcctcccaagtagctggagttacaggcatgtgctactgtgcccagctaattttgtatttttagtagagatgttggtcaggctgatctcgaactcccaaccttaggtgatctgcccgcctcagcctcccaaagtgctgggattacaggcgtgagccagggcgcccggtgattcatttgttttttcaaaaaatttcctcttggccattgcttttcacttttgttttttttttttttttgagacggagtcacgatctgtcacccaggctggagtgcagtggcatgatcttggcttactgcaagctctgcctcccaggttcacgccattctcctgcttcagcctggcgagtagctgggactacaggtgctcgccaccacacccggctaattttttgtatttttagtagagatggggtttcaccgtggtcttgatctcctgacctcatgacccgctcaactcagcctcccaaagtgctgggattacaggcgtgagccaccgcgcccggccctctcttgtctttttattgtggtaaaatgcacataaaattgactgtcttaaccatttttaggggtacagttcagtatatatattcgtaatgttgtacagccatcactgccatctacttcataagtttttcttctgtcaaaactgaacatctgtcttcattaaactccctatcatccattctttcctgtagtccctttctactttctgtctgtatgagtgtaactgctctggagacctcatgtaagtggattcctacaggatttgtgttttttttttggtgatctgcttatttttaatgcctctgtgcatttgtattatatactttcaaagtgatttcacaaaaccgtttcattttaggttaactcatttctgttgtttgtgaaatactgtgtatgattctgttctgtttctgtctaatttgtggaaatgttgtgggaagaaaatgaaataacaaatgagcatatgtcctgaaaataaaaatataaaaattctaagttagcatgctattgtagaatacaacgctatgataaaagtaggaaaaaaaaaggtttgaattctatctctgctacctgtgtaagctgggtgactttagataagctgtaacgtgtttgagccttactggctcatttttgaaatgtaatccctagttacacagttcttgtgggatcagatggtacatgtgaaacactgtgaaaaagcaactgcatagatatgttcattagccacctgagcgggaagcgtatcccattgcgatgcccatcatccaaagctatatgttatctttacttttttttttttgagacagagtcttgctctgttgcccaggctagagtgcagtggtgcaatctcagctcactgcaagctccacctcccgggttcacgctattctcctgccccagcctcccaagtagctgggactacaggcacccgccaccatgcctggctaaatttttgtatttttagtagagatggggtttcaccgtgttagccaggatggtcttgatctcctgacctcgtgatccgcccgcctcggcctcccaaagtgctgggattacaggcgtgagccactgcccctggccatctttactttttttgtgaaatgactttaaatacttggcaaacatttggtcattgttcatctgatctccaccatccaggtctcagagaacataatttctctctgaaagcttattgacccaggaaataagatctctttcaatctgagtgcgtcaggctttattcttgtcattttgtcttttgataattttcaaatggaattcatggaatgttggcttatattcatatattagtaaagtatgttgagacatcttaagattgatttgtggttctatatgccatattaaatcaaaataatagctgttaatggttttcacattagtctgtctcttgtttttatggagtaatgctgagagttcattatgcttgttctacagaagagcatgttaaaaggagtttttggagtcagagaggttattcttggtttcataggatacactctatactttttagggatttcagagtatatagctgaaggtgatattttatgtaaatatgttttatggaaacttattgctcatcgctgtttcctgttaactctcctaaaatataattaaacttttggaacttttttatagcttttgtgctagactaatttttgtctctaatgaggttatataaatggcagcttctgacgttttcaatgtaggaagtcatttaaaacttcatgtatattgtgaaaatgtagtctgctttaagctctctaaagtggtctaagttactggttcctaagtatggatgagcatcaaaatcatctggaaaatttgttaaaaatacagtaatgaaggcacctcactgtcctttttcccaaacatacttctgcattctgtttgagtaggtagggactacacatttttcacaagtatcctcttgggaatacccaggaatgcttacttgagcaacctcttactaatatgtaccttgataaggtggctaggtaaacataaatatacaaaaatccatagatctcccatatattagcataaatcagctagaaaatataacgtttaaagatctagttcacagtagcaccaatatatcgaactctaaggaatcgataaatatgcaaaaactttataaaaacttctgttaatgtttctgaaagatataggtgaccactttctagataggaagattttatattactaagttgaattttctctaaattaacacagaaatttaaaataatcttgatcaaaattctagtagaggtatttttgaacttgttcactgcaagaataaatacataattgcaaagaatatctcaaaatcatcaccaggcctggtgtggtggcccatgcctgtaatcccagcactttgggaggctgaggcaggcagatcacctgaggtcaagagtttgagaccagctggaccagtgcggtgaaacactgcctctactaaaaatacaaaaattagctgggtgtggtggtgcatgcctgtagtcccagctacttgggaggctgaggcaggagaattgcttgaacccaggaggtacaggttgcggtgagcctagatcgcaccactgcattccagcctgggcgacaagagcaaaattctgtctcaagaaaaaagagaaaaaagaaaaagaaatcaacactaatatggtgagacttaatgtatgtgacattaaaatagtgattggatgttaaaacaggtatagaacagaaagaagagtgtatgtgtgtatctgtatgaatttatgatgggtgtaacatatatgtattagggaaatgagggaaatgatacatttctctgactttgggagaacattatatctctacctcatattgcaaacaaacataaagttcagattaattacctaaatgtgaaaaaatgaaataatttctttaaaaaatgtaatcttagtttgaggaaggttaacattataaaggaaaaaactgttttgagtggaatatagttcaatatgtcaaaatccaccttcaacaaaattgaaagtaaattgaacttggggaaagtattgacagcatatagatcaaaggttactagcctgtgtaaagagcagttataaatatcgttaagaaaaacactgtcgacctgtcggcaccttgttctccgactcccagcctccagaactgtgacgagtaagtgcttattgtttaaaccacccagtctgtatgtggtattttgttatagaaactcaagctgattaggacactagtaatcagtagactgaaactgaaacaaaaataagaaccttttttacctgtcaaattggcaaacattaagaatattcagatttttgtcagaggtgatacaaccttctaagaaggcaatttgggaaaatataaagctttagattattatatgtctgacctagcagttttacctctagggtgcttacccctaggaaagtgtgtaatgatattggtgcagtgcccttcatcccattagaaaattaaaaataaccttaatggcctaccactaaaaggggattgaaaatttaagatatatttatttatgtgtttattgagatggagtcttgcactgtccgcctgggccagagtgcaatggtgcgatctcggctcactgcaacctctgcttcccgggttcatgtgattctcctgcctcagcctcctgagtagctgggattacaggctcacaccaccgcacccggctaattttttgtatttttagtagagatggggtttcactgtgttggccagactggtctcgaactcctgacctcatgatccgcgcccctcggcctcccagtgttgggattacaggtgtgagccactgcgcctggccagatacatttatacaagagaatgttagttaacattcatagatatttatattttgtttactttttattaaaaaaattttttttagagacaggatcttactctgtcacccaggcaggatgcagttgcacaatcatagcccactgcagcctgaactcctgggcttaagtgatccttctgcctcagccttttgagtacctgggggactttaggcagtgctactatacctggctaatttttaaatgttttatagatgagatcttgctgtattgcccaggctggtctagaattcctgggcccaagtgatcctcccaccttggcctcccaaagcgctgagattacaggcatgagccaccacttctgaccaatagatatttatatttgtgactggaaaatatattaacaatgtgttaaaaaattcagttaaaaaataatgaaagatttttgcttctggctaagatagaataacaaggacagcatttatcttcttgccttgaaatagttgaaaacggaagaaatatatgtaacagtggttttcaagttattgggcatcaggcaaagaagaatagttatcccaggaaaatgaatgtggagagccctacaatttccttacattactgcctggtcatggcaagaggaaaaactgagaggagactgaggctgagccagtggtttgctgggttgaggaggcagagctgggagtgcagagatgcaaggtggtgagagcccatatggaagaataccagggaagagagctgcagagggagctccggagacctgcaccctgccctctcagtaccctgtcatgtgtgtagctgagtactgacgagcacttgcttgtgcggaaatgacccagggctggaggtagagccacctgaaaggattagaaggaacagttgctgaaagtcacacagggccaggaagaatttctaatcacaccagttggagtggaaaacctcagctctcatagagcaggtagggtactcagaagggtttgcccacctagccccagactaagtttcgttactctgaccctacctaatattaaaaagagattaattaaattgttcgcaacaaaaataatatatttcagtgtttgtaacacgtagaagtgaattgtatgacaatagcataaaggctggaagagcagaaattgacatgtatttgcgctgggcagaataatgctcccctctttccccaaaagatatcaagtcctaatccctggagcctgtaaatattactttatatggaaaattgttttatgatgtgattaaattcaggatcttgagatgagggggctatcttggatgatctgggtaggcactaaatgcaatcacatatatataaaaaggaggcagagggagattttacacacagagagaaggccctgtgaagatggaacagaaagatttgaaggtgctggccttgaaaattggagtgatgaagctataagccaaggaatgcagcagccaccaaagctggaagaggcacggagcagttctcatttagagcctactccagagggaatgtggtgctgccaattccttttttttttttttttttaagatatcatttacccctttaagttggttttttttttttttttttttttttagtatttattgatcattcttgggtgtttcttggagagggggatttggcagggtcataggacaatagtggagggaaggtcagcagataaacatgtaaacaaaggtctctggttttcctaggcagagggccctgccacgttctgcagtgtttgtgtccctgggtacttgagattagggagtggtgatgactcttaacgagtatgctgccttcaagcatctgtttaacaaagcacatcttgcaccgcccttaatccatttaacccttagtggacacagcacatgtttcagagagcacggggttgggggtaaggttatagattaacagcatcccaaggcagaagaatttttcttagtacagaacaaaatggagtgtcctatgtctacttctttctacgcagacacagtaacaatctgatctctctttcttttcccacatttcctccttttctattcgacaaaactgccaccgtcatcatggactgttctcaatgagctattgggtacacctcccagatggggtggcggccgggcagaggggctcctcacttcccagatggggcggccgggcagaggcgccccccaacctcccagacggggcggcggctgggcgggggctgccccccacctcccggacggggcgggtggccgggcgggggctgcccaccacctcccggacggggcggctggccgggcgggggctgccccccacctcccggacggggcgggtggccgggcgggggctgccccccacctcccggacggggcggctggccgggcgggggctgccccccacctcccggacggagcggctgccgggcggaggggctcctcacttcccggacggggcggctgctgggcggaggggctcctcacttctcagacggggcggctggtcagagacgctcctcacctcccagacggggtggcagtggggcagagacattcttaagttcccagacggagtcacggccgggcagaggtgctcttcacatctcagacggggcggcggggcagaggtgctccccacttcccagacgatgggcggccgggcagagatgctcctcacttcctagatgggatgacagccgggaagaggcgctcctcacttcccagactgggcagccaggcagaggggctcctcacatcccagacgatgggcggccaggcagaaacgctcctcacttcctagacggggtggcggctgggcagaggccgcaatcttggcactttgggaggccaaggcaggcggctgggaggtgaaggttgtagtgacccgagatcacgccactgcactccagcctgggcaacactgagcactgagtgagcgagactccgtctgcaatcccggcacctcgggaggccgaggctggcagatcacttgcagtcaggagctggagaccagcccggccaacacggcgaaaccccgtctccaccaaaaaacacgaaaaccagtcagacatggcggtgcgtgcctgcaatcccaggcacttggcaggctgaggcaggagaatcaggtagggaggttgcagtgagtagagatggtggcagtacagtccagccttggctcggcatcagagggagactgtgcgagggcgagggcgagggcgagggaattccttaatttcagtttagtgatactaattttggactctggcctctaaaactgtgaaagaaaaaattttttgtttgtttgtttcttttaagccacatagtttgtggtaatttgttacagcagctgcaggaaactaatttatgctgcatgtgaaatggtgtaataaggtagattgtgatgaagatacatagtataaacaattaagcaacaactaaaagcacaacaaggaattatagctaatgaaccaaaaaaggagattagaataataaaaatggtgaatcccaaagaagccagaaataggggaagaggcaaataaaggaaagaaagagcttgatggtagatttcaacctaactatgtcaaaaaggacattacatgtaaaaggcagcgatttttcagattgaatggaaaagtaagactcggtatatgctgctgcctgcaagaaacacattctaaatataaaggcaaaaataacctacaggtaacagaacggaaagaagttcactgtgcttacaagaattagatgcaagctagactggttctgttaatatcagacaaagtggatttcaaagcaaaggctcttgcccaggatgagatggtcatttcataatgatgaaggggattcgttcatcagcctggcatagcaagctgaaatgtttatgcaccggactacagagctaaaatacatgaagcaaagcctgacagaactacaagtagaaacagacaaatccacagtgatagagatttcagtagccgctctcaatgatttgtagaacacgtagccataatatctggatctagaacacttgaccaacactgtcccctgtgcaacctcattggcatttacaggacactccacccagcaccagcagaagagacactctctcaagtgctcacagaatgtttgccaagatagagcagatgctgggccataaaacaagtctctaaattaaaagcattcaaattattcagagtatgttttctgacctcagtatcattaagttggaatatattataggaagataacctggaaaagcctcagatatgtggaaaaacccatttccacatggcccatgggtcagaagtgaagtcaaaagggaaatttgaaagtcttttggattgactgatataaaaacaatagatttctaaacttgtggggtgctgttacagcatagtaaatggaaatttctagcattaaatgcctgttttaggaaagaaagatttcaaatcaatgacctcagcttctacctttggaaacttgaaaatgacaagcaaatggaatccagagttaccagaagggccaggtacggtggcttatgcctgcagttctgccactttgggaggccgaggcaggtggattgtttgagactggcagttgaagaccagcctgggcagcctagggagaccccatatctacaaaaaacaaaaaaattagccaggtgtggtggcatgtgcctgtagtcccagctaaccaggagtctaaggtgggaggattgcttgagtctgggaggttgaggctgcagtgaactgtgattgtgccactgtgttccatcctgggcaacagaatgagaccctgtctcaaaaacaaaaacagttactagaagaatggacatcataaagataggagcagaagtcagtaaaatagaaaacaaaaatacataggaaatcaataaaaccaaaagctggttcatcaagaacatcaataaattggtaaagctgataggaaaaacagtgaagtcacaaattagcaatatcaggaatgagggagatgacagtagtatagattatatagatattaaaaggactgtatgaggcaggtgtggtggttcacgcctgtaatcccagcaccttgggaggccgaggtggacagatcacctgaggtcaggagtttgggaccagcctggccaacatggtgaaactctgtctctactaaaaatacaaaaattagttggtcgtggtgctgtgtgcctgtaatcccagctacttgggaggctgaggcaggagaattgcttgaacctgggaggcggaggttgcagtgagctgagattgtgccgttgcactccagcctgggtgacagagcaagactccatctcaaaacaaataaataaataaaaaggactatatggtaatattatgaacaactttatgccaataaatttgacaacttatagatgaaatggatgagttccttgaaagacacagaaactattaaagctctctcaagaagatatagataagctgattagccctatatctattttattgaatttaaatgtaaaaatcaatatttagttactggaaaacttttaagtgtggttggaaatggtatacgaactttttcaactgaattttatgaagtctaatcacaggtaaaggttttctgatgaaaatttagtgtctgaattgagatatactgtaaaaaatgttatatatcttaattatttcttcacattaattacatgttgaaataatactttgggtgtattgggttaaattaaatattatgaaaatcttgcctgttttctttttacttttgatgcgtcagctaggaaatataaaagtgtagctcacattctgtttctgttgacagtactgctttggagcacagtgtttgaatgatctatcatttcaaagacctttcctcagttcgttattcatggctgtctgtattccacatagataaggtctgaaatactgctaagtggcatgttttgttttatgcttttataagtttgttgatcattactgatgtggacttttggtgcctcttaggctcattgctatcttccaaccattgtttgcaatttttacctagagataaagagaaagagacatttggtttcagagtagttagattgggatcatgaaagagcaacctcattttgatgcttcaaaaatagcacatcccccgtattactgggatttgctattcttgggattacttcaagaacatccttgtgttactggtttggatgcttctgaatgctgtgaagtcagtttcatgtacatggctcatcagtttagctctctcttggctttgtttagacagttggagcatgatggcctaaacagcttctttcaattaaacattttaaaatagtttacaaatagtaaacaaactccagtttttgtgactctttgtctcgcacaacaaaaacacaatctgaccatgatcatctggcatcttagggtgaaatatggttatactttggcccataccgaaagcaagattaaaaaggggcaggagagatagactgctgaactgattttcaaggttccaagaatattgtaggttaagagtaaaagtaaacttttggtagaaagcagtgggttgtctaggattgaagtatctgaagtttttaaacgaaaatttaaaaagaaaaatgagaattgccttacaagtacaatctcttcttttttaaaaaataaactttattttgaaatagttttagatttatagaaaaaaattagatagggtaggaagttttcatataccctacatccagttaccccagttattatcatcctaatttagtgtgagacattttcatgtttaatgaatcaatattgatatgctattaacttaagtccagactttattcagattttcttaatttctatgtaatgtcctttttctgttccagaattccatgcaggacaccggatacctcattacatttcattgtcatgtcaccttaggctcctcttgacagtttctcttctttttttgcttagaaattctccagaatttcagaaacttctgggcatcgctatggaactttttctgctgtgcagtgatgacgcagagtcagatgtcaggatggtggctgacgaatgcctcaacaaagttatcaaagtaagaaccgtgtggatgatgttctcctcagagctatcattgttgtaggctgagagaagaagcgatcattgagtgttcttctgttttgagtccctgaggatgtctgcacttttttcctttctgatgtatggtttggaggtgctctgttgtatggtttggaggtgctctgttgtatggtttggaggtgctctattgtatggtttggaggtgctctgttgtatggtttggaggtgctcttgtatggtttggaggtgctcttgtatggtttggaggtgctctgttgtatggtttggaggtggtcttgtatggtttgcaggtgctctattgcatggtttgcaggtgctctattgtatggtttggaagtgctcttgtatggtttggaggtgctcttgtatggtttggagatgctctattgtatggtttgcaggtgctctattgtatggtttggaagtgctcttgtatggtttggaggtgctcttgtatggtttggaggtgctctgttgtatggtttggaggtgctctgttgtatggtttggaggtgctcttgtatggtttggaggtgctctattgtatggtttggagatgctctggtatctgcctgcattgcttgccacacctgcccggtcagaaggcgctatgttgacaattgtgcctgcacggtgcctaggtcaatgaagggaaccgatggtagccactggatgctcctgggaaaatgtcactacaggcaccagagaagccagagctatgcccaaatttctatgagtctcagttttcttaaccataaaatgggatcaatgtttttgtggcatgtgtatgagtgtgtgtctgtgtatgtgtgaggattaaattgtgtatgtgtgaggactaattgccactactggatcctcaaagtggtaagaagtgttcttattaataatgacatccttacactcttacccagcaagattgatgggtgtggcactgcttctctttttccatcacatggtttccatggtatccttttgcccagggaatctttgctttgtggctagcactttgttgtttggctaatcacgctttctgtggtcaggacgctggcttctctggagccatgggattctagctccctgtcttgtccctagagtggtcactgtcttctctctccgcttgcaattcctgctttgctcgcatctcacttatgcagtgacgtatatcagtttcaccttgttctccgtgcctgctgatcattggcaccacttgcatggtgccatttagggcctgcttccagttaagcttgcttctccacaggcctaaatatccttgcttgcttcttttattctcactggcaggaccagggcggtctgtctttgcatgagacagggtctcgctcagtcacccaggctggagtgcagtggctgatcacggctcattgcagccttgagctaccgggctcaagctatcctcctggcttggccccttgagtagctgggactacaggcgtgcaccaccatgcccagctaatttttaaaattatttgtagagatgggatctcgccaggttgcccaggctggtcttgaacgcctgggctcaagtgatcctccctccttggtttcccaaagtgctgggatcacaggtgtgagccactgtgcctggcccttgatgtttcagttcttgatatttgatcctcagagtcagaaaatctaaaaagagggctatcccaggttgccttggttcatggcaaatgggacgttaagagggcagagagaatatgaacagaaactgttctaatattggtcatttaatgtgtaagtattgttcttttttaaacctccttcattttttttccaggaattgctggacacagtggcttggtgtgtgtctgaggactgtaggccatggccctaggttgtggttttaggtctcaggtgctcttcctggctgtctccttgcttctttcccatgtcctcttctttgtttccagccatttctcccttatgcttaagtttggtgcagcagggtttggctgctctcagattcctgcttcctcagatgctgtagttgtcaggcccagcgggctggcagcgggatcaggatctggctaggtttgctctcactgtggcagagtagggggaggcgtgggagagcacgtgtgaccccaggccagctgtagggagcataggcatggtcacgtagccttcaggtcctagactttgtcttctcatgagtatggctgtgtgtgtatggtgaaaactaggttctacttagcccaagaaaatgggcacattttgcatgtggtttctgtagagaaatgcactgggtatctgacatagcctggcagcatgcctccctcaggtaggttagtctcaggcggtgaagcacgtgtgtccagcaagaacttcatatgtggcataaagtctccgttctgtgaggtgctggcaaatcaccaccaccgtcaagaggctgaagtgatttttgtctagggaggcaggaaaggcttcctggagtcagcagccagtaggtgaaagagtagattggagaccttcttaatcatcaccgcctcttgtctcaaggggtgccaggaagctgtggaggctgaacccatcttatgctgccagagagtgggacaccatgagggtcaggtcaaggggttgtaccttgtttggtagagaattaggggctcttgaagactttggatgtggtcaggggagtgtatcatttaggaagagtgacccggtgaggacgtggggtagaggaggacaggtgggagggagtccaggtgggagtgagtagacccagcaggagtgcagggcctcgagccaggatggtggcagggctgtgaggagaggcagccacctgtgtgtctgcggaagcaggggcaagagggaagaggccagcagcgtgctgccatcacccagcgactggcgtagattgtgagagaccattccctgctcttaggaggggctgagttttagttttctcttgttatacaataagcttggtatttgtttacaaaacatttgtaaagctaaatcaaggtttgataaggcttctagttttatttaagaagtaatgttgaaataaatgtttgtccaattcgctttgctcatttaaggactttcagtacaaactgcaacaacaggattaggatttaaacgtttctgagatgtttttactcctcagaatttcccagaatgtgatctggttttgattttcaagcttgctgacccaataggttaacccacaagttttacgaagaccatctcagtccacttacatcaactgcccatgccacggttaaagagatcatcgactgatgtttggcacagcttcctccctcttgggtgggcaagcatttggaagagaaggctcctatgggtgagagtggggcaccaaagtcttccctgtcccatcccctagcttgagaagcccttctctaatgtggactttgtgccgttagcatcgttactagcttgaagttgaccatctggacgtactttctggtttagcctcacaagtgagcaaggagggttgagagatgtgctgtgaggaatgtggggccccagctggcagcaggctctgggtcaggggggcagggaccacgggcatacctgacagtgaggaggggccacacctgcagaaaaggatgcaggactccgccttgggaagtgttctaggccagagcgagggtctgtggtttataagtacacccacagtgctcgggaccctgcagatgtccagggtgccgtctgagcccgtatcatccaacagaatgttctgctagtgaagattaaagatttactccaggggctttaggatttattatatatatataaatcctatatatataattttttttttttttttttttgagatggagtttcgctcttgttgcccaggctggagtgcaatggcgtgatcttggctcactgcaacctccgcctcccgggttcaaactattctcctgcctcagcctctcgagtagctgggattacaggcgcccaccaccacacccggctaatttttgtattttttagtagagacggagtttctccatgttggtcaggctggtcttgaactcctgacctcaggtgatctgcccgccttggcctcccaaagtgctgggattacaggcatgagccaccccacctggccaggatttattgtatttgaaccatctaccattttaattttgatgttatgtagtatttgatgataatgaaagttaaattgtttttctttccatttttctgtttaagtgaatgacctgtatctagtttattcagtaacttcctgcatatatttgtttctttcattcttaatgaatatattcttaatttagttgctattatgttttgctttgccccaaaattgaaatcttagtttccttttagctcgttttagaactagtgatgggatgtgtcttccataaatctcttgtgatttgttgtaggctttgatggattctaatcttccaaggttacagctcgagctctataaggaaattaaaaaggtgggccttgcttttcttttttaaaaatgttttaaattttaaatttttataggtacacgtattttgtaggtacatgtaaatgtatatatttatggggtacatgagatattttgatacaggtatacaatacataataatcacaccatggaaagttggatatccatgccctcaagcatttatcctttgtgttacaaacaatccagttacatgctttacttattttattttatttttgagacagagtcttgctttcacccatgctagagtacagtggcatgaccttggctcactgcaacctccgcctcccgggttcaaccgaactttgggctggtctcaaactcctgacctcaggtgatccgcccgcctcggcctcccaaagtgttgggattacaggcgtgagccactgtgccgggcctgattgtacattttaaaataactaaaacagtcagggcacagtggctcatgcctgtaatcccagcattttgggaggctgaggcaggtgatcacctgagatcaggagttcgagaccagcctggccaacatggagaaaccctgtctctactaaaaatacaaaaattagccaagtgtggtggcgggcgcctgtaatcctggctactcgggaggctgaggtaggggaatcgcttgaacctgggggtggaggttgcagtgagccgagatcacgccactgcattccagcctgagcgacagagtgagactttgtctcaaaaaataaaaatgaaataaaattgggccgggtgtggtggctcacaccttagtcccagcactttgggaacctgaggcaggtggatgcttgagaccaggagtttgagaccagcatgggcaacatggcaaaacgctgtctgtacagaaattagctgggtgtggtggtgcacaactatagtctcagctacttgggagattgaggtgggaggattaattgagcctggaaggttgaatctataggtagctgagattgtgccactgcccttcagcctgggcgaccaagtgagaccctgtctcaaaagaaaaacaaaaaaacaaaaaacaaaccactattatcgactatatattattgtctatgatccctctgctgtgctgtcgaataccaggtcttgggcccttatttccatcactgagcaaacttcactctgttaagcagcaggtgtgggatttcatcgttattcagtaattcacaatgttagaaggaaatgctgtttggtagacgattgctttacttttcttcaaaaggttactctttattagatgagatgagaattaaaaatggtaacttactttatatctttataattgaagcccactagaccttaaagtagttaccagatgttttatgcatttaaatggccttttctctaaaattagaaagtaacaaggaaagaaaatgcttcgtttctatgcaaccctcttggtgactagtatgtgactcttaatgcaaccctcattgcaccccctcagaatggtgcccctcggagtttgcgtgctgccctgtggaggtttgctgagctggctcacctggttcggcctcagaaatgcaggtaagttgtacactctggatgttggtttttgtcgggggccagctgctactgatcctttatgtctcagctcagatgtcatttcaaaagtctgctctgccctctccaaattgcagtcgaccttgccctgtttatgtttccctcatagcactaatccatgtcagaaattgtcacgtacagtctatctgtgtgcttgtttattttctatcccacccttccgcaagagacttatgggatgtgtgccccaggacagcaggggtcttactgtcttatgctctgttgcagcccagcagcgataacagtgtctgcacatagtacttgcttaaaagatacttgccaaattgttgaaggttgaggtaccaatttcattattgctgactataggagttatagcaaaatatccatttgtctgttacatgagttaaaaatatggttgttgcactgtgaatagtttggtttagtcaaaacagttgtatcttaacggattgagaaacaaaagcaggaccacttttcatcagctccctccttctccttaaccagcaatacatgctgatgctgatatcccatagaccctcagctccatcctgagtcactgggaatgtggtctaaaccctcactattaatatgaactgagtttcaataagaatcttatatgggtcgggcatagtggctcatacctttgatcccagcacttcaggaggccaaggcaggtggattgcttgacccagactaggcaacatggtgaaacgccgcctctacaaaaaatacaaaacttagccaggcatggtggtgcgtgcctgtggtcacagccactcgagaggctgaggtgggaggatcacttgagcctgggaggtggaggtcgtgttgagccaagatcgcaccactgcactccagcctgggcaacagagtgagacctgtctcaaaaaaaccaaaatccagaaaagaacttatatggctgcagaggtataatcactaaggaaatttccttttgtataatcttttttcttttactatcatttaaaaaaatgtgttatatttctgaagcaacacatccaggttctgcacatagcagccaaagtgaccttaaagaatataactgggtcttgtcattcccttatttaaactcttgtacccatttcccagtgccgtttagatagagattccagactcgtcaatggctctgtcacctcagacaccctgcattgactcattagtctgattagagtcaggtttttcttcctcctgatggtttttttttcccccttagttctcagcggaacagtcacttccttagggaggtttccccagccaccctctgaggccgtgcttgttgccagactctgccactagagggcagggctgcaccactcctggcacctcgcacccggcctgccctgtcactctgtgtgttgggtgaattcctgtgatctgtgactcactgctctgtgtcctacacattcggcttttcttctctccccacaaccccattttataattctcctttttcaggaaagctttattcccatttaaaaatttttgtttttaaaatggtattttcttacacttattttctaattaaaaatgagtgttttaagaagtattatgatttactgcaaataatttttaaacccagccttttagatcctctgtgatcataagagaaatgaaggatgtctcccaacacttgagcttcatccacatttcatcctcctgttctttcagctgagttttccccatcccattagggactgttggaatataaaactggcttttccctaacagggaatgaattgcttctgtttctcctgaaggagagctggaagaatgacttgcgttcttttgcatacacaggccttacctggtgaaccttctgccgtgcctgactcgaacaagcaagagacccgaagaatcagtccaggagaccttggctgcagctgttcccaaaattatggcttcttttggcaattttgcaaatgacaatgaaattaaggtatgattgttgcctcaggtcacaaacatgcgagtgatgctgtgagtgagtctgtggagggtgagggcttctgaacagggagtcctgtgggagtgcttcttggggtatgttgtatgtcgtaatttagactaccatcatttgtgttatttttgaggcacctaaggacttctttccacttctcatttcttactgtggggtgaagagttgaattgggagatggtttctagatgcaaattgaaaaggcatttttccagagcagatttgttttcggcgtactagagtgactctttaacctagctgcgggaagatgactgtgccaagactgcaggtaggagaaagctcactgacgaggccttgtgggtctgaacgtcctgcagctatcagagcctgttggcttcctgttgtgcattccaacaaatcatcttcaaacccactttagtgttttgtttataatgtccagaaatagtgaccctgtcacatgctctacagattacaggattcttagcctcttcctttttggtaggtcagtcctgggtttgagcccaagtgaccctcctgggaggtgatgatacacactgggtagagtggaatcagatggacttggattagaattctgtcctctttactagttattttcctctaggcaaactgcccaacagctctaagctatttccttcgtattctgaaaaataagccttaatgggacccatatagggcaactctgagagtaaaataaaggaatatgtgttagagtgtagcatagtcacccacgggaagggcttagatgttagctgctactgctcttattagctgaatgatttggaataaactgttagcctctctcatgttttttctcttgagcttcgaagttttcttgttaatactaaggagatattcaaactagtcatggggttttggaatgacgaagggagatgatgaatctaaagaatttagtgtaatatttcttcatgctcagtaaatggtagtttctgctgctgttatttttattaccatctctttggaatgggagtaggtgctcctttgtggtcagaggctgtgagagctccacagcgccagtttgcccatctgtacactggggtctgttgaaggcagtcccctctgtgatatctctggctgtcagagctcagatgatagatggtatttttgtactcttagttctcatcattttcatgatttcgatcaccatttgagtatgatgatgctaacactttgttgaacgtagaatccgttaattacttccttcctgaacctttggcattaaaaaaaatctattctgctacctctctgctcatttatggttattcaaatttattatcaagagcctggtacagtggcttgtgcctataattgtagctacttgggaggctgaggtaggaggattgcttgaggccaggagtttgagaccagcctgggcaagatagtgagaccctatctctaaaaaaactgaaaaaaaattagctggacatgatggcatgtgcctgtggtcctagctactcaggaggctgagacaggaggctcggttgagcccaggagttggagttcgaggctacactgagctgtgattgtgccaccacactccagcatgggtggtaaaacaagatgccatttcttaaaaaaaaaaaatatatatatatatattatcaatgaaattcagtagtaccaacaggattataaacaaagatagtagttcccttcctactttttctcttaatccttgtgtctcacaggcaaacataactcttagtatttcttccaatatttactttcatgtttctttctttctttctttttttttctttgagatggagttttgctcttgttgccaaggctggagtgcaatgacgcaatcttggctcaccacaacctctgtctcccgggttcaagcgattctcctgcctcagcctcctagtagctgggattacaggcatgcatcaccacgctcggctaattttgtacttttagtagagatggggtttctccgggttggtcaggctggtctcgaactcctgacctcaggtgatcctcccacctcagcctcccaaagtgctgggattacaggcgtgagccactgcgcccagcaacttccacatttctaaataacatgcttctactgctattttttttttcaattttagacatttttttactttcactatagttctatcagaattcagtgtgtacgttattatgcctaagtaaatagtcatggttgcttacgtattatatttctttgattgtgtttcttatttgatgagaaagctgtgttttttgctctgggttgaaactggagagaggacctggggaggaggaggaggacagatgaagttggtgactgtaccttcatggccatagctgggttctcagcacccggggatctgctgatcacctactcataggccaggcccctatcgaagttctaggtgacccagtgctggggacgggggggccacctgcaaggtctaatcatggaggtgggggctacagtgttggcttgtgctggggccagcatccttaggaaggcatcttggaggtggaggagacagccgcccacttcttgattggggccttcagcagcaccagcttcttgggcaggctggtgctggctttcatcaccatgtcgtgttcaatcttcttccagatcctgacttctaggttcagctttcctcagaccctggttcctttcagaggccattgctgctgccttgctctttgctggcttgtgccttgattatatgtctttgtacaactttttgttttcctggagttaatcttcacatctgttttcttggagttaatcgttacctctatatcgcttgcttattattctttggcctttttgtcttctcacaccttccaacttctttgtaatatgtgtttagtacaatttttcatgacaggtagtttactgaatcagtttttccccagtgtggtcatccaacttgagttatccagctctctgccccagtctgggcaggttgatcttcaggtctgtagtacacttgtatcctaggacttctctttgccattagcctggaatttcctttgcagttctcccgttggatgcccagttcctagatgccatatgtttttctatcgtctagtagcttcctgagagaagatgaatgggagggaaattgtatgaggttttgcattcataaaaatgccattttttttcctgtacacttggctgggtatggtgttctggggtagaaatcattttccctcagaaatgcaaagtctttgccctgttgtcttaaaatctccaacgtgacccgattccttaacctatgaatgtacttttctttggaagctttccatttttggggaggtgaagtgctaggtacttagtaggccttttaatttggaaacttacatcccttcagttctgggaaaattttcttaacatttctctgagaagttcttgccttttattttctgtgttctctcctgaaattggttagttggatgttggtcctcctagattgactcacatcttacctttttcttttctttttctggtactttttagatatccatctcaaactcttctattcattgttatgtttttaacttctttcttttctttgtctcttgatggggtcttgccctgttgcccaggttgtggtgcagtggtgcgatcatagctcactgcagcctcaaattcctgggctcaagcagctgttctgcctcaccctcccaagtagttgggactacaggtatgcaccaccacgtccagctattttctttacttttttttttttttttttgagatggagtcctactctgtcgcccaggctagagtgcggtggtgggattttggctcacttaagcctctgcctcccaggttcaagcagttctcctgcctcagcctctcaagtagctgggattacaggtgtgcaccaccatgcccggctaatttttgtatttttagtagagccagagtttcaccatgttggccaggctggtctcgaacgcctgacctcaggtgatccgcctgccttggcctccgaaagtgccgggattacaggcgtgagcccatcattagatctttaaataccagtatctataagtcttttcctcttgagtcagctagtatccctggaaggaaattactcattttcctgcttggaggctataagcttggctatgtttatcctgcaaccggggactggaagggaggggactgacagtgttgctggtcagggtgccctcttactttttgttttctgtgtgcatctcacgtctgtcctcagcctatgtaaacacctcttgagattatccctctcaatctttgccggaggtgggggaggggctgcttcctgggctgccttggattggagggaagacctcaggtgagtgggtgggaatttgcccaaggagccatgagaccagccactatttcaccctctccatccctccactttcagatgtatgtggcgcctccaaagcccgagctcttcttggcgtctgtggcttcaataagcttgctttttgctggtatccctcctaccctcccctgtccccagcaaagcttgcatttgaacttcttcctacgggctaacaaatcagtcagttatgtagctcttgttactttttagcttccgaagttttgttgacacccgtagtctgctaatgtccctgttctgttctttctgttcgtgtaaatatatgctttatacaacttctttacatgatttttgtggggtttctgggtagcagagcttcacaagttcaatccagcgtgttggattagaaatctcccaccctctggtttattcttattctcaaaattacctgccaaacactgatactcccttgtttttccttttcctgacaggaaatgtacataccatacaggacagaaatcattagtgtatcccttggtgaataaccacaaagtgaacttaacccttgtaaccgccacccaggtcaagacagaatattaccaagcactcagaagcctctcccctattcccccgtcactgctcctgccttcctccccaaggtcatgactgctggcttctaattccagagtctgtttttaaattctgtgtacatagaccatggattaagtgttctttttgtctggtttattttggtcgacattaagttcatgagagtcttctatattatcgtgtgtattagtattcctgtagttttaggagcttcatagcattccattgtagggatataccacagtttattcattgtattatcactgggttgtttctagttcttggctattgcgagcagtgctactgtgaccactcttaggtgtgtcttttggagtacatgtgcaggtttccatcttgcacagctagaggtggagttgttgggtgatagggtgtgtgcatctcagctgcagtagaaactgccaaatagctttccttgagtgcttgtaccagctcacccttttgccactgtgtatggggattccaggagctctggtcctcgctagcacttggaattgctgatgcttttactcttagccttcctgatgggtgttttctggaatcacattatgattttaatttccattccttaaagtacccttggctctgaagtttaatgattcatgcatctcttcccttttgaagtactcttacaggtatgttgtgcatgtgttgaaaagtggcactatctattctaaaatacagtatgcctcctctgtgtttgaacagttgtagcgtggccttggggcctcctgttagctggcttggagaagggattcttgggattgtagagattagacctgaggaggccccttggagctctctgactaaattttattctttattattccaaactatttaagctcaccgtgtgctgactcatcataataatgagtagctctcattgtgcttgtctatttggactcatacaatgattttttttttttctttgagacagagtcttgctctgttgcctaggctggagtgcagtggcacaatctcggctcactgcagcctccacctcccaggttcaagtgattcttgtgcctcagcttctcaagtagctgagactgcaggtgcgtaccaccatgcctggctaatgtttgtatttttagtagagacggggtttcaccatgttggccaggttggtctcaaactcctgacctcaagtgatctgccttcttcagcctcccaaagtgctgggattacaggtgtgagccactgagcttggccaaagtagttttttaagatgttagtatcttttcttgcagctaaaaaagtttgtcagagatgattctactttgttctccaggtgttttctcagggagaaattggaggcagtaagccactgggggagtcctgtggctggggggtggggtagtcctgtggctccttgtcagggagtcctgtggctggcaaggagagaagtcctgtggctgggttgggagggagtcctgtggctggggtctcatcctgtgcctaacagtgtccagaggtgccgagaccagctcagtcggggagaccctaacccagcagcgctagaggaattaaagacacacacacagaaatatagaggtgtgaagtgggaaatcaggggtctcacagcctttagagctgagagccctgaacagagatttacccacatatttattaatagcaaaccagtcattagcattgtttctatagatgttaaattaactaaaagtatcccttatgggaaacgaggggatgggccgaattaaaagaagaggttgggctagttaaccgcagcaggagcatgtccttaaggcacagatcgctcatgctattgtttgtggcttaagaatgcctttaagcggttttccaccctgggtgggccaggtgttccttgccctcattcctgtcaacccacaaccttccagtgtgggcattagggccattatgaacatgttacagtgcttcagagattttgtttatggccagttttggggccagtttatggccagattttggggggcctgctcccaatacagaggtctcgtgtaaattccctgggaggcgataagcctctgagaaacagactatgctaaccacgccatgaaagagaaacttatttataaatcagatgccagttactagtttactgcttatttgcccaggcgtagctctgacagagtccccgactcatagtgcttgctcagtgcatgctgaacaatgattggaatcaagtcatggctcagagcatagttttgaataatgggaaatggatgttcttaagtaacatagtcaccaagataatgcgactagctgggtcaccccttttcaattttaggatatttttatcaagatttaaatggccatcattagagttatagcactttctcctttggattgtcctagaggcccatgagaaagtattccctaatttcttaggagaacagtttgtgggtagtatgcggtcatgtccagttaaattgcagatatttccgatcgaagatgttccagtcctgagaacttcgtgacattagcaggacttctacaagccatctcttagggtggggcatttactgcagttggctagtactcttttctccttaactttgtcatttgttgatttttttttaactgtccccaaatactgtgggcagagtgtatctagaattgaggcctccaccattgcggagaggacatggatgctgagcagtcccctgagtgaaggttataaagaagcaaatagactacacatgtctgtaaactgctcttgagtgtcccaaatttggggtacttcagttcagctgtaggaaaagcctcaaactgtttatactttgcaagaattggaaacttctaattcacgttaagttttatgtaatacatgataagcttcataggagcttcatcttttatctacttggacttttgcttccgtaggttttgttaaaggccttcatagcgaacctgaagtcaagctcccccaccattcggcggacagcggctggatcagcagtgagcatctgccagcactcaagaaggacacaatatttctatagttggctactaaatgtgctcttaggtaaggtggaggcatatgagtggaagagtctccagcatgtactcaagatagacctttgaaataaataaaaccagatgatccctcagcttctagaccaggctatttggcactggttgattgaatgtgaactgcactggggctgctgtgagcccgcatgggtctctgtgaccctgcagatgcagccgtgcccagggactgggcagtgggtgtgggctggtgtgagccctgtctgccacccagggcctggccctctgtctgtgtcggccatgactatggtgagtcttgtaggcttgagactgtgcctcgggttcctgcgggttctctgtaggtcagttgacagtttctcctgttgtttgggtaactgtggaaacgaacactggcaagtgctgaagcgagcatgtggacgtgcgatatgaaataacgacctggctttcaaaggcagtgaggctctctggaaaggaccttgctgagctagggatgtgggtgtgtagccattcccagtgggcctcatggcgtactcgttcatgatcatgtttgtgccatcttgatctctcaggatctcttcttttttaacagattaagccgggaatctccaaacagtgagtcagatgttaagatgtcttgcttccacccccacaggcttactcgttcctgtcgaggatgaacactccactctgctgattcttggcgtgctgctcaccctgaggtatttggtgcccttgctgcagcagcaggtcaaggacacaagcctgaaaggcagcttcggagtgacaaggaaagaaatggaagtctctccttctgcagagcagcttgtccaggtaggagcacagggtttactctaggccctgcatgtgaatgactgacattcaaagaaccgattaatttggaagagaagcggcagaaccgagagttagaggtgtggactctggagctgcgctgctcgtttccaaccctaggtgctgacctctagctgtcttccctctgtatgtccctgtcaccgtgagtcaaatgcgggtgatgcctcctcaggtgccgtgttacctaagcctctcagagaccactgctaccctgtttctaaaaccagaggtcacgatatgtgttcatccacccagtaaatactgattgagcacccactgtgtgctaggctctgggataggggctgggtatacaatggtgagtatttcagctgcagcttctgccccgtggaggctgtggcctagcacactggtctaggcacggtggtatatgctcactcaaggagatagggacgtggtcgtttggggtgtcggaacaaaatgtcggaacttctctttccaatgcagagaaaccttgcagtaattctaatgtactgtgattggcagttgacttcagttctttgtagcacgcttactcaggttatttcactaactatgtaaccatgcagcctcattttaagcaattggattttttgaactttacttaaaatgttatgtcagggtttttattgtgcttaatgtgtgccatttagctaagttttgtaggatacgaaattgtaagtggcttaaaatgattcttaatagaatcatgaattgaagataatgctaataatttaagcactgagttaggtagtgtttgtaaaatgcttagaatgcttcctggcacatgttaaggccatgtaagtgctgcgtgttgataaacagctgagcaaaagtggactcttaagaaagtattggggctgagagttctgttccaaccagctgccctttggttatttttcagaataaaagcagagtctcatgggatatgacatttatatttccttcacaaaaaacactgctgagtgttttgttgagtaaaaagggtgtagccatggtaataatacatttaaaatatagtttatttcatctttaccttgccttgttttttttttaagctagctttttattgagaattccacacatacaaaagtatcaactcatgaccagttatatttcatttataatcctacttctccctttttttattatttgaaagcaaaccccaattatcctcttatttcatctataagtatttcagtatctctatagatgaggactcttctttatttttaaaactttatttttaaaatgatggtcagatgcagtgttcatgcctgtaatcccagaactttgggaggccaagctgggcggatcacttgaacctgggagtttgagaccagcccgggaaacatggcgaaaccccatgtcttaaagaaaaaaatcagccaagtgtggtgatgcatgcctgtagtcccagctacttgggaggctgagatgggagggtcacatgagcctggaagatcaaggctgcagtgatccatgattgtaccactgcactccatcctgggtgatggagcaagattctgtctcaaaaaaacaaaactgcaaaacaacgtcacaaaacagtgccattgttagacctgaaaatattaaacatttcctacatcaaatacccaccaactcattatcaatttttctctctactcttttggaatcagcatctaaataaaattggtcgataaggattgtaaatctctttgatgaactggttcccctccatcccagtttttttcccttagagttcatttattgagaaaccagattgtttgtcttctaagttttcctgtggtctgatatactgcttccatctccactgtgtaaattaacacctttttctcttctctgtatttcctgtaaatcaataattggaggaaaagccttgtcagatttagtgtatattttatatctgagtccagtatttcttatataatattttaagataagtgtactcttttaaaaagtattgaaactatatgctcaattttttttaactgatgcttttaagaaggctgcttgatcataaaagtttagagatcattggtctgatgggaaaagcaaataattactaaaccgtttagcaaggttgaggtgcacatggtggggcctggagaagttcagtcatgagccgtcacttatgggcacgtggaatctgacccggcacagagttgggagaagacaggagctttatagacagaaaatgtggtctttgctaagtcccaggagtgaaagggtgagacagtgctcacagcacacgagtgtgggtgcgtagacagagcaagggtgggtcctgaaaaggcctgcaggctttctcatagattagcaagagtgctggttacggaggtttctaacatttgtgaacagatcgaaactgtgttaaattgggattgcagtaatcctggaaggacagggatagagggtgaaggggaaaaaagggtatggatgtgagacttaattgctgattttcttaagacctttctccaaagtaaataaatgatgtggcacatttttgaactggcaaattctaaactctagatatgattatctctataacatatcttactccatcttcttttgactaaaaactgttcttaattaaattaccatgagacgttcaattcagcaaatgtagtttggctaaccatatttaattagaatttaatataatcctaggcctggccaaactattaagcaagtgtgggcaaaatattgataattttagatatgcaggaacttagtttgctttccatgtgtgcttttcgaaaaaggaataaattgaaaaatagaggaagccctgaaatccaagaagcaaactctctcacctaggcatgcagtaaaagcaattctaggatgattgctgtttggcgcgtagttcgtattagaaaccattcttcttgaataaatagtatgtttaagaagctgggcagagggaaggcatatgcatatattatcaacaaggagggagaaaaaggcaattagtaaccatccataggagggtcagcaagatttataaaggaaatttgtgatccaagtatgaagcaaaataaggtgcagaataaattttaagcaagtaatagattagagtaagagaacccatttgaccattaaccttgggacattctctttcaaatgacatggagtagtactgaaatctttctttctttctgagtctaggttattgtgactggactcagaaagaaatatttcattattgcagtgaataacatttgtgaacattattgttcataaattatgcagtgaataacatttatgaacacgtgatgtgtaagatacatactgtttatttttagttaagttttttggctcaacttctaggcagagaacattaaatgtaaatagtgttacctaggagcatgtaaatggaaatctccatagtatgaaagcagtgctgttgctaacagaatttaggagggggcagatgaggtgaaggaaatgtgggtgctgatttccttattacattgagaggagccaggagattctttgttcaaaatggatggcttaagaagtcaaagtataagctgattacgtagagcaggtacccaaaaatgttttgtgtaaggggccagatagtaaatattttcagtcttgcaggccatcccaagtctgtggcagctactcaacactacctttgtagcatgaaagcagccacaggcagcccataaatgtggctctgttccggtgaaactttaggtacaaaagcaggtgcaggccagacctgacctgtgcactgtggtttgctgacctgggattcaggggtatagaagttaccatcagaagagctaaaagtgagactttttactttatactcttctacactgtctgattttgaaaaaaagaaacatgtattttataatattaaagatagggttggcaaatagcaaataaaaatacagaataccagtgaaatttgaacttcagatacattatgagtaattttatggtgtaagtatattccaaatcatgtgggacatacttacactacaaaattatttgttgtttgtttacagtttaaatttgagtgccttgtattttatctggcaactgtaattaaagggaaaaagaataaattcattatgttcatataatgtgatatagcaggggtccccaacccccaggctgcagagtggtactggtccatgggtccccaacccccaggctgcagagcggtattggtccatggcctgttaggaaccaggctgcccagcaggaagtgagcagcaggtgagctggcattcccacctgagcaccgcctcctgtcagatcagtggcagcattagattcccataggagtgcaaaccctattgtgaactgcacatgtgaggggtctaggttgtgcgctccttatgagaatctaatgcctgatgatctgaggtggaacagtctcgtcttgaaaccatcccctggccctgtggaaaaattgtctcccatgaaaccagtctctggtgccagaaaggttgggtagcactgtgatatagtattaaaagtgctaataaatatggcatactgcctttaaaatgtctggtagctctttctcagtggcactcataatagtgttttttgatttttaaatgtgtgtcaagctgactctcccctccgtgtatgctgggctttattttccctttcctagtcaccagttttgggaaatagagatcttcattctcatgctgctcctctagtgcaagtgctccatttatttttaaggaattaatataacaaaaaatcatgggaatttagaaaacaacatggaagctaatgatcacattggtggaagtgatagggaaatatttagggggagaagttaaggtataaactttgtcaatgaagtcctattaaaaacaacaaaaaagtgaagcttaggatgcattttataaactctgaccagaacacctgtgtttctctgtttctaggtttatgaactgacgttacatcatacacagcaccaagaccacaatgttgtgaccggagccctggagctgttgcagcagctcttcagaacgcctccacccgagcttctgcaaaccctgaccgcagtcgggggcattgggcagctcaccgctgctaaggaggagtctggtggccgaagccgtagtgggagtattgtggaacttataggcaagttattagcaaggtctactcttacaattaactttgcagtaatactagttacactctattgattatgggcctgccctgtgctaagcagtctgcattccatcttccttgccaaaacttataatacaaatttcatctttattttataaataggggagttgggctgggtgtggtggctcacgcctgtaatttcagcactttggaaggatcgcttcagcccaggagtttgagacaacctggccaagtgagaccctgtctctacaaaaaaaaaaaaaaaaaaaaaattagctgggcatggtggcacatgcctgtagtcccagctgctttggaggctgaggtggtaggattgcttaagcccaagaggttgaggctgcagtgaatcttgatggcagctgcactgagcctggtgacagagcaagatgctgtctcaaaataaatttaaaaataaaataagagaattaaagtttagcaggttgggtggcaaaatgaggccacacatttaaagcccctcctcctgattcttttctctgccttggctgcctcctgtggcattttaggtgctgagaaatgaaaacagtagggaaaatagttccaggatcctcatgttaatttgccagaaatggcatcttcaagtcgtcagagggatctgagagttccttcctggcctgacttgagaaaatccgtctgtccccagctctgcgtctgcctccactgcccagtcacctcctctccatgctcttggggctgggccctaccccaccatgcagtgctgccctggagcagtgagcttggtgggtcctgtctggcatgagagctgcctttgggagctggatcccagcctctaccactgggtctggtgcctagcaggctatggataaacttctgctgactccggcctctcctaagccactgcaacgtggtcggtgtagtgcacagtgtgtgtgcagcgtggccttactcacagcctccacattagagagaatctgactgaagtcttactgctgcctcgtgtgaacataaatgtttgccagaaccatgagcaggaaatgttaatctgccttgtttcctgtcctttacacggaagaatttttttctgtatggaatgcgtgccttacaaataatgagtggaaatacccatcgctaatgaaaagttatacttgactgttagtcagctaaataatctgagatttctaatacttttaatttggcttttacaatgcaatttatcttagcttttttgatttcttaggtcatatctttagaactatatatttgaatgttaatgtaattttcatattgaaattaaaatgttgaactgcgatgttaagtgtttcctgtggaaaaacgttcacattttctctagttttaaagttgaatcaagctgtttgaagattttcacatttcttctagattttatcagcttgttactttatctgtcactttctgtgatttgcagctggagggggttcctcatgcagccctgtcctttcaagaaaacaaaaaggtgattatttcagaaatcagagtcttgtgttgaatcttactgattttcttgtatttctgtaatgtaatgtatcttgtatttcttgtaatactgtattggactctgtgtatatctcttctcagatgagtgattatatgtgtgaatgttgctggaatctgataaccaggcctgaatagttttgtagggtggcttttaaaaattactttcatatcagaattgctttgtcataaattttgaacgcatcataaatttctaatgttcggggtcagcagactttttttgtaaagggacagagtgtaaacatcttagctttatgggccatatggtctcttttgcaacattcagctctgccctgtgacaggaatgcagttgtaaagacatgagctactggccagctatgttccagtagaactttacttacagaaacagacaggctgtagtttgccaatacctgccttagggaatgtgttgttatattttgtgagttaccttctcagtaaattttatttagtattagtcaggaatattattaagtagcttcttttccagcctggtcaacatagtgagacccggtctctaccaaaacaaaacaaaacaaaaaaacagccacgcatgtggcatgtgcctgtagcctcagctgctgctcagggggctgaggcaagaggattgtttgagcccaggagtttgaggtcacagtgagctgtagtcatgccactgcactccagcctaggcaacagaatgagaccttgtgtcttaaaaaaaaaaagtttcctttgttgggttattttaatttggacctggttatcatttttcagccatatttaactttgtacatatcagaatgttctgataaaacttaacttttattaaagtgtttgtgatataatctgctagttttggtacacattatcttttgcaatgccagttattttcttttccagtgtgggtttgcataggaaaagaattgctgtcactttctattttgaaatcttaaaagactgatccttttttgtgtcatgatttgagtatttaattgagagcctaatgcctaatattatttgcagtattaaatgggatcttaacaggaatagcattctagccttcattgaattaagtaaacatttcttaagagaacttggaatctataatatttgcgtcatcatagtatgagatacttaatcaagtttgagattttagtgaaacattgtttagaagccaaaaggattctaggaaaaattaatgtctatattcttgaattaggagagattttgggacgtgtgactaagttacgctgacacttgtttgtttcttagtcgctttttccagtggcggtgagaacgaagatgactgattcacattgctcagatgagtttatcctcttctggctgggacatgggatatatcctgtctcttttaagcctttttggtatttttcccccattgagagctgtgtcttcaaactcttctgttatagctggaaaatcctttttaagtgaaatctgcccaaattataagacagatgaaggtagagttgtgttggatataggattagggtgaaagtagtgggggtgtcctggagcctctcttctggtggcagcctagctcttgtgcctttgaggaaattaccctggggacggctctgtggaacatatttgcaaaccactgatttggaagatagagatggcttttgttaagatctgaattcacctttttggcattttatttgatttctcaaggtaaagaacttattttgtaataaagtttcctattatttagtagataggccaagttgctgtgttaattccatgtagattttgggtttcctttgctcattttttcactcttaatctcacatcattgtaagtttatggaagttatcatacttctgactttttctttgaagagcagaaattagaaattcccaataattattttgatagtgtcatttaatgacactcacatgtgatgtagccacaaagatttaatgagttcagttttaaatcatattaagactgttggtttcatttgttctcattaatgtaattctgaagatgaacaataaaatgtatttttagaactttcaaatgaaatattatttcatccttccagatcatataatgcttaagttctgattgttaatcataaagtctagaaaattaaaagataataaaatgaaagtgacttttaggtattagagttttattataaattctggtgtgtcattggagctatgacatgaatatttcaaaggccaatagcattggatctttacagttataacttaccatttttaagtttaagtagtaatatagattatttaataatcaaaatcaataaatattaattattaaaatgttttgtggtatagtttgagaatcattgcttttaactttttccatataggtttattgactttaatagcattctaaacataacatctctacattctttgtgtttaatactgtggaggtataaaaatacttatatatgatgataaactatattagagtaaattaaatattcttatgagtttcattttagagtgcatttacttaattttgaagtccttatttttagcaaactaaaaggaatgttggtacattatttactaggcaaagtgctcttaggagaagaagaagccttggaggatgactctgaatcgagatcggatgtcagcagctctgccttaacaggtagttctcactagttagccgctggtgtggaccttcactgtctgccttccaccccttgcccttcctgctcgtccccctgcacctggtggacagcacgactgggggcagcagtggagccaggttgcttaaatggggcatattcgggcttcttttataatacttactctgaagcttgtgtgtctgtggtgtttgcatcatatatttgttgttttccatggtttaggctgttttaaaattaggtttatggcttgagcatagggctttgtgagtaggggatggcaggtcgaaacatctcatgagttggatgggttatgctgggggttgggaaatgggatgaaaaattatgggatgaaaaattgcctatggatagtttaacttgaaagaatctgcctttgtttacagatagttatcttttttcttttttgagatagagtctcacactgtcacccagtgcagatacccagtgtcactggagtgcagtggtgtgctcttggtgcactgcagcctccgccttctgggttccagcgattctcctgcctcagcctcccaagtagctgggactacaggtgcccgccaccacgcttggctaatttttgtatttttttgtggagacgggtttttgccatgttggtcaggctggtcttgaactcctgacctcaagtgatctgcctgcctcagcctcccacagtgccgggattacaggagtgagccactgtgcccggccagttacagatacttatctaatgaaattctctgtgtactttataaaagatgaggattaactgaaggtactaataactggattatatgagggtggttttggttgtataatcctatctaaaagaatattttagctataactgaaagtaagacttaaatatttagagaggaaaatctgaataattctagtagtaattatttatttacaaaataaaaatagatttttttttgattacacaaattaaacaacaataaaacatcacagcaatccggatactataaagctcacatgcttaccgacccaactgccccaggagtgaccactgccaacagcttcatgtcgacctttttgccataatttttatatagccttttttgtttttaaatggtaatttagaaagtcaactaggaaaatgtgttacaggtttatcttccaggagaataggactggagtcgagatcttgaatgtggcttggaagaaggcaagcccaccccagagagatgagttgacagttgtttctgaccactgcttgcttagagggcctgcgtgtctgtgaccgcctagctttgcgcccctgactaggctgccccttaattacaaatgtctttatatattgctccagctaaggcttggagtagtcggttaagaacttgaacttcggtttttgcagtgaaacagcatttgagaatatcaccttctgataagccttattttataaggtgggtactgtagtgggaggcagtgtgagagatgcttgaaggatgcactgctgtcctgcatttcagcatcttcaggatgctgtgcagctgaaacatttgataacggtggaactgttcgttattttgcaagcctgtgattccctattgaatgttttctctcgccatttgacaaatgagtgtttctctgtcttcagcctcagtgaaggatgagatcagtggagagctggctgcttcttcaggggtttccactccagggtcagcaggtcatgacatcatcacagaacagccacggtcacagcacacactgcaggcggactcagtggatctggccagctgtgacttgacaagctctgccactgatggggatgaggaggatatcttgagccacagctccagccaggtcagcgccgtcccatctgaccctgccatggacctgaatgatgggacccaggcctcgtcgcccatcagcgacagctcccagaccaccaccgaagggcctgattcagctgttaccccttcagacagttctgaaattgtaagtgggcagaggggcctgacatctttttttttattttttatttgagacagagtctcactccatagtgcagtggaggccgggcacaggggctcatgcctgtaatcccagcactttgggagactgaggcaggcggatcacttgaggtcaggagttcgagaccagcctggccaacatggtgaaaccctgtctctactaaaaatacaaaaattagttgggcgtggtggcacatgtctgtagtcccagctgttagggaggctgaggcaggagaattgcttgagcctgggaggcagaggttgcaatgagccgagatcgtgacactgcactccagcccgggcaacagagcaagactccatttcaaaaaaaataaaaaaataaagtgcagtggctcgttctcagcccactgcaacttctgcctcccaggctcgagcgattctcccgcctcagcctcctgagtaggtgggattacaggtgggcaccaccacactcagctaatgtttgtattttcagtagagacagggtttcaccatgttggccaggctggtctcaaactcctgaccttagatgatccacccaccttggcctcctaaagtattgggattatagttgtgagccaccatgcccggccctgccacctgccatcttttgagttcttccctggagacctagacctgaaccctcctgcttgttctcttgttatctaatacccctattgacagcgcagcttagatcattaatggagagcttgacctcatctgataccttcactgaaggaaacaacttagtgtcttttgtgttgaacactgaggtaaaaaattggaatagttgattatatgaactctgctaaaattgagtgcattttacattttttaaggccttgttgggccctggttaaataattatttttaaaaatccttaaggagcctattataaacagatctgtggtcttaatgaaatgtgattaatactgtgcattattttaagaacttttgacttttcaaaaaacttttacaacatttcccatttgatagcggcataggtttaagcacttctcatctctaagttagtggacaaaaaaccctcatggatagtctaataatgtttgctacaagtccatgttgagttttatactccattttattttcagttttaaaaactgtggttaaatatgtgtaacataaaatttatgttcttaaccattttttgcgtatacagttcgctggtattaaatacatttaaataatgtcatggaatcattgctaccacccatctctgtaaccttttgatcatgtaacactgaagctctgttcccattgaactctattcctcctttcccgccaagtccctggcaaccacgattcttctttctgtcttctgaatttgactactttgggttctcatatactttaggagtcacacagtatttgttttacttagcataatgtccccaaagctcatgcatgttgtagcctatgttagaacttcctaatgtttcaggccaaatactattccattgtatggataggccacattttgcttttccattcctctgtccatggacacttgtattgcttcatgttttagccattgtgaatcatgctgttatgaacgtgggtgtacagatagctcctggagactctgctttccatttttttggctaaatacccagaaatggagttgcttttacattccaattttaatttaaaacattcatatcattgagtgttttacttaatagtatagtagttaacaaacttaataaaatagtattttggtaataatttgctggtagtccattgttcagtttttttaggtaaattacacaggacatttcaagtggacatgaaacatcttgtgatgtggaatcatgccccaagctgatggctaaacatatgaaataccataccctaaatttagtagatttagtctttgcaatttaggagataacctgttatattgttaggtttttgtcgaaaagctttgtcctcatatttccaacttgctgtaaaatttgtttgtgaagacaaatatttttgtatgggttttttctttttcatattaaaaagaaatgtccacattggaatttttttggagtttttagagctaatagagcttttcataatgtagtgggaatgagtgatcagtaagctcttagcagtttccatgcgtgcatttctgtgccttgaaataaatgacagatgagtacatttgtgttctgtgtgtaaaatgtgctctttcctcattgcacttccatgttggagggcttgtctcttggtgatcacacttcaaaattctcacagccccccttgaaccgtttaggtgttagacggtaccgacaaccagtatttgggcctgcagattggacagccccaggatgaagatgaggaagccacaggtattcttcctgatgaagcctcggaggccttcaggaactcttccatgggtatgtggactacaggtgatgcgctacaaagtggtttgtattcagacctggacatcttaattatatctttgcttccaagaagaagtcctttgatactgttttctgagttctgaatagctgatgaaaatgaccaattgaggaataatcatactttttcttgatctaaatcttatacttttgagttatcttagcataaatgtataattgtattttaagtggaaatttgtcacttaatcttgatttctctgtttttaaagcccttcaacaggcacatttattgaaaaacatgagtcactgcaggcagccttctgacagcagtgttgataaatttgtgttgagagatgaagctactgaaccgggtgatcaagaaaacaaggtgagggacataggcttgagacgacttggtgtttctgagcttgtgtgaggatttaaaatcgccctggctactgtctactttattgctttcccatccctgggcctttaaatttcccctttaaataccagctcttcccaggcctgttgttttctgcctttccaggtactacccacagccttgagaattgcctgagttctgcctcctttgagagtgtgccccagacaaatctattctgtactgaatgtttccttgtctgatttcttggatcattcatttgatggttgcgtatggcctgcaacgtttcttgttttggttctactgaactgttctaaaagtctctcttcatattatctttttacatgtaaatgtaactgtcttcacttttaattcctcaaggacaaggaatagcgtttcacagttcgtcccatcaatcagaattatagcctttggcatctccctatctaccaggcccacttcctcttagatttgggcttccccaggctgttgcctttccccaagtagcttctgcttgtcctgtagaagacctttcatgctttgcttctgcagcagccgttcctgaatgcctagtgtcaactgccttcttaccacgcccaccctccctgcatgctgcatttatcccctgccacagccctgtgaccctgtgtcctgctgcctctgacttgtctgtttctgcttggccatggtctctgtgaggtcaggtgtgcatatgggcacaaaccagggcatctctttatccccagcacctggcttaagtgctgctctggaactatctgttgaatgaactaatgcatgaatgtattgttgagtatgagacaaacaagtgtcattgtctcctttctagccttgccgcatcaaaggtgacattggacagtccactgatgatgactctgcacctcttgtccattgtgtccgccttttatctgcttcgtttttgctaacagggggaaaaaatggtgagtacaaaaggggatgtgcacagttgaaggaaataactaggtttcagaggtcagcttggtggcctgtttttgccttgcgtgcagcagaggaagtagaatctgaggatgagtttggttttcactagccgaggggagggaggaaatgatgggagcaggtaggttattgggtctggttttgttcatttgaaaacaatctgttgtttgaggctgaaggtggcttgggtgatttcttggcagtgctggttccggacagggatgtgagggtcagcgtgaaggccctggccctcagctgtgtgggagcagctgtggccctccacccggaatctttcttcagcaaactctataaagttcctcttgacaccacggaataccctggtatgttaaaagttcacatcttattttctcagatttaatcattattgtaaaaactatttcagtattgactattttagttttagagcagtaagtgttttgagttcatttgggatatttgacctgcgttgtagctcttcagaaaacacatgaatagtgaagttctttgtttcatgggttccctttagatgaaacccatagaggagaaaagtagaaacctcagcacgtaagagccaacatatatacacatcggatttaaacctaaagcacaaattgtgcctggtcgcagtggcgctgagtcgcactcagccaggccaggcattcacactcagggtgagtgggaaccaggactggctgaggcagcagtggacccaagtctccatcgcgcccatgcttactatggagccttctcgttctctctttttctttgggtgagagggtacacttgtgtttttgaatttatatgaggtaagtgtgtaatagggttttttctaatcttttttaagtggaatctggaattttaatcagatttattatctgacaacctagaattataatccagaaagtctgtggtattgaggacatattggcaatatgatgaatctctaattcttaaatcctgaaacttttttttttttaatcacttagggttattatagtgaagtcatttctgaatttggatcttctcttcacacctctttttctctttcctgagaattaagcttttgtttcgagttagaaagttgatagtagggaattgttccatggctgagcaatttatctccacagaggaacagtatgtctcagacatcttgaactacatcgatcatggagacccacaggttcgaggagccactgccattctctgtgggaccctcatctgctccatcctcagcaggtcccgcttccacgtgggagattggatgggcaccattagaaccctcacaggtaacggccagtttttcagctgtgttttttctagttatgcttactaaggtttaagtttagatgatgatgtttgttgcttgttcttctggttaggaaatacattttctttggcggattgcattcctttgctgcggaaaacactgaaggatgagtcttctgttacttgcaagttagcttgtacagctgtgagggtgagcataatcttctgtggaaccatttcttcacttagtggacattttatcattgctacaattaaaattggagcttaataggaaatatttccatgcactctaaagctgtaaccagtaatacccaccatgtatccatctctcagctttagaaagaaaacgttgccagtaaagttaatgcttcataaacttcagtttaagttctaattctcagaatatttgtttgaaatagacctcttcctaaaggatatatttagaaataacctatcattaagtgtaaagtctgttgaatatgctgggcacggtgactcacacctgtaatctgaccactttgggaggccaaggtggaaggattgcttgagcccaggagttcaagactatgggcaacatagttgaccctgtccctacagaaaattaaaaaaaaaaaaaaaaaaagtagctgggtatggtggtgcatacctgtagtctcagctactcgggaagctgaggtggaggggggattgcttgagccccagagatcaaggctgcagtaaggcgtggttacaccactgccctctagcctgggcaacagagtgagactgtctcaaaaataatagtaataataatcagttgaattaaaaaaaaaaaaaaaaaaaccactgtgctaggcccatagtatggtaagagttaaagtgagccttagggattatttactcaacctctgtttctgtataaagtggaataggctcaattctttaagtgatagcatgttgaacctttccataccaactggctcataagtcacaactggccagtcaacaagagtaaaaattaactggtaaaaatcaaagcaaaaaacctacaattgtcaaatttgtgggataactcccccttttaaaatgtcatgcctgacagtaatttctctctagtttccaggttttcagtcagttgtgtcttttttgagcagaaggaagcatgctaagagctcaatcttgtggctagctgggggtctttgtgtcagccatgcatgtgatggtgcccctgggtgcttggggctgcaggggaggggtacagcagtaggggcctgttctgttctctcgtgctgtggagtacatagtgacatagtggggtggtccttggtgtaggtcccttgttcctacccctgggtctgagatttatttagaagtggtgttggggctgtgcggcaggcccctctgtaactgatcaatgtttgtgaagttgctgtttgagagttgaaaccatgacataagcagaaatggaaggaagaaagaaccagttatgtgaaagggacacatttacttttaagcttgtatttactgagataaagtattcttaatcaatgttcttgagaggtgtgggaaaaatgcaacatcctggttgcagttaaacccagaacattgtgtgttgaagagtgacggttctcaaaccgtcaagacgcgggtactgagtgggactaacctgctgtcctcttgccttggaccttgtgttccagaactgtgtcatgagtctctgcagcagcagctacagtgagttaggactgcagctgatcatcgatgtgctgactctgaggaacagttcctattggctggtgaggacagagcttctggaaacccttgcagagattgacttcaggtaagtgagtcacatccattagatttcatgaactaagctcaattgaaagttctgggatcacttgatgcaaggaatgatgttatcaagtaccctgtccatcagaaatccgagtggtttaggtagatgacagtgattttctcctcccagtggctttttgctgaactttgccctatgcttggaattttattttattttattatttatttagagacaagatcttgctctgtcgcccaggcttgaatgcagtagcacaatcatagctcactgaagctttgaactctaggactcaagtggtcctcctgcctcagcctcccgattagctaggagaataggtgtgtgccgtcacactggctaatattttttgtagaaatggggtcttgctatgttgcccaggctggtctcaaactcctgggcttgattgatcctccatcttggcctcccaaagtgctgggattacaggcatgagccactgtgcctggcctagaattttaaaatataagtagaagagtagatttttttttttggtagtcctcgtcatttaagtattctggatagtgggaataaaagagcttagaatttttcatctttgtcttaaacttttaaaaaaatgtagcttatattaattctgcttgtttaaaaagaatatactcttcattatactgaacctaggtaagacagctggtttatattttgttgcaattaaaaaacgtgagctgtggttgcagtgagccaagattgtggccattgcacttcagcctggcaacagagtgagacttggcctcaaaaaaaaaaaaataacatgagctgtgttggcactttcattttctaagagtagttttggctggagaagttttctttcagtactttcttttagaagggaaattttcctttataatttagggtttgttttttttttttccaagccaccttttatagagcccttgtgggttatttcatttaatccttagaatgtttataaatctgggcttgttctcggctccacccacagatagggacgctgagcgtgcatgagtgggcagcaagatagcaggttatggagggcccagctcaccccttctgtggcttgagccaattttatagggcacttacagagtcttttgaaatagtatttattttgaagaaaaagaaaaacagtttactgagtactgtcttattgagtctggaattgtgagaggaatgccacctctatttatttaaagccattggccttttttgttgttttgagtaagtgctgcccaaggtccttccagggcacctggatgagcctgctctggagcaagctggcggtaagtgtttactgagtaactaaatgatttcattgttaaatgtgctcttttgttaggctggtgagctttttggaggcaaaagcagaaaacttacacagaggggctcatcattatacaggggtaagcggtttatttttgtgagatgctgttttaccttcaagaaggtgaaagtgaggctttccttgtggaatttctctaaatgcattcgtcatgttttagatgtttatttcacagtttatatcatgaaagttataatcttgtcatatggatttaagtctagtaatgttgagttctttctcactagctttccaaaatatcttacctaaaatttagtcaaatacaagattatgtttatttttattatccttctctctaaagcttttaaaactgcaagaacgagtgctcaataatgttgtcatccatttgcttggagatgaagaccccagggtgcgacatgttgccgcagcatcactaattaggtatttaccaatattttatctcttttccttttttggttgaagtactaaaagatacgagaatggaaagagagggaagaattcaaaggatgtagagcagtattcctgaatctgagctcatttcagccattctattcttaaactataatgaaaaaaaaatccaaaaaagtctaaaattataattaaaaaaacaacaaaatactaactgtccattgtaaaaagtaatgcactttcattgtaaaaattttggactatagagaatagtactaagaagaaaaaaaaaatcaccttcaattctgctgccacctggaggtaatcactgttaatattttgctatatactctatgagtttcttgttcaaaatcaggtcaaaattacatgcaattttgtaatctgacaatttccacttaatattttattagcattttcctgttatgaaacagtaattttagttatgggtcgttgttttgctatgcggttgggataaaattttatatactttttttggcaattacttattatacataaatgtttgtgtatagttttctttttctgagaattcctggaagttgagttaccaggcccggctttgaatttttttttttattttttttttgagacagagtcctgctctattgtccaggtgctatctcggctcactgcaacctctgtctccctggttcaagcgattctcctgcctcagcctcccgagtagctgggattacaggggcacaccaccacgcccaattaatttttgtatttttagtagagacagggtttcacgatattggccaggctggtctcgaacttctgaccccgtgatccacctgcattggcctcccaaagtgctgggattacaggcgtgagccatggcgcctggccaggctttaaatttaaaacaaatcttctaatagctttatggaggttataatttacatttcttgaaatgtactcactttgagtgtatagtaaactccaattttatcacatttctgtcaccccaaatgtatccttgtgcccatttgctgtaacctccggttcctgccccaactcctaggcagccactcatctattttctgtcccttaagatttgtgttttcgccaggcgctcatgcctgtaatcccagcactttgggaggccgaggttggtggatcacttgaggtcaggagttcgagaccagcctggccaacatggtgaaaccttgtctctactaaaaatacaaaaattagtcggatgtggtggcacacgcctgtaatcccagctactcgggaggctgaggcaggagaatcacttgaacctgggaggcggaggttgcagtgagcagagatcgcgccactgccttccaacctgggcaacagagagagactgtctcaaaacaaacaaagatttgtattttctggacattttatagtactggggtcatagtatagatggacttttgcatttggcttcttttacttaattgtgagattggttcttgttgtagcatgtatcagtagtttgttcatttttattggcgaaagtattctattatatgaataataccatattttatctatccatcagatggatattatagagttcatgttttggctaatttatgaattatggtactgtgaacatttgcctgcaagattttgtgtagacatgtcttcatttctcttgagtagatcacctagaagtggatttttaaataattttggtacttactgtgaaactgctcttcaaaaacataccattgttccttccttccttccttccttccttccttccttctttccttcctcccttcctccctcccttccctacttccctctccctttccctttcccttccccttttcccttccccttcccgcctgcctgcctgcctgccttccttccttccttccttcgtttctttctacatatacacatttttttaaatttcaatggtttttggggtacaagtggtttttggttacatggctgaattttggttacatggtgaagtctgagattttagtacacctgtcacccgagtagtgtaccttgtacccaatatgtagttttttgtccctcaccttccagccttccgccttgtgagtctccaatgtccattataccacactgtatgcccttgcgtacccacagctcagctcccacttctgagaacatatagcagaaacatgccaaagtatactcccactaccagaatgtgattgtgcctgattcttctcaccagtacaaatatttcaaaaaaagttaaatatgtatcagttttttgggcagaagttgatacttctctttatttatttattttttttgagatagggtctcattctatgatgcccaggctggagtgtggtggtgcgatctcggctcactgcagtctctgcctcccaggttcaagtgattcccacgtcagcctcccaggaagctggaattacaggcgagggccaccactgccagctaatttttgtattttttggtagagatggggtttcaccatgttggccagactggtctcaagctcctgacctcaagtgatccacctgccttggccttccaaagtgctgggattacaggcgtgagctaccacacccggctgatatttctttttaaaataacttaccttcttttgaaagtaatacatgtttaatgaacagaatttaaggaaaatataaaaaaacgaaataatctttgtaatcaaactactgaaaagaaaaccaaagttacattttggtgcatattctttttcattttcatcattgtaatttgcatttctttgattacttgtgagacactcctttcatttacttaataggtttatatgacttgcctattcagagattttgcagctttaccattttctgcaaatgatagcaacttctttttgtttgtttgtttgtggagacagagtctcgctctgtcactcaggcaggaatgcagtggtggaatcttggctcattgcaactattgcctcctgggttcaagcgattttcctgcctcagcctcccaagtagctgggattacaggagtgtgccaccatgcccggctaatttttgtatctttagtagagatggggttttgccatgttggccgggctgatcttgaactcctggcctcaagcggtccccctgtctcggcctcccaaagtgctgggattacaggcgtgagccaccgtacccagccagtagttacttcttatattctagaaaaaattctactcatgatcaagtctccatgaggaaagagactttaattgaagatcatggggcttgcagaccaatatgataaaatagttcattgtttctaaaagtattactgagtgttgatggcagatatgaacccttttgtttttgtaggaaaatgttacccgtattctccatttgaattcagtttagatttgttaggaatcgcagcttaagctttgccatctgggagtgtttgggacagttttgcagacaaaattgcaaaagtgcctaaggaatgcagctggcattcagacctgctctgtgctcagtactctgtggacagacactgttcagcacttgttgatcagaaggtttagaaagagaactttcaaagttggtttttaattaaagcatttaatagtgtaaatagaaagggattaaattttatgacagacaaaagaaagtacagcacccagctgggcgtgggggctcacgcctgtaatccagcactatggggggctgaggtgggtggatcacgaggtcaggagttcaagagttcaagaacagcctggccaaggtgatgaaaccctgtctctactaaaactacaaaaattagccgggcgcggtggcaggcgcctgtaatcccagctactcaggaggctgaggcaggagaatcacttgaacctggacggcagaggttgcagtgagccaagattgcaccattgtactccggcctgggccacagagtgacattctgtctcaaaaaaaaaaaaaaaagaaaaaaagaaagtacagcacccagttatgtccgagtgggtgcatgagagtgaccctgagattggagacaacgctgtcacgtgcttgaagaacgccacctgagaaagggggcgagaagtggtgtccgctggtaaccagaggtgttggcttagccatctgcagggaggagggtggtctatcacaggtgagtttcatctactttcttaagcaaattaaccttacttttgtgttaggcttgtcccaaagctgttttataaatgtgaccaaggacaagctgatccagtagtggccgtggcaagagatcaaagcagtgtttacctgaaacttctcatgcatgagacgcagcctccatctcatttctccgtcagcacaataaccaggtatgctgacccagtggcatcttcacattgtcgggaaaatgccctttcctgatgcctttctttaggctttaattgaaaacattttattttctagaaaaaagcttcagctcaggatgtttgagtgtaggtcagtcctttgataggatattatcattttgaggattgaccacaccacctctgtatttaagctctgccacaatcactcagctgtgacactgtaaatctcttaatagtttattacattccatgtgctgacagttgtatttttgtttgtgacacttacgtattatctgttaaaacattttcactttagttgtgttacctttaaagaggattgtattctatcatgcctgttgattttttggtgagcgggctattaaagtcagtgttatttagggttatccactagttcagtgatttgcgagattatcattcacatttattgtggagcttttgaatatcgtgtcaaatggccacatatatcccattcttatctgcttcttaggtgagtgggacacagtgctttaatgaagctataatcttcagaattctagcttgcagagaagattgcagaagtgataagacttgtgctttttaattttgtcttttaaatgttattttaaaaattggctttatatgatactctttttttctgctgagtaacagtgttttacaaaacttggactaaatgacttctaagcttaaatgatcacttgatgctttttttctgaattaggaactcagcttatcaaatatcaaagtcataattcctgaataaataacgtcttttttcatgtaaagactgctttaaaaaacacatggaaggctgggtgcggtggctcacgcctgtaatcctaacactttgggaggcccaggtgggcaggtcgcttgagctcaggggttcaagaccacccagggcaacatggcaaaacccacctctactcaaatacaaaaaattagccaggcgtggtggcgggcccctgtaatcccagctactcgggaggctgagggatgagaatcacttgagccccggaggcagaggttgcagtgagccaagattgtgccattgcactcccagcttgggctacagagtgagactctgtctcaaaaaaagacacacacacaaacaaaaaaaacatggagacatttttttggccaccttaatatttcccctcagataatttcctttgtttaaactcagaactggcattttctctcttggagaagattcaggacaaatactcctttaagataagtagaagcagtgaaagaggatttgattatcaggaatttgataagcttagaataaattgttgcttcttaatgtcatttcagaagatgaatatttattaatagatgccaactgagatatcattaaaattgattactaactactacttggaaaagtctcccagttccaaacttcagcaggcctcttgacaattcagctgtggtcaattgggtcttgcgtgatagatacaatgaccaattgtgcagcagagtgtgctgcttagctgcctattctgttagcattcatgtgttaacttaaaatcataatctccttagttttgttgagtgtctccgtggacaagacactgtgagggatacaaaatcagattggctttattcaaaccactggggtattataattcatttataatttattttattttttgccttttttccatgtgttctaaaggaattagagtttgtatataactataatgggggatagaaattgacatgtgccatgaagggaatgcaaaaaagtgccgtgggagatgagaagtggagaaaggaatttcttttttcttggaagcaggaataacttcatgaagcatgtatttcaacttaaacagatagtaggcaacgctgtaaggggagtatggctgcagcaaaagtgttcggggcagactgggaggaagggagggaataaattcagccattgttatggaataatgatcaaaatttattttcagcccgtttcacttaaaagttgagactgcttaactttttttaatctttaatcttaaacttttaaatgccatttgatctttaaaaatatatgttttaatagtgtattttaagtctctatatttttgttattagaatatatagaggctataacctactaccaagcataacagacgtcactatggaaaataacctttcaagagttattgcagcagtttctcatgaactaatcacatcaaccaccagagcactcacagtaagtctctttcttgatcggtcttactgacattgtaatagtttttggtagcttgtatggccagttagttgtatggtcatcttacggtgaggtgcttgtcttacagctcttacttatccatgaggcttgctaagaaattgtgcttctgtgaaaagaatctcagcttactccaggaatgtaaatgactatgttttttctgattattaaagtaatacacgcccaaaataaaaaaattcagccaatttaggaagacacaacaattaaaataagccaggcatggtggctcatgcctgtaatcccagcactttgggaggccaaggttgggggctcacttgaggtcaggagtcggataccagcctggccaacgtggtgaaaccccatctctactaaaaatacaaaaattagctgggcgtggtggcgggcgcctgtaatcccagctactcaggaggctgaggcaggagaatcgcttgaacctgggaggtagaggttgcagtgagctgaggtcaagccactgcactccagcctgtgcaatagagcgagactctgtctcaaaaaaaaaaaaaaaaaaagaaaagaaaaaagtaaactactgtcacctgcattggtaatgtatcagaagtttaaaatgtctagattataattaactcagtgacctggtaatatatactaagggaaaaatatttataatttacatttttacatttttatttttttaattttattattttttttttgagacagagttttgctcttgttgcccaggctggagtgcaatggcatgatctcagctcaccacaacctccacctcccgggttcaagcaattctcctgcctcagcctcctgagtagctgggattacaggcatgcaccaccatgcccggctaattttgtatttttagtagagacagggtttctccatgttggtcaggctggtctcaaactcccaacctcaggtgatccgccctcctcgaccccccaaagtgctgggattacaggtgtgagccaccatgcctggccttacatttttataataagaatttatgttgctgacattagaaaagaaccataatatccaagaatccaagaataattaaattatgtacatatgctagtatatagtgtgatgctttggagaatttttaacaatatggagatgtataatctggattgtaatattgagtgaaaaaaggcagaatacaaacctggtgggggtatagtcggatttcagttaagaaaaataatatttacatatatacatttctcacactggcagataatcaccaagataaattttgggattgtggatgatttttttcttctttatatttttcagatattctcaaattttctaaaatgagcaagtataacttttgttatcagaaaaaaataatatacaaaagtaatgttaatttgctggtgaccaggttaaacctttttatttttattttttgagatggaatctcactctgttgcccaggctagagcacagtggcatgatcttggctcactgcagcctccgcttcctgggttcaaatgattctctggccccagcctcctgagtggctggaattacaggcgtgtggcaccacacctggctaatttttgtatttttagtagaggtagggtttcaccaggttggtcaggctggtctcgaactcctgacctcgtgatccacccacctcggcctcccaaagtgctgggattacaggcgtgagctactgcgcccagccagacctttttattttatttgacaaaagaaatacttccatgttatagaagactaaatattgtttgggctgtctgcagtatggtcttcccttgatttgttcaaaatatcgtaaactttgcttatttatttttattgtggccgactgtgtcgggcactgttgtaggcttgggatggaaaaacaggattcctgcccttagggtttctgcaggctggtcagggagacgatgtggtaagctggagctcagctcctaaggatgtgcaggggcagttgagaggcggaagggtgggagatcattccagggtgtgggcagcacaggaacctctcttcattgggatataattgccattctgataacacgtgtttgaggtgtctaaagtaggaagttgtaccatggtgggacagatatcctgtggttatcatacacagatctcagttttcttctcattgtttgtactttttataaagggtaacaggagatataattcaataaacctttgtggtgtttgggtgtgattttattgtttctttcttctcagtttggatgctgtgaagctttgtgtcttctttccactgccttcccagtttgcatttggagtttaggttggcactgtgggtatgtattttcctcagtatatattaatagttgtctacaacagtatgacataaacatagttattaggatgccctttttctttctttttaagtcttttatcaatttggctttttggaaaaatatctgatggaatacttgtttctgctatattagctgtgtgagactagtgacaggagctgtgggaaatgaatgccaaatgttcttaggcattgatgggaatttcagggtgtggtcttcaagttcatttaagggaattttcatatgctggcaaaaggcttttctcattagcttgactctttccaaaattatttgctgtgaattagaagtttaggaaccttttttcacttaattgtgacctagcatacgaaatggtgatgatttaggaactactgttcttgtattaacagcttttatttaaaaatgattttcctccagtagatggccctactagcatctgggaaataatttcaagtcttctccagcattcaggaataggctttcattttgtgtatcaattactgagaatgattttggtgactcacatcacatttgagaagtaaacctgcagatttcttgtgtgtgtcagcaaatgaccaactgatatttgcttgaagtggattacattatctgctctagaatgattgctttcccaccttcctcacatacagactgagcagctacggtttctaatcataggtctggcactagacttcacttctgggcaactttggcattggagtaaaatgtattaatttaaagaaagttaaaaatccgttcaagtaaacatacagttctaatactttttacaatttaaaatatagatttaaatgataaaataaaaaagaaaatatgggtagacaccataatcctcgtttctgcatctgttcacaaggggttgatatttatgagttctattctccatatccattctatgttctcttaatgctcagtcagcacctcaggtggttggagttcaatgcttggtagtttgacttacactgtcttttctaggggattgagccctgggtagtcctgcttatttgaggttgcaatttgtctttcaataacttttactacaagatatggcgtgttaaaggataccattggggaaccaacataataatatcaggaaaactaaccacgtcagacctgccccattgtgtatcaagtacactatttttccatagtaataaagagttcaccccagccaattctcttttattttgtgcctgtttactcaatggcattaacatgcccaaatgtctgggtagctgtctcatctccagttcagcagaaccattgtcatatgccctagtaaaagcattccttcattggacacttaggccccaatactttcattcagatctactacctgatttcatttctcaaatgatttttatggagctctgatttataggaaagatgttagttgattaaaaataaaacaatttctgagctggtataaaatgtattgtgacatgccttcctcttggaattgcaagagaaaggaagactgttgtttgcttaaaaattgtctataatttgactttgcaaatgtctgcttccagagtgcctccactgagtgcctcagatgagtctaggaagagctgtaccgttgggatggccacaatgattctgaccctgctctcgtcagcttggttcccattggatctctcagcccatcaagatgctttgattttggccggaaacttgcttgcaggtactggtactgagttgaaacagggactccaggacttggattttgatttccttagggggaatgggggtggtgagcatatgaggggaaaatactataaggtcattgccagtgatggcttgtccctttagtcaaatttcagatgttacctatatgcataaacacatgcagttggcagctgttctgtgctgagtattttaaagtagcctcttcccaatatagcccctcagttaactacaagtaaactcattttgaatttcattttaatgggcaccatatgccagtactccctcgggcactgggatgttaagaaagtataatgtatggacttcattctcaagttagttttagattagagggggatacacgtaaacaaaagtgcagtggtcacacagagtggccctaatcactctccttgggcagatttatgggctggtaggaaagagcacaacacggagagggtgtagcaccttggcgatgataatggaggatgtggccagcaaggaagacggagtccattgaaattgattttgggagaagttgccaatctccatgaaagaattggggcctgtgctatttgcttcagggggctataggagagtttcgtgaaagggactaaaagatgagtattttaataagatcattcatccaacttgaacatgggctggaggagaaggtagggagactcaggagattaatgttgatgctaaggcaagataatggctttgggactgtagggaagacactgattgtaagagaatgaaggaggcagaattgccaggcctggttcaccaactgaacttcggttgtgaagacaaagaaacctgggatgacttcacatcctgggcaggtgtgtggtggtgacagtcatggaaattgggaacacagatttgtgcgggaaacatcagtttcagtttgagtttggcttatcagttgaatatcaggcacagatgtctggccaactctcaacatagggtcttaaatgacttcagttccccaagcaatttgtccttcccatgctattggggtggagaggtaatgtctgtgcccatatcacagccagtgctcccaaatctctgagaagttcatgggcctctgaagaagaagccaacccagcagccaccaagcaagaggaggtctggccagccctgggggaccgggccctggtgcccatggtggagcagctcttctctcacctgctgaaggtgattaacatttgtgcccacgtcctggatgacgtggctcctggacccgcaataaaggtaatgtcccacttgggtgctggattcatacagccttaatgactatgggtttccagactacctttgtttagtaatctgtcccttctttattctctttttgctttaaatgaacaaaattgctcagattgtgacactaaatttaacatcaaaatgtgaccatgtggatgggtgcagtggctcgtgcctgttattccagcactttgggagactgaggcaagtggatcacttgaggccaagagttcgagaccagcctgggcaacatcacgaaaccccctctctactaaaaatacaaaaaattagatgggttgggccgggcgtggtggctcaagcctgtaatcccagcactttgggaggccgaggtgggcggatcacgaggtcaagagatcaagaccatcctggctaacacagtgaaaccccgtctctactaaaaatacaaaaaaattatctgagcatggtggcgggcgcctgtagtcccagctgctcgggaggctgaggcaggagaatggcgtgaatccgggaggcggagcttgcagtgagccgagatcgtgccactgcactccagcctgggtgacagagcgagactccgtctcaaaaaaaaaattagatgggcatggtggtgcgtgcctgtaatcccagctacttgggaggctgaggcaagagagttgcttgaacctgggaggcggagtttgcagtaagccttgattgtgccgctgcactccagcctgggtgacagagtcagactctttccaaaagaagaaaaaaatgtgaccatgtgttttatagctcttttagtatcatcagtcactgttatccctaagagggaaatacctagctttagttttaggtttccagcattagccaagaaagctcagaattgatgttcctggccaagtacctcattgctgtctccttaaatcttggttaatggctactgtcctggctagcatagttatggagcatttccatggttgtagaatgttctgccaatctcagggacagttttgcttttctgtgaagcaataaaatcaacttcaaaacaaatgttaactatttgtacaatggatttaagatagaccagttcacatacttttttttttttttttttttgagatggagtttcattcttgttgcctgggctggagtgcaatggtgtgatctcagctcactgcaacttctgcctcctgggttcaaacgattcttctgcctcagcctctcgaggcagattacagctgggattacaggcatgcaccaccacacccagctaatttttttgtagttttagtagagacggggtttcaccatgttggtcaggttggtctcaaactcctgacctgaagtgatctatccgcttcggcctcccaaagtgttgggattacgggcatgagccaccacgcccagcctaagatagaccagttcacttactgtttatatctgattactctctctttgccttgtcttctacctttaaaaatctccctactaacttcccattctcctttagctgccatcagtcttctcccttctctgcaaacatctctggagagtcccagcctcagcccacagagcttcccactgctctgaggtggaccttgtttgcaaggcttctttggctctcttggcctggaccctgtctactacttcagccatccttccttaacccctgctggtggtttctgttgccacactccatagcagcgtttcccgcccagatcatgtctttacatctctgggcactgctctggtcctgcctgcctttccctctttgtatcctgcaggctgctacccccatcttgagtgtcctcttcagttggctttcagagggcctcctgggtgttcccttacccacttgccactccccagtcactgggttcagtccttcctgcccaccagcacatgctttctaggctctgtcctaggccgtcttctctctttgtagtctctgggccagtgctgttctagagagtggcagaattttctataaccatggcagtgctccatagctatgccaggcaagacagtagccactaaacacatatagctgttgagcccttgaaatgcagctagtgtgactgaagaactgaaccccgattcggtttaattttcattaaatttaaatttaaataaccttatgtgggtagtggctccagtattgggcagggcagcctgagagtcggggctgttctcctgtcttcagtgtctagatgagggacctcagaggacctgtctctggagctgcagttcaatgtagccagctgccccgtgacacttacatatagctgatttgtggatatgtcagacacggtgtgatgagctcagctttctgtcctcctccccacatctgcccctgccccatttaccccactttgtgtcttatcaagctagaaacaggtcaccacaagtcttcatttccactcaccaagtcttttgtttcccctactaaatattttgcgagaagaaagtgtgtacctttgtattcacatacatgtacatgcacatatacatgcacatatgcaggggtccccaacctctgttaaaaaccggactgcaggccgtgcgtggtggctcacgcctgtaattccagaactttgggaggccgagaccagtgcatcacaaggtcaggagatcgagaccattccggctcacacggtgaaaccccgtctctactaaaaatacaaaaaaaaattagccgggtgtggtggcgggcgcccatagtcccagctacctgggaggctgatgcaggagaacggcgtgaacctgggaggcggagcttgcagtgagccgagattgtgccattgcactccagcctgggcgacagagcgagactctgtctcaaaaacaaaacaaaacaaaaaaaaaaaaaaccaggctgcacaggaagaagtgagcaagcattaccatctgagctctatctcctctcaggccagtggtggcattagattctcataggagcgtgtatgagttcgttctcacacttctgtaaagacatacctgagacatataaagaaaagaggtttaattggctcacagttctgcaggctgtacaggcttctgtttctgggaaggcctcaggaaacttgcagtcatggcagaaggtgaaggggaagtaggcacatcttcacatggcccacaggaaaaagagagaaggagagagagagagagacagagagagagagagaaaaagaaagattgagagggagagaggagggagaaaggagagtgcctgtagggggagttgctacacaaaggagcaccagggggatggtgctcaaccattagaaactacccccatgatccaatcacctcccaccaggccccacctccgacactggagattacaattcagcatgagatttgggtggggacacagagccaaaccatatcagagcatgaaccctattgtgaactgcacatttgagggatctaggttgcatgctccttatgagaatctaatgcctgatgatgatttgaggtggaacagtttcatcccgaaaccatcccccgccaaccctggtttgtggaaaaattgtcttccacagaaccggtccctggtgccaaaaagtttggggacctctgcacatatgcatgcacctgtacatggacacataatacatgtacatatgcatactttatattctctgccacttctggtccagactgatatactatctcatttggattactgcactagccttttgttttggaaacagcattttttaaaaaatttaatttaatttttttgagatagggtgtcattctgttgcccagcttggagtgcagtgtcatgatcatagctcactgcggcctcgatctcccaggctcaagtgatccttctgcctcagccttctcagtagttgggactacaggcatacccaccatgcccagctaattttttgatttttttttttttttgagacagagtctcagcctgtcgcccaggctggagtgggttggcgcgatctcagctcactgcaacttctgcctcccaggttcaagtgattctcctgcctcagcctcccgagtagttgggattacaggcgcctgccaccacacccagctaactttttgtatttttagtagagacggggtttcaccatgttggccaggctggtctcgaacttgtgacctcgtgattagcccgcctcggcctcccaaagtgctgggattacaggcgtgagctaccgctcccagccaggaaacagcattcttgagataattcatataattcacccatttaaagtatataattcattctctttagtatgcccacagagttgtacagccatcaccagaatcagttttagaacccataaaggaactctgtactctttacccaaaacctccatgcctccagctgcaggcagccactaacctgccttctgtctctgtgactctacgtcttctggacattactgtggatgggctcatacagtcagtgagcttgtgactggtgccttctaccaagcagggttttcagtgtagcagcctctctgtttttcttttttttttaaattgtgacggaacttctgcctcccgggttcaagcgattctcctgcctcagcctcccgagtggctgggactacaggcccatgtcaccatgcctggctaattttttttttttttttttttagtagagatgggtttcaacatgttagccagggtggtctcgatctcctgacttcatgatccgcctgcctcggcctcccaaagtgctgggattacaggcgtgagccaccatgcccggctaacctttcatttactgtctgcatttcttccctgatgccttccagtccatgcacccgattgtagccattcatcctattatggtttaaggtgactgtcttagtcagcatgggttgccataacaaaataccatagcctgggtggcttcaacaacagaatttacttctcacacttctggaggttgggaagtccaagatccaggactttcgccttgccctcatgtggtgagggggtgaggaagctctgtggggcctcttatatatggatgctaatctcattcatgaggggtctgccctcatgacccagtcacctcccaaaggccccacctcctaataccatcaccctggtaattaagtttcagtgtataaatttgggggactatagacattgaaaccataacaagcacttttctaagatcagggagtgagtaagtagcagagctaggacctcaattccacatgtcagtcatcttgccttcactctgctccatgatggctgcctcctagagcattgggagtctcgatgttctatatgctctcatgtgttgtgtattggagatagttgaggctttatgaatacatctggatttgttgacttctagctttgctggtaaccagctgtgaccttgaataagttacttcatctctgagcctgtttcctcttttagaaacaggagtttaaaatgctgctttgggttgggcacggtggctcatgcctgtaattccagcactttgggaggctgagatgggaggatcactggagcttggagttcgagaccagcctgggcatcatagtgtgagatcctgtctcctcaagaaattaaaaaattagctgggtgatgtggcgtgtgcctgtggtcccatctactctggaggctgaggtgggaggattgcttgagcccaggaggttgaggctacaatgaaatatgattgcaccccatcctgggtgacgagtgagaccctgtctcaaaaaagaaaaaaaaaatgctgctttgtacccctttcatgtcatggcgtcatggccaacatagaatgccctggttgtttgctgttggagggcatgggcctgggggctccctgagggctccttccatcttcaactcattctctgtgcacctgttaggaagttgtgggccagtccctaccatgtatcattgtgtgggtaaaagtaaataaaatgtgtacagtgtctgaactgtacatatcagggtccaagaacaaaatgagtgacatgggttagctctttttaataaatggtaaaaccaaatattctaattttcagttttgttatacttccatcacatgtttttgtttttttgttttttgtttttgtttttctattttaggcagccttgccttctctaacaaaccccccttctctaagtcccatccgacgaaaggggaaggagaaagaaccaggagaacaagcatctgtaccgttgagtcccaagaaaggcagtgaggccagtgcaggtaggaaacagcgtggggaagggagggacatgagtgcagcatctgtcatgtagaaacataggatttaagtaacttggtgttttagagaaataaatataatacacatcagtaaagtgagagaaagtttctccaggtgcggttcaagatattagaaactaatgactgatgtacacagaccaccttttggtctgaagcatttctaagtgccactggctgacatgcagcccctacagcctccaggcttccagccctagcatggagcatcactctcctatgcttccctggttgcaggtgatggctggagaggcctcctgattttcagtaagggaagtggtgtagatgcttaggaatagatgtagtgagtgaaaaaactgattctgatatgtcaaaaattctgattggaaatggaatatttacatttggaagagctaaaggcgagagaaagtggggataaagtcatctgagttggaggagcttaaaccattcacaagtttggaggacctttttttacccatgaaaaggtcagaacagaaggggctaggatttaggtgtgactgcagtttattgaattcccatccatactgctctcggtgggcagtggcaggggcaggagaggagcctggcaaagcatgaagtgactgctgctgcctctgctatctgggacgcctggccacctgtctgtacagtctccctccagacccattctcacgctgtctcttggcacccaggggccagtgatggttctcccatttgttttgtgtatatagcatttatatcaaggctatttatttatttatttattttatttatttatttttttgagacagagtctcactctgtcacccaggctggagtgcagtggtgcaatctcggctcagtgcaagctctgcctcctgggttcaagcaattctcctgcctcagcctcctgagtagctgggactacaggtgtgcaccaccacacctggctaattttttgtattttttattagtggagacggggtttcaccttgttggccaggatggtcttgatctcctgacctcgtgatccgtccacctcagcctctcaaagtgctgggattacaggcatgagtcactgtacccggcctatttatttatttttaattgacaaaattgtatatatctgtaatatacaacatgatgtttgaaatatgtgtacattggccaggcgtggtggctcacacctgtaatcccagcactttgggaggctgaggtgggcggatcacgaggtcgggagttcaagaccaaactggccagcatggtgaaatcctgtctctactaaaaataccacaaaaaaaaaaaaaaaaaaaaaaagccgggcatggtggctcgcgccagtcgtcccagctacttgggaggctgaggcaggagaattgcttgaatctggcaggtggaggttgcagtgagctgagttcatgccactgcactctagcctgggcgatagagcgagactccgtctcaaaaaaaaaaaaaaaagaagaaatacatatgcattgtggaatggctaattaacctgtgcatcacctcacgtatcattgttttgtggtgagaacacttaaaatctactctttcagtgattttcttgcatatggtacattgctattaactgcagtcaccatgctatacagtagatctcttgaactcattcctcctgtctataaatgaaattttgtatccttgaccaacacattcaaggttttttttgagatggagtcttcttcacccaggctggagtaccatggcacgatctcatctcactgcaacctccgcctcccaggttcaagcaattctcctgcctcagcctcctgagtagctgggattacaggcacatgctactgcacctggctaatttttgtatttttagtagaagtggagtttcaccatgttggccaggctggtctcgaactcctgacctcaagtgatccgcctgccttggcctgccaaagtgctgggattacaggtgtgagccactgcacccggcctcaagcgttttaaaagatgctcttttctaaggattgactgtagtacaggaggaagattgacctgttgaaaagcctcagcctttacaagtgtaaaattatcagtatattactatcatctttctgatgaattaaataaactaaggactccaagtcaaaagtcttcaaactgaagtagaatagttgtatatagtgcttggcactttaatatttagtatcggtttaatgataatgtttgtgcctttgccgtctttaaaacatttttacatcatccctgtttgattacttggtgtgctcatgaagttgttggccactaaggaatcttaggctcagagaggttctggaattggccagtggtccttgaatcagctgctcctatgattctctaactgatttctcacaaagcaaacaagcaatcataacaaaacaactgtgcacactgctcttcttattttgttatttaaaaagtacttaggctctacttatgtttgttagtcaatttctcattacttctagttaatcaaaaggtcagaggaaatacttgaatattttcatactagaatactttaaaaaatcatgatttccagtaatctctttaaaacttggcaagttattttgatctaaaagtttatcttttgtgtgcatatttttaaagcttctagacaatctgatacctcaggtcctgttacaacaagtaaatcctcatcactggggagtttctatcatcttccttcatacctcaaactgcatgatgtcctgaaagctacacacgctaactacaaggtatgggcctctgcatcttttaaaaatatatatgcacacatacttacgtctaatggatagttgatgtttttcttatgatttgtaggatgtataagccctttgagatatgagttacatttagttttttcaagtttgtttgtctttcagctttgtttatgatagcttctatcatacaggtgttttggattttcatattgtttgtactcacagctaagattgattacagtgacagagctaggatgtgcagccaggttatagggggaagtggccctggtggagtctggagggatccgtgtacaggcttccttccctcccgtgaggctcacacaaaaatacagcaacatgctggtcctgcaggtaccctctgcctaacatgagccacaattccagactcacagaagaaaagcaggtgttcggcataaaccatgtgtttcaaatagtctgggcatggtgagccacttgttatcagctagggaaagtttatgtcagcgtaagaaactgttcaccagatacccccaagagccagcctttctgtctagggatgttttagttttttagttcatttttttttttaactttaaaattttctgttcatctgcaatttgttagatatgaagtatgtgtctaatttaatttttgtttttggttgtccccaataatgtttacagaagaatttttctgcactaattggcttgagttacttacattctcatagttctctagtttcagtagtttcatttattattttgttatatcaatctatctgtctgctcatctattagaagcatccttgttttttttttttcttttttagacagagtcttgctctgtccccaggttggagtgcagtggtgcaaccatgcctccctgcagtctcagggctcaagtgatcctcccacctcagctcctgagtacctgggactaccggcatgtgccaccacacccagctaatttttacattttttgtagagacagggtctccctaagttgcctgggctggtctcaagctcctggcttaagtaatcctccctccttggcctcccaaagtgctgggattacaggtgtgagcaactgcacccggctacaagtatacttcttaattattgtagcttaatggtatttatgaggggatcagttcccctgttgttctttagaattttctggatattcttctttattgattttgggatgtgaacaatagaatcaacttctacttgtagattgatttagggagaacttatacctcagatgttaagtcaccctgtccagaatgtgggatgctttcctatttgttcagaactttttaaattacctcagaagcacatgaaatttaaaggattttaaaaaaaacttaaagattatttcacatagctcttgcacatttcttgataaatgaatcctcaggtattcctctgtttttgttactaatagttacttcttatgggttttttttcccctgaaaatcatttatcaaacgtatgtggcttattttctgaaggatgtttgataattttggaagatatgaaagtcttcatattttacaaggtttgaggtctctttaagctgcatggttctcatgtcagctcccaaagcagaagacggcatgttgaaaaatgccgtagagaagatacttcttttccacctgttttcaactcatatcatcttgaatttcagggcacctttccatgctcctagtgcttgctatctgtttattattttccttcctgaataccctgaactccagcatgttctgctgtaattctggcctccctggcatcttggactcctgtttcctttgctctgtcatccccgcggtcagctcctgctgcgcagcttctcagctgaagtgcgtttggagtgcctggcgtgtcttgctggatctttgagtattgcctctggtttccttggttccttctgctgagttgctcagcgtctccactccccatttcttgtgtggcccttcctgcactcctctgattccttttgtcttccctggtttcttgctttggtttcgagtctccacagaacttttgcagctcttctgaagacctggaagctttttcatcttaattctcatctcatgacctcttttcccttctttgagagctagaacttcccatggtgaacttctctttccagaattccatgccttcttttccctcccacttacctgttgtccaggagaggtcagattgctgtgcatattggaggagaaccctttcttccctgggctcttcatctcacatgacatcaccacatcacctcgttccttggaccctcagtggtgtcactgctggatttttctttcctttggctggccttagggcacacccaggttgactagcgtagtcatggtatttagatccactcacattttcagtttctgtgtctgtctcttgcctgcttctgacttcgcccagagaaagcttctctttcacaagggttcttagatttatgttcactgagcaccttcttttctgaggcagtgttttaccaatatttattttcctagtcagtctcgccttacctttcttgttatgcatgtctttggtcctgacccattctctgagtctgtaaaatagaattgctgtataatttaattacatgaaatcctttagaatcttaacacatcttacacctgatttaatattttattgtatccaaattgaaccaaccctatgtgaatttgacagtgatttctcccagggatcctagtgtataaggaataggacttagtattttctattttttgatataccacataccagatactgattatgatggacatttaacccttttttctcattatgaaagaaagttaggaattatttcttccagtagcgccagtgtaacctgaaagcctttgaaagagtagtttttgtatagctatctgaaaggaatttctttccaaaatatttttccagtgctgacaacaaacacgcagacacaccctgcaaggtgagtgtacggcgccgcacagtggaggcatctgctgcagccgtcgatgtttgtgtctttggttgtacattatgagatcgtgacagggccagtaaccgtgtgttctctccttcaccttcccaaggtcacgctggatcttcagaacagcacggaaaagtttggagggtttctccgctcagccttggatgttctttctcagatactagagctggccacactgcaggacattgggaaggtttgtgtcttgttttttctccttgggttgtggctggcacacttgatgtgcgtcttctgggctgagttcatctaggatggagcctggttctccagggtgcctccgggagactcctccctgccccacgtgcttgcgtcacaggacccaagtctgactctgccttagccatgaagtttagggggaagtttctatttgtattctatttttgtctgttatcatgtattagcttagacccagtttagtttggaaaatcagtgggtttcaaaatgtgtttgtagagtcctttatttcttaacttgaccttttcaagtggaaaggggcaaaacagacgggtaagggggcggggcgggaggtgtgacttgctcttttgtgcctgaggaagtaacagagctggggttgacagtcatattctctgacacagatagtctctgacttatctcacagaaagtcagcggcagagcctgagttaaaagtctcgtagattttctttttcttttttttggtggctaatttcagttttatttatatttgtttatttatttattatactttaagttctgggttacatgtgcagaatgtgcagttttgttacataggtatacacgtgccatgatggtttgctgcacccatcaacccatcacctacattaggtatttctcctaatgttatccctcccccagtcccctcactccccatgggccccggtgtgtgatgttctcctccctgtgcccatgtgttctcattgttcaatttccacttgtgagtgagaacatgcggtgtttggttttctgatcttgtgatagtttgctgagaatgatggtttccagcatcatccatgtgcctgcaaaggacatgaactcatccttttttatggctgtatagtattccatggtgtatatgtgccacattttcttaatccagtctatcattgatggacattcgggttggttccaagtctttgctattgtgactagtgccacaataaacatacatgtgcatgtgtctttatcgtagaatgatttataatcctttgggtatatgcccagtaatgggattgctgggtcaaatggtatttctagttctagacctttgaggaatcgccagactgtcttccacaatagttgaactaatttacactcccaccaacagtgtaaaagtgttcctatttttccacaacctctccagcatctgttgtttcgtgactttttaacgatcgccatcctaactggcgtgagatggtatctcattgtgattttgatctgcatttctctaatgaccagtggtgatgagcattttttcgtatgtctgttggctgcataaatgtcttcttttgcgaagtgtctgttcatatcctttgtccattttttgatggggttgtttgcttttttttcgtaaatttgtttaagttctttgtagattctggatgttaatcttttgtcagatgggtagattgcaaaaattttatcccattctgtaggttgcctgttcactctgatgatagtttcttttgctatgcagaagctctttagtttaattagatcccgtttgtcaattttggcttttgttgccattgcttttggtgttttagacatgaagtctttgcctatgcctatgtcctgaatgttatggcccaggttttcttctaggatttttatggtcctaggtcttatgtttaagtctttgatccatcttgagttgatttttgtgtaaggtataaggaaggggtccagtttcagttttctgcatgtggctagccagttttcccaacaccatttattaaatagggaatcttttccccattgcttatgtgtgtcaggtttgtcaaagatcagatgattgtagatgtgtggtggtatttctgaggcctctgttctgttccattggtctatatatctgttttggtaccagtaccatgcagttttggttactgtagtgttgtagtatagtttgaagtcaggtagtgtgatgcctccagctttgttcttctagcccaggattgtcttggctatgcaggctcttttttggttccatatgaagtttaaaatagttttttccaattctgtgaagaaagtcagtgatagcttgatggggggatagcattgaatctataaattactttgggcagcaaggccattttcacgatattgattcgtcctatccatgaacatggaatgtttttctatttgtttgtgtcctctcttatttccttgagcagtggtttgtagttctccttgaagaggtccttcacatcccttgtaagttgtcttcctaggtgtttcattcccttagtagcatttgtgaatgggagttcactcatgatttggctctctgtttgtctgttattggtgtataggaatgcttgtgatttttgcacattgattttgtatcctgagactttgctgaagttgctaatcagcttaaggagattttgagctgaaccaatagggttttctaaatatacaatcatgtcatctgcaaacagggacagttttacttcctctcttcctatttgaataccctttattgctttctcttgcctgattgcgctggccagaacttccaatactatgttgaataggagtggtgagagagggcatccttgtcttgtgccggttttcgaagggaatgcttccagtttttgcccattcagtatgatattagctgtgggtttgtcataaatagctcttactatgttgagatacgttccatcgatacctagtttattgagagtttttagcatgaaaggctgttgaattttgtcaaaggccttttctgcatctgttgagataatcatatggtttttgttgttggttctgtttatgtgatggattacgtttattgatttgcgtatgttgaaccagccttgcattccagggatgaagctgacttgattgtggtggataagctttttgatgtgctgctggattcagtttgccagtattttattgaggattttcacatcgatgttcatcagggatattggcctaaaattctctttttttgttgtgtctctgccaggctttggtatcaggatgatgctggcctcataaaatgagttagggaggattctctctttttctattgattggaatagtttcagaaggaatggtaccatctcctctttgtacctctggtagaattcggctgtgaatccatcctggactttttttggttagtaggctattaactattgcctcaagtttagaacctgttatcagtctattcagagattcagcttttttctggtttagtcttgggagggtgtatgtgtccaggaatttatccatttcttctagattttctagtttatttgggtagagatgtttatagtattctctgatggtagtttgtatttctgtgggatcggtggtgatatcccctttatcgtttttattgagtctatttgattcttctctcttttcttctttattagtcttgctagcggtctacctattttattgatcttttcaaaaaaccagcacctggattcattgattttttttggagggttttttttcgtgtctctatctccttcagttctgctctgatcttagttattttttgtcttctgctagcttttgaatttgtttgctcttgcttttctagttcttttaattgtgatgttagggtgttaattttagatcttttctgctttctcttgtgggcatttagtgctataaatttccctctacacactgctttaaatgtgtcccagagattctggtatgttgtgtcttcgttctcattggtttccaagaaaatttttatttctgccttcatttcgttatttacccagtagtcattcaagagcaggttgttcagtttccatgtagttgtgtggttttgagtgagattctcaatcctgagttctaatttgattgcactgtggtctgacagacagtttgttgtgatttctgttcttttacatttgctgaggagtgttttacttccaactatgtggtcagttttagaataagtgcaatgtggtgctgagaagaatgtatgttctgttgatttggggtgcagagttctgtagatgtctattaggtccgcttggtccagtgctgagttcaagtcctggatatccttgttaattttctggctcattgatctgcctaatattgacagtggggtgttaaagtctcccactattaccgggtgggagtctctttgtaggtctctaagaacttgcttcatgaatctgggtgctcctgtattgggggcgtgtatatttaggatagttagctcttcttgttgaattgatccctttaccattatgtaatggccttctttgtctcctttgaactttgttgatttaaagtctgttttatcagagactaggattgcaatccctgctttttttttgctttccatttgcttgttagatcttcctccatccctttattttgagccaatgagtgtctttgcatgtgagatgggtctcctgaatacagcacaccaatgggtcttgactctttatccaatttgccagtctgtgtcttttaattggggcatttagcccatttacatttaaggttaatattgctatgtgtgaatttgatcctgtcattatgatcctagttggttattttgcccgttaactgatgcagtttcttcatagcgtcagtagtctttacaatttggcatgtttttgcagtggctggtactggttgttcctttccatgtttagtgcttccttcaggagctcttgtaaggcaggcctggtggtgacaaaatctctgcatttgcttgtctgtaaaggattttatttctcgttcacttatgaagcttagtttggctggatatgaaattctgggttgaaaatactttttttaaagaatgttgaatattggctcccactcttttctggcttgtaggatttctgcagagagatctgctgttagtctgatgggcttccctttgtgggtaacccgacctttctctctggctgccctttccttcatttcaatcttggtggatctgatgattatgtgtcttggggttgctcttctcgaggagtatctttgtggtgttctctgtatttcctgaatttgaatgttggtctgccttgctaggttggggaagttctcctggataatatcctgaagagtgttttctaacttggttctattctccccatcactttcaggtacaccaatcaaacgtagatttggtcttttcacatagtcccatatttcttggaggcttggttcatttcttttcactcttttttctctaatcttgtcttctcgctttatttcattaatttgatcttcaatcactgatatcctttcttctgcttgattgaatcggctgtcgaagcttgtgtatacttcacaaaattctcgttctgtggtttttagctccatcaggtcatttaagctcttctctacactggttattctagccattagtctaacatttttttcaaggtttttagcttccttgtgatgggttagaacatgctcctttagctcggagaagtttgttattaccgaccttctgaagcctacttctgtcaattcatcaaactcattctccatccagttttgttcccttgctggtgaggagttgtgatcctttggaggagaagaggtgttctggtttttggaattttcagcctttctgctatggtttctccccatcattgtggttttatctacctttggtctttgatgttggtgacctacggatggggttttggtgtgggtgtcctttttgttgatgttgatgctattcctttctgtttgttagttttccttctaacagacaggcccctcagctgcaggtctgttggagtttgctggaggtccactccaggccctgtttgcctgggcatcaccagcagaggctgcagaacagcaaatattgctgcctgatccttcctctggaaacatcgtcccagagcacgaaggtgtctgcctgtatgaggtgtttgttggcccctactgggaggtgtctcccagtcaggctacatgggggtcagggacccacttgaggcagtctgttcattatcggagcttgaatgccgtaccgggagaaccactgctctcttcagagctgtcaggcacgtatgtttaaatctggagaagctgtctgctgccttttgttcagatgtgcccttcccccagaggtggaatctagagaggcagtaggccttgctgagctgcagtgggctctgcccagttcgagcttccctgctgctttgtttacactgtgagcatagaaccacctactctagcctcagcagtggtggacacccctcccccagccaagctcctgcatcccaggtcgatttcagagtgctgcgctagcagtgagcaaggccccatgggcgtgggacccgctgagccaggcacaggagagaatctcctggtctgctggttgtgaagactgtgggaaaagtgcagtatttgggcaggagtgtactgctccttcaggtacagtcactcatggcttcctttggcttggaaagggaagtcccccgaccccttgtgcttcccaggtgaggcaacaccccgccctgcttcggcttgccctccgtgggctgcacccactgtccagcaagtcccagtgagatgaactaggtacctcagttggaaatgcagaaatcacctgtcttctgtgtcgatctcactgggagctgtagactggagctgttcctattcggccattttggaagcatcccttgttttttgaggtggagtcttgctctgtcgcccaggctgacgtgcatcggcacaatctcggcccactgcaacctttgcctcctggtttcaagcgattctcctacctcagcctccggagtagctgggattacaggcacctgccaccatgcctggctaattttttgtatttttagtggagatggggtttcaccacattggccaggctagtctcgaactcctgaccttgtgatccacccacctcagcctcctagagtgctgggatcacaggtgtcagccaccacgcccagccatattttcagatctccctctctttgccctaaaccactgtgcttaataagtagtttttagtggccagcagtctccatgtataacacattttagcaaaatggaaaatactatatgttttaaatttgaacgtgagattatactgaaataaaaatcatctaactgggattctttaaatagtaagattttcttttttgtatgtgggtttttttttaaccttattattatgactgtcatatatagaaatggctgtttttcagttacagtcagtgaatgtatcaaatgctgccttatccaaataataaaagtaaattattaataagtcacaatttaatgaagattgatgttagttgatctttatattcttgaaatcagccatatggttgtgtgtgtatgtatatatttttaaaggtacataaagataataagctcatctctgaaaatttttacatttggcataagaataactggataattaagcatcttattctctggcctgtgtctttacagttaaaggtagatttactcacctctccttttttgtttttctaagttcatcttttttgctgtttcaagacagaggcccattttagctttctcgcatatccttttgtttgtactttggaagcctcacctgcttaattgttgagtttttatccgtggtcttttagagggggatatgtagggtagaagctttcacaggttcttgtttgcacttggcccctgactgttttgaggaatctccctcactgactcacagcatggcaaggtttcagatctctttctgccacacagcagttctgaggcagctggaaagatatccagatgcttagattgtcaggccaggcttgagatatacaaactattgagccttatctgtgaccttgcttaggtgaaggcatcagagcccctgcaccaacatgcataggcctctgcatgtgtgcggggctgggtgttgaggtctgagcacaagtgtagctggagaggtgagcttgatgtggcgacgggtatgagcaggttttcttcagacttctgtgagtttacctagttccaggatttaaaggcacagagactttagaattaaaatagaatcattttctttttctaaatagcaacactaggaataaaaaataataattccacattcttgacaggtaatgttttttcttgtcttctaatccttatttattccatactcatttttatacataattgaaatgtattatgcattggatttttcttttgcattatattatagacgatttttcatgtaactccttactgttccattttatatgttttgtctggtttaagactttatctgcaaaccgggaaactgtctctacaaaaagaaaaacaaaaatagttggccgcagtggcatgcgtctgtggtcccagctactcggggctgaggtgggaggattgcttgagccttgggaggttgaggctgcaaagagccatgatcatgccattgcactccagcatgggtgacagactttatactgtctgttttgggtgatttgataatgatatgccctgatgtagtttttttatatcttgtgtttcttgtgcctgggtttattgaggttgggtctgtggcttcatagtatttttaaagtttggaaaattttaggccattctttctttctttctttcttttttttttttttgagacagtgtctcgctctgtcgcctgcgttggagtgcagtgacactatcttggctcactgcaagctctgcctcctgggttcacgccattctcctgcctcagcctcctgagtagctgggactacaggcgcctgccaccacgcctggctaattttttgtatttttagtagagacgaggtttcactgtgttagccaggatggtctcaatctcctgacctcgtgatctgcccgcctgggcctcccaaagtgctgggattacaggcgtgagccactgcacccagctaggccattatttcttcaaagattttttttctgccctgcctccctccttttttccctctcttaaaggggctgtgatttcctgaatgattgcttagtgttgtcccatagcttactgatgctcttttcagtgtttgattgttttatgtgttttctgttttgtatagtttctattattgtgttttcaagttctctgatcttttcttctacagtgtctactctgttgttaatctgttaatctgttgttaatcctgtccagcgtatttttttttttgtttttgaaacagtctcactctgttgcccaggctggagtttagtggtgcgatatcagctcactgcaacctccacctcccaggctcaagcaattcttctgcctcagcctcccgagtagctgggactataggcacgtgccaccacacctggctaatttgtgtatttttattagagatggggtttcaccatgttggccaaactggccttgaactcctgacctcaggtgattcatccgcctcggtctcccaaagtgttgggattataggcatgagccaccgtgtctggcccctgttcagtgtatatcactaattttgtttttatctctagaagtttgatttaggtcttttaaaaatgtctccctgtgtttctgtttagctttgtgaacacaattgtaataactgttttaatatccttctctgctagttctaagatcttctaataacttcccagttcttggtgtttctcattggttgattgatactcctcgttttgggttgtattttcctgcctctttgtatggctgccaattttttattggatgcccaaccttgtgaattttactttgttggatgctatatatttttgtgttcccatagatcttcttgagctttgttctgaggttagttgagttacatatagatggtttactcttttgggtcttgctttataatttgtcagatgggttggagcagtgcttagtttaggactaattttttttttggactaattattcctctttaggaataattaggtaccatgcttaggaggcaagaccatcctgagtactctacctaatgaaccagaaagtttgggttttccagtccgcctgctgagaacagtgactttctagccctgtgtgagcgctgagctctgctccttctaatcctttccaatgcttctttccctggcctcagggagttttctcacacacatatctctgctgagtactcgagagggaccttccccagatctccagagctctctctgtcttgttttctcttctctggtgctctgtcttatgaactgtggctgtcttggtctccttagattctcagcacctcttcaattcagagggttgcctgtccctcctccttgtgccacagcctaggaactctctcaaagcagcgagttggggcagccatagggctgacttagtctctcgtctcccagggatcactgtccttcattgctcatgtccagtgtcttgaggactctgggttttgtctgttttgttttttggtttgctttggttgtctcaggcaggagggtaaacccagtccctcaccctcattgtgctcagtagtggaagtctcactctattacattagatattagtatttgtagcagagccctggttccctggtacttggggagctcttgaaaggccagaaacagcatgctttctcaccttttccagggcttcagtttctggtgcacatcaagcattccatacacatttgttaaagtcctttgttagacaagtagtgattcacaggttctatttgtaattttttcagttaacatgtattgggtatctgctgggagctagtaaaaacaaaaagtggtgtgtgacaaattcaattctgacaagaacaaccttaaacacttagaatatactttgagcatatcagaattttaaaaatgtgtggcccttgagtatttgaaaccaacaagaatctattgcttattagtagaggatattttgttaaacaagtggagagagaggcattttcagtctaattggtgttggcttttagcagctgatggaaaccagttcgtgattagccaggcagtggtgaaacaggctgtgcattctgaatgcctaggtatctaggcattcagaatggtggcgctctttgagttagcatcttcttctttcttgattcttttttttttttttttgagatggactttcgctcttgttgcccaggtaacaactccagtgcaatggcgccatctcggctcactgtaacctctgcctccctggttcaagcgattctcctgcctcagcctctcaagtagctgggattacaggtgtgcgccaccacgcctggctaattttgtatttttggtagagatggggtttcactatattggtcaggctggtcttgaactcctgacctcaagtgatgcacctgcctcgatctcccaaaatgctgggattacaggcgtgagccaccactcccagccccttcttgattcttgaaaaggacattgggtgctgtacatctcgttatagatgttgataaaaatgcttgtgagaagagtaacattaaggtagttatttggtcatttttgcagattattttaagacaattctaggactgatttgtggtaaatcacacattgctgtatcatagttgtgttcactgaacatattcaggggctctacagatgcagggctcttagctgctttgcacacttctgaattcctgccctgcgaacaggactggatacctaatagacaacaggtacttgataacagtttattgaattaatgagtgaatgaacagatacataaatgcatgaaagaatggttgtaatgtatataacttggatttcaagactttttactgactgttcaaaataagaaattgaaaactttcctctgattttcctctactatttacacaatttaaatggaagttatcttgtaccttcaatttctgtctaggattcgtacaataacgggtcatctctgagtcgcttaatgtctcacttgtctttctacagtgtgttgaagagatcctaggatacctgaaatcctgctttagtcgagaaccaatgatggcaactgtttgtgttcaacaagtaagagcttcattcttttcctcttctgttaagacgttcgggtatgacagcaaaacgctgctactccttaagaggcaggcgctgttggcataatcagctgggaggattgtggggtccagcgcagcactttttggctcagtccatgattgagccaagaggccatccttcccttcactccccaggaggacgaggtctgtcactgtggagggcagaggacaccagaagctcctctgcaacctcgctagttaacttccagtccctcggagtttctgtttagaatgctcaatctcatttagaattgcaaggaaacccaaaacgcctatttaaggtacaaacagcacttcatacaatatctcatgaggtattaatagtgattcacaggaagaatttcacgctgtgagtctttgctaacatatccagttatttacagatggatttgatatttgtgtgggagattcttaaaagtgttgttcacgccacattgttgatgcctcatttttttcactgtagttgttgaagactctctttggcacaaacttggcctcccagtttgatggcttatcttccaaccccagcaagtcacaaggccgagcacagcgccttggctcctccagtgtgaggccaggcttgtaccactactgcttcatggccccgtacacccacttcacccaggccctcgctgacgccagcctgaggaacatggtgcaggcggagcaggagaacgacacctcggggtaacagttgtggcaagaatgctgtcgttggtggaagcacgaaagagcaagcaggaaatactttgtaaaagaataaaaacgaaaaatgttagcgaacatcttctaatagtctgctgtattcagagaactctaggagatatatatggttgatgcaaagatgatttaaggcatagcccggccttccaagaagtgtgtggccagtgagtgagatgggcttgggacttacacatctcagaggtgggggtagaggaggaggaacactgagtgggctgagaagcagccagctctcattgccaaagtgtgtcagcaaaccagaatgcagttcataatgtccccacccattcaaagcacaggacctgtagagtggtgtggcatgtgttggtggcacttttcaggcctgtaacaaggatgaaagaacagcttcatagcagcacagtagtgctggtgttcagaggtgtgtgaaggccatagaagcatcttggatatattaccttgtgttttgtcagctttatgactagaagtctcttttcacttaaatttgttttttttttttttgagacggagtcttgctctgtcgcccaggctggagtgcagtggtgcaatctcagctcactgcaagctctgcatcctgggttcatgccattctcctgcctcagcctcccgagtagctgggactacaggcgcctgccatcacgcctggctaacttttttttgtatttttagtagagacggggtttcaccatgttagccaggatggtctcgatctcctgacctcgtgatctgcccgtcccggcctcccaaagtgctgggattacaggcgtgagccaccgcgcccggcctcttttcacttaaatttatgtttgtgtttttaatgcctagtatacaggacttcttaaattgccttaagtatgaacaggtatttgagttgctaatctgtatagtagcaataatagaatcccttgtttttccttttataaatttagcgattaaatagctacaattaaaacactagagtcaggagtcaaggaaaatacccatgttccaggctgtatgttagtgatgtacttactatatattggagtttcaggagtaagtctgtttcaatgctttctgtaaccatttggggtattaataagcatgtgagtgtgtgcatgtttgggttaatttcatatatgtttcttagaagggatatcattgatgtaaatattttaaaggcttgtcctccaaaaaaatcatgtaatttcttctaaattactgatcttttaaatgaccttcacctttctctcaaatctcacttaagactgggctgagtagtcagtttcctgtagcagaaaaaagctcagacttgagtagccttctgcgagtgaggagacttgatggctgtcaggcagctgtaaactctaaatagagtgtcattatctgaagagggcgatgctgccacactgagtggcctttcaagttgtttctcaatctgacacgttctgatcgtgtgaatgtgaaattggtttgagcaggagtatatctgagtgcagaggagattatttaaagatattctcattctctgcttcccttttattcccatttggcagatggtttgatgtcctccagaaagtgtctacccagttgaagacaaacctcacgagtgtcacaaagaaccgtgcagataaggtaaatggtgccgtttgtggcatgtgaactcaggcgtgtcagtgctagagaggaaactggagctgagactttccaggtattttgcttgaagcttttagttgaaggcttacttatggattctttctttctttttttcttttttatagaatgctattcataatcacattcgtttgtttgaacctcttgttataaaagctttaaaacagtacacgactacaacatgtgtgcagttacagaagcaggttttagatttgctggcgcagctggttcagttacgggttaattactgtcttctggattcagatcaggtttgtcacttttatctttcatccatcatacctgttcctaatttagtacaaattaccctaaaagacactgaaatctactttaaagaaatgtggtctgcatgtttccctcatcagttgctgctgcttatctttttcatgcacctagctggtgcagaaggcctggggcatagccagcctcagcaagtcagcatccttgccccagctccctggactcaaggctaacctggggttggctgttagggatttccaaaggtttgtcccatccacttgcctcccctccaaaataagtttgaatttaaattgtgagatacaattaagatttattgtttggggaacatttttgcaaaatctagagttagtttaaacagattatcaattattaccataattgatcatctgcagtttcaagctatctaacaggttcacttacctctttaaaaaggaatggaatttagcaggacagtaactgagacccgtgctcctggagtccatgtgggagctgtgtggctctgcacaagcatttgcacgcttcccctcttgactgcattaccttcctcctatagttgctgtgggcaccagattctggctagtcctgtcccttcatgatgcacattttcctcaagattcgtcccagttaaatcactgcagatgaaactgccttttcatcgtcaaaatttaactgtcatttttgagccgtgatcttgggctactttcttatgtggggtaggaatatttgtgagttagaaatattacacttctctatttccttctagacgtaaatctgttaatcctgtcagcactgttactcacctgaaagggtctgtttccctaggagaactgagggcactcggtcaacactgattttccacagtgggtattggggtggtatctgcttgttttttttgttgttgttgtttgtttttttttgttttttttttgagatggagtctcgctctgtcacccaggctggagtgcaggggtgcgatctcggctcactgccagctccgcctcagaggttcacgccattctcctgcctcagcctcccgagtagctgggactacaggcacccaccactacgccaggctaattttttgtatttttagtagagacgaggtttcactgtgttagccaggatggtctccatctcctgacctcgtgatctgcccgcctcggcctcccaaagtgctgggatgacaggcgtgagccaccgcgcccggcctggggtctgcttttaatgaaggaggcatcaaggggtgggctttgcgttggcctgatgctttcatctttctttcacaaaacctgtccgaagaaaatccgtctaaatgggccattgctctcctcaggaaatagtcattgggaacttcttttcctttcctttgacactaggaggctgactggggagaagccctggtctatggctgtgggcagcaggggctgagaggagcaggctctcaggggggcacgggtaccccaagggaagccagagccctgatttgttccattctagtaagaacaaagactgctctggtttcatgtttgttctgattgcctttcatcaaccggtcccctttctcccagttcttaagattcagtacagtgacagttttatgaacaagaatagaacactagaacagacaaaccattgaactctatgctgataaagatttattgagctcctgctgtatgtttgcattctgcccagaggctctgagaaaaccaggccatatgctccatgctttatccatggaagctccccgtcaggttgggaaagctgacagctgcagggaatacagtgtgacacaaaactggctcccatgcagcccttacgtgtcgcctctcagatggttgggggacgaaggtcgactcctttgggtatcttattactaaaccagtttcagggaatctgtgccaccctatctgccattaacgtgaacagatgagtccccaaggtgtaattttgggtattgtctgatgtctcttggaatttattatttgtttttccaatgagatttcacctcagggtatagtaaagttgttgaggggattcctggatgtgttctgcaattatctaggctgatttcagaatagagttatgcttatagtcaaatttatcagctgtcaagaattttatttaaaatttatgcagataagcaggaggaaaagaagcctggtttttacattttaatcctattattgatgtgaaattttattttccttcctgtaggtgtttattggctttgtattgaaacagtttgaatacattgaagtgggccagttcaggtaatagcattttattattttagatttttttcttcttcttgtgtacttacatgtaatttaggttattaagtgaatgtttaaactactgttaggcatttttgctgttttctttaaatggaaatctgactaacatactgtgcatttttgcttctcttaaaaattaatgtatatctcaagacttgtttggaagtagttatgtatctgaaaattccatatgttgtcagtattcattgcacatttcaaagcatttaattgtgttgacagatggtggaatgaaatcttgtggtggagcactagtttttaaatcttcttagagaaagcagttttatataatgttgtctttagtaattattatgcatttgtattctctgcagctttttcttgctagatgttgaggttttaatacttcttgctagtccattacaggtttataattattaaaagttaaaattcttttagtacctaaaatgcttaataaacattgtaattaggaaaatttagtgcagaaggaaagtgttcccagattccctggggtctggaaacatagtgtttattctaattacatgacacctccactgtgttttggggcaagttactgtttctcttttgagtttcaatttcttcaagagcaaagaggcagaggagagctaggaagatcgtagctgctgtgcccctgtgccgtcgggtgccttctacctgctgcctccgaacctttacacatgtccctgctctgcgcgagggcacagatgggatgcactgtggcaggggtggggttagagtagatcacggacacctgttagcttgatgtgtgcttgctgtcaaggttgaatcatgaattattttatgttgcttatattgatatgtatcttaattttaaaagaaaggtctaaatggatgtttttgtttttagggaatcagaggcaatcattccaaacatctttttcttcttggtattactatcttatgaacgctatcattcaaaacagatcattggaattcctaaaatcattcagctctgtgatggcatcatggccagtggaaggaaggctgtgacacatggtaacgggacacacctttcactgtcgtcttcggtgtcgtgatgtgcttggcagtgttcgttttcatatacccactttgaacgttgtcagtggcagccatgtgcttctcaggctctgcatgtgtgtctgtgtatgtgaaggtactggttagagacgtttcaaaagagaagagagcatattctttactctcagcaatttgtaatcttctcagggaaaaaaattcaagaaacagtaagataacctaaggtacagatagattctgaatataaagttcctgttcattcacatgaaacgctaaaagttcttcacttgatcttagccaaaaggccaagaagcgatgcaacactaaaaattcttaaatcgaacttgccgtgaattaaattttgatctctcatccagtggtattggagatatagtttgacttgggttcagggctttctgttttgcctgatgattttgctggagcttaaataaggaacccaggagatggccagctgtgcaagcccccagcctgtggaaggagctagtgtggttttatgaatgagttgcaaatctttctttgagctttttgaactgatcttccagcattgccctattgacccctccctgactcctttgctggaatctgtaggcttttgaactttgacagggacacatcctaagacccttgcaaactcccagatgtgagaatggcactactacttagagtcttttcgactcagcgtgtgtgcagaagagcatcaaccgggctgtgttgcgaggcagggccttggctgacctctcagtgtttacatagctaagccagttagtgtttgccacggcctcacaagggcttcagattcacacagccaaagtatagattattaaaggcataggtgtttggtttcctggacttggagggtctttggacagaaaatcagtaggcaaccacacccagtactttgtgctgggaagcttggtcatctgtgagagggtcagagagtatacccatgcgtgcatgccaccgaagggtcagtgagtattcctgtgtgtgcatgtctcagggccggagagagtatgtgtcactgagaggtcagagtgtttgtgtgtgtgtcaaagagggttgcattgtgcccttcactgaggggtcagagggtgcctcgcgtgtgtgtgtgtgtacgtgtgtgtgtgtcactgaggggtcagagtgtgcctgtgtgtgtgcttgtgtgtgcgtacatgtcactgaggggtcagagtgtgcctctgtgtgtgtgctcatgtgtgtgcatacgtgtcactgaggggtcagagtgtgcctctgtgtgtgctcatttgtgagcgtatgtgtcactgagggggtcagagtgtgcctctgtgtgtgtgctcatgtgtgagcgtatgtgtcactgagggggtcagagtgtgcctctgtgtgtgtgctcatgtgtgagcgtatgtgtcactgaggggtcagtgttcctatgtgctcatgacattgagggtcagagtgtgcctgtgtgccaatgaaaggcatttcttatatttttttatatgtggtcatagtagaccagttaatttattttgactcctgtgttagaccaaaataagacttgggggaaagtcccttatctatctaatgacagagtgagtttacttaaaaaagcataataatccagtggctttgactaaatgtattatgtggaagtctttattgtcttttcagatgaatcaagtagattattcttgagaccaggaatgttgctgttttggttatttggaaagttttatcattttcaaattgacttttgaatttgagtcaccttttttcagaagtggtgttaaattataggagccctaggttttttttctttttttagaagtcatcacaaaatgatcagtgttcagaggaagagctttgaccttccacatggtataatgattgataaccttaattcatctcttaccataaaccaagtatgtgtaagggttttctttatttcttgaaagcattttgtagatgttgagagcagttttccaaatgtaatttccatgaaatgcctgataagggtacccttttgtccccacagccataccggctctgcagcccatagtccacgacctctttgtattaagaggaacaaataaagctgatgcaggaaaagagcttgaaacccaaaaagaggtggtggtgtcaatgttactgagactcatccagtaccatcaggtaagaggaatgtatgttggaactgtcgtggatactttattgacccgtgcagatggaaggaagtgccatgtggtaacgctcactgttaactgtgttactttgaaccaggtttgggctttctggggcctgggtagatgccggtgcagggggatggggagggaggcggggggtgggggggtgtggtggagttggggaggtgcagtggcaggaggtgttgttggtgtgtatcctttttttttttttgagatggagtctctctccgtcgcccaggctggagtgtggtggcacgatcttggctcattgcaagctccacctcccgggtttaagcaattctcctgcctccacctcccgagtagctgggattacaggcatgcaccaccatgcccagcaaatttttttttttgtatttttagtagagatggggtttcaccatgatggccaagctgtttcgaactcctgacctcaagtgatcctcctgccttggcctcccaaagtgctaggattacaggcgtgagccaccatgcccagcctggtgtttatctttaaagtgggcacagccacaggagttcacctgactcctggtctgagagtcacgagatcgttcaagatagtgaggccctcttttccaaaacgaggaccaaaaatcaattgacagtgttggtcaagatggtagaaaccttaaaatgatagaaatctcaactctgaaataaaaactttatttgtatatttatttaccactattttgacatagggctaaggtctttttctttgagctgatttctggttttgttttcttaaagtggcataagaattcaaagacattttgaggaaggctgagtgcagaaatctctctttttaaatgacttctcctttcttttaacttgcactgttgtctagccctcacttattttgtcaattctttttagctgtttgtctttgaatcttcataaagccatagcttttctcataagaagcagcactttctttgttcattcatattttaatgaacccctgtagtatttaattaaatacttaatgcctaattaaatcacataattgcaatgcaaaagtacatgtatcataaagaggtctgaaaatgagcaactggcaagcaggtggtggcaggcagagctgcttgggtgggtgggtgtcatggagaggagttcatcagccacatgttcagtgagctctggatatgtctgtttagaaatgatcactaataaacttgtgctcaaccatgtatacctctgggaagcaggtgctcttcagtagattgcctctgcagagaacacagaattgaagtgaatgtccacaaaggcaatgagccacctgcagaatagtttagtcaaggctgtgtttgaagtttgccaaagattaatatacatttgattttcatgttgtgccttttctctgattgtgaaatattacaaattctatacaaataacaatgatggcaaatcctcctgagcaaagtgtgcaccttgtatgtgccctagaggaacttgtgtttcgttctgattcccctacatttctcatgtcatagagtgggggttgcattagtgtccccctgtcctcgctgggatcacatctgtttggatcctagagtcttccagctgaactgggacaagtataacagacggacacgtaggggtggaaaggcgtctcttggcagcagactttctaattgtgcacgctcttataggtgttggagatgttcattcttgtcctgcagcagtgccacaaggagaatgaagacaagtggaagcgactgtctcgacagatagctgacatcatcctcccaatgttagccaaacagcaggtttgtccccgcagccttggcttgttgttgcatagtgatggtagcttaaggtccttgtgaaaggtgggtggctggaatcagctcttccttcagtcctaatctgtgccttgatagcagttctccgtgctagtcatgggacagctgacttcatttcttctcacaatgccatctcaggttggtattgcccacctactttacaggggggatcccacagctccgagaggttatggaggtgatcaggcagcacacagctttagagtgctggggtgagggcgggccaaggctaactctaaagcccgaacccttacctcctacactgcctcctgcattctggtcaacccagtgttttatttggtggttagatttttgtttttgttaccttactgcttgtaatttagcagttttcctttcctttcccttcctttcctttccgacagggtctcactctgtcacccaggctagagtgcagtcgtgtaatctcactgcaacaacctctgcctcccaggttcaaccaattctcccacctcagcctcctgagtagcaaggaccacaggtgtgcaccactacgcctggctagttttttgtatttttagtagagatgaggtctcgctgtgttgcccaggctggttttaaactcctgggcgcaagtgatccaccaaccttggcctgccaaagtgctggcattacaggtgtgagccacctcgcctggcctattcatcactaatcagaatttctatgatcaaatgacatgaatcattgtttccacaactgcagtggaaggaaatggcctggcagtgccagtttcagaagcagcctgcccccagtcaggcacaggccactgtgcccccagtgtagcagcacctctgtagctcacagagaagggtggtggggacctccttgaggcagctctgccagaaaatctcatgagctgcctggcacagcttgaggttgccttttaagtggactcagcaaatacatgtttgttcatcttgattatacacaataaacaactactctgtatagtacgagtagtccgtggtttttggcatttgatttaaacttagaggcatgtgatattgatgttactgccttcatgactgcacccccattctgatttcataatggaatgttatcttgagaccagttagacaacaggacagggatcttggcttctggtgagattgacagcagttttagtgtggtcagggtctccctgcctacagatggttttagaatggtgccctggaagctttatcccattcttttctgtgcgtaatctgagtagagtggagatcgaaggcctgaatacatagtaaatacctgacttaatatctgccgcaatggaaattgtgtgatacaacatttatgaaacgcttagtgcagcacctgccaggtagctcaccacaggtgcatgttgcattcagaagtagtgctagatactatcctgttactggcagtgcatacatcagtgatcaaagcagattaaagaaagaccccctgccttcttggagtgaagattttgttgggatgcgggtaaggggacagacaatagaaaagcaagtgagtgaagtctataccatggcggctgatcaggaacaccgtacagaagaatccaggagggaagagagttaggtggtgtctgcggtgggagtggcattgttcagctggtgatgagaagaagctttggtgatctggtgacatttgagtgaatttgcagaaaggaaagatacaagcctaggagatacctggggaaggaacattccaggcagagcaaatagcagtgcaaaggccctggcggggggcggacatgctgttagggtacaagcaatgagggtggaggagtggggcagccatggggagggaagggagtgaggcctggtggggtgaggccagtgtggaggagccttgagagggtttgcgctgatgtggtgtaggttttagcaggatcattcttattcctgagttgagaatagccttgagggggaggtgagggcagagcagggccacccatgtgagacccggcactggagtggaatggcccaagtcagcatcccttggcagcatgaaagcaaaaccagcaaggtttgctggtggcttagatgtggcatgtgagagagagcagggctttgggggtgatttcagggtgaggacagggtggctgtggacaaggtagggcagacattgggggcagcaggaggtcagagcctgtctggatgtagcagttgagaccccataggtgcctaatgaggtgaggccagcatcaggtgtatgagcctggagttgtcgagagactgtggggcagggggtcagcatctgagatgtccactcacagtggacccagactggctggagaggaggaggagcttgaataccgagcctgctgagtcccagctccaaggtcaggtaggtgaggggagccagtgctggggcagggggagtaggcaggtgtggggttcctaaagccaagattttttttaaggcattttgtgcaggagggcgacatctgctgtcagcaccttgggaacttggcccaggtttggcagcaccgagggcactgatgagtgcttttggaggagcaaagggagccaaaccctaatgggaatgtgttcctgaaaggacaggagagagacttgggaaaaggttttacttgaagagggaacggagaaatagggcagtagccagaggaggagaggagtcggcaatgggttaagttggcagaaatgaaggcctgtttacgcactgagggcagaagcaacagggaggatcagttcatgacacaggagacacaaatcgccgttgtggtgttcacagacatgggttaggattggctgcatggatgacagagcactgtgggttctcccagagttgctggggaggaggcagagttggtgagcacaggcgagggtccaggatgcaggaatcctggagctcaagtcagttgttcccttgttgtaagatgtggccagtgttgtgagcttcacatctgtgccttgaaaaacaccacatctgtttgcagagttgtttactatgtatacacactcagtagaaacaaaaattggaaacagtcagtgcccaccatcaataagtaatggttgaacacactgtggtataagcttagactattttagcttgggctattttgcatgattaaaaatgttctggccaggtgtggtggctcatgcctgtaatcccagcactttgggaggccaaggcaggcagattgcttgagctcaggagtttgagaccagcctgggcaacatggtgaaaccctgtctctactagaaatacaaaaagtagctgggtgtggtggtgtgcgcctgtagtcctggctaactcaggaggctgaggtgggaggatcacttgagcccattcgtgcgccactgcactcctggggcacagagtgagactctgttagaaagagagagagagaaagaagagagagggagggaggaaggaaggaaggaaataaatggaagaaatggaagggaggaaggggagggaggaaggaagaaaggaagttcagccagttgccttgggagttctccattgcactgggttaagtgagaagagcagagacgtttatgatttttcaaaacaactaaaacaaaacctctgtgggtgagggggcaaggatatggctataggaacatggggcagattaagaaagggatatacacacaccacttagcatttgttacaactgttgtgggagggatggagtgcagaaaaagaaaaaaaaaagtgcacaccatcccatgtatgtgtatacaaagggacgcttggaagactggtccccaaaatgttggtaatgattgtgtcagggtgctgcagtgctagttgattttttttcacacttttgtatatttgagtcttttacagaaagcatttattatttatgtaataaaaatctaaatgacaagatttctgttatgggaaaaatgtagctatacagtgttgttgtaaaaatgtttgcttggttcaccactgaacttaaaatgcttttaaatgagggaaggtgacgatgagatgattatgatgatttgcccttgagttacatagctggtgtacaggaagctgtcgtttcttttggcttacgtagaaatgtttgtggtgtctaattccacagatgcacattgactctcatgaagcccttggagtgttaaatacattatttgagattttggccccttcctccctccgtccggtagacatgcttttacggagtatgttcgtcactccaaacacaatggtgagtctctcgcctggctcagcagatgaatctggacggcttgttcaggctctgattactgggaccacccccagaatgtctgagtcagtcagtttgggtagggcttcttgagagtttgcttttttttttttttttttttttggtgtgggggtggtgcggaacagagtctcactctgtcgcccaggctggagtacagtgtcatgatctcggctcactgcaagctctgccttccagcttcacaccattctcctgcctcagcctcccgagttgctgggactacaagcgcccaccaccacgcccggctaatttttttgtatttttagtagagatggggtttcaccgtgttagccaggatggtcttgatctcctgacctcgtgacccgcccatctcagcctcccaaagtgctgggattacaggcgtgagccaccgcacccggcctttttattttttttggagatggagccttgctctgtcacccaggctggagtacagtggcgctacctcgactcactgcaacctccgcctcccgggttcaagcaattttcctgcctcagcctcccgagtagctgggactacaggtgcgtgccactgtgcccggctaattttttgtatttttagtagagacggggtttcactgtgttagccaggatggtcgcgatctcctgaccttgtgatccgcccgcctcggcctcccaaagtgttgggattacaggtggctctcgcaccaagccaagagtttgcatttttagcaaattcccaggtgaaactaatgcctgcttttctgggagcacactttgggactcagtgatagagaggtttattggtaggatagtaaaataggagttattttctttcacaaaattggcaattgggggaaatttaatcttccttttttcttcagctgtgacttatgtattatgtttattttaggcgtccgtgagcactgttcaactgtggatatcgggaattctggccattttgagggttctgatttcccagtcaactgaagatattgttctttctcgtattcaggagctctccttctctccgtatttaatctcctgtacagtaattaataggttaagagatggggacagtacttcaacgctagaagaacacagtgaagggaaacaaataaagaatttgccagaagaaacattttcaaggtatgctttctatctgagcctataactaacccatgccttttgggaagtcacgtgatgtttcacagtcagtaagtctggaataatacctggtcttgcttcacttctgagttgggtaaagaagtctgtatcagtgtaattttctaatccgtcctgcattatctatggctcttggttcatacctgtcttgaagttctgtcatgttctgtctcttgtcctcagtagagatgctacagcagtggctcgcctcaggcagggcagggcagtggggtggctgtcctgggggcaggcagtaggggcacgctgacgtcagggaagttgaaacccaagagaagccagtaaaagtgagtctcagattgtcaccatgtgctggcagttttacacgctgtcagtaataaaagtcttctccctgcagggcagcctgcctccaataaatacgtgtagtatcaaatcctgtcttccctcataaattgtttggaagctccccaaggacagtgatgaggcactcgtaagtgcttgctgcctagatgggtccctctccacctttgctagattctgagcattcactgagttagagctgcttctgcaaatgtgctgcttctgctaagtggctgtgacttcatgcagccttcacttggtttgtcatcagtggagatgccctgtgttgtcgaaggagataagcccagtaagcctgctgggcaccttttggtttgcaggttcagcaggcagcccatggctttccctgtgtcgcattgaagcagctggctaaaattgatgatacattaaattcctgtgacagatgatcagcttgtatttgtgtaatggtgtacagttcacaaagcttaaaaaaatgctacctgccatttcatcctcagtgaggaaggtgatacacagagagaccaagtgactgtgtccacggcgacggcgctctgcatttcactttagcggttaatgtactctacctatatttttactttatatttaccatatatcttttcatgtatacttggcgtaagtgctttatagtagtcacctaattcactgtcatcttttttgtttcttggaaggtttctattacaactggttggtattcttttagaagacattgttacaaaacagctgaaggtggaaatgagtgagcagcaacatactttctattgccaggaactaggcacactgctaatgtgtctgatccacatcttcaagtctggtaggtgaatcacattagtcttcctggagtgtctcgttccccattctgcactatacactctcagagtgtaggagctgtgctgcccggtagaaactctgccttgcccagtgtgccagttgaaaatatttgttgctgtaagagtacacctgataccatgtgacccagcagttccactcttgggtatatacccaaaagaatggaaagcagggtggtgaaaagatatttgcatgccagcattcatagcagcattattcacgatagctaaaatgtggaaccaactgaagtgtccctcgatggatgaatggataagcaaaatctggtgtatatttacagtggaatattattcagccttaaaaaaaggacattctgacacatgctacaacatgggtgacccttaaggacattatgctaaatgaaataagccagtcacaaaaggacaaatactatgtgattccacttacatgagggacctggagtagttaattcatagatatagaaagtagaatggtggttgccaggggctgcaggggaggggagttatttttacaagatgaagagagttattctagaaatgaatggtggtgatggttgtataacattatgaatgtacttaatgctactgaactgtacagttaaaaatagttaagaggaccaggtgtcatggctcatgcctgaaatccaagcactttgagaggccaaggcaggaggattgcttgagccaaggagtttgagaccagcctcagcaacatggtaggaccccatctgtacaaacaaactagccggggatagtggtgtgcatgtggtcccagctactcaggagactgaggctggaggatcgcttgagcccaggaggttaagtctctagtgagatgtgttcatgccactgcactccagcctcggctatagagtaagaccctgcctcaaaaaaacaaaacaaaacaagacaagagccaaaaatggttaagatgggccaatcacagtggcttatgcctgtaatcccaacactttgggaggtcaaggtaaaaggatcacttgaagccaggagcttgggaccagcctgagcaacatatcgagacccctatctctacaaagaaaatcaaaaactagctagatatggtgggcacatgcctgtagtcccagctacttgggaggctgaggtgggaggatctcttgagctcaggagttcgaggctgcagggagctattattgcactccagcctgggctacagaatgataccctgcctcttattaaaaaaaaatccaaaaaaaaaaaaaagtaaacctgagagcttcctcctcctgtgttaaatttggaggccaagatgtttttgttacttttacaaatgatcaaggacggtgaaggttgggcatggtagctcacacctgaaatcccagcactttgggaggctgaggcggggtgatcgcttgagcttgagaccagcctggacaacatagcaagagaccccatctccacaaaaataaaaaaataaaaaaaaatagccaggagtagtggcatgagcctgagcccaggaggtcaagctgtagtgagccatgatcatgccactgcactccagcctgggcgagatcgagaccatgtctctagagaaagaaaatgacaaggacagtgaacccaagaaagtcataagatgccagctgtgcagcaagcatggaaagcagccagtccaaattaggacagtgtgttttccaagaagaacgatcgtttgtaatgagaatgctttgctttaaataaatgactaaatagctagaagcctagttctaggggataggcacgtctttcttctctcaagaaaatagaaaggcaattctaatttctagtaacagcaaacagcattaagtcatggtccaaatatgaggcaaaccaaaatgtggcttgattgttcagcagttgatctgttggaagcccttgatattaaaaaggttctcctttaagcggcttaggagtcacgatcaaagacctatagaaagagatgccatccttctaggatccttggctctcttgggaactagattcagatagtcataatgtaaatactgcttgagctttctttctttctttctttctttctttttttttttgagacagagtttcactcttgttgcccatcctggagtgcaatggtgccatctcggctcaccgcaacctctgcctcccaggttcaagcaattctcctgcctcagcctcccgagtagctgggattacgggcatgcaccaccacgcctggctaattttttgtatttttagtagagacagggtttctccatgttgaggctggtctcgaactcctgacctcaggtgatccacccgcctcggcctcccaaagtgctgggattacaggtgtgagccaccgcacccggcccgagctttcatttttgaaatcaatgtatgactgaaacactgaagacttactgacttaattatggtttcagaacagaatgaaaatgtcttcggttctgatgaatataaaaggaaaactaaccaagttaatttggcaagtagatggtagagatagaggtggggagtggaaggggaactaaaatcttcacctagcattgttgggattatatggttacatcatctgaagttgacagaccaaaatatagaggcttcagaggtctccaaatagaactaaacatgtaattcagattgttaggaggtagtataaatgagctaaatctcatctttattacggtagagttaatgggtgatgtctaaagttgtctgaagtctataaatcatgacaaattatgatgtggtgattgtattcaacagtctttcagttgcagggataaaaccccagtttaaactagagtaagagaaagaatgtgttggtttaagctcctggaaagtgcaggcaagggtagttggtaggactgcatctagtgttgtaattctgtggtctgcattgtatatttatgcatctcagctctgctttcttcttttcatttatataatttttaaattttattttaaagatagggtctcactttgtcgcctaggctgaagtgcagtggcatgaagtgcagtgcgaggctcactctagcctcgaactcctgggctctagagttcttcctgcctcagccttctaagtagctgagacaataggcatgtaccaacatgcctggataggttttaaaatttttttgtagaaatggaagtcttgctgtgttgcccaggcgggtctttaactcttagcttcaggcgatcctcctgcctctgcctcccaaaatgctgaggttataggtgtcacccaccacgcccagtctcatctctgcttcctgtgttagttttgttctctggtgggctgttttcacatgaccgaagatgacctctagcaggctgtgttctcagcccctcaagtaggcctatgtgattggccttgcatgagtaatatgggtgaccataaacccctgaatgctctggtccacatgggccaaatgggagactggacagcattccattgatgaggaggtggggctggtctccgggagtaagggagaggagcacatgcagtaactgatggtctgctgcaagggatagcagcacagcagttagaattttggaggtaactaccagaactgaaaacagaaatgataacaagtagttgccttaaaaagggatgggagcagggtgcttttgtgatcaaagctcctttctcttactggatttttgtacacattttgcatacatatcttagagtaaaagatagcattttcagccttggtccatttgaggatactcttggcgtggcccgcctccatgctagcaggctctggttgtgccaagttcagttgagcatcctggctcttgcctgcacggaacttccagtcagtgcgtcagtatcacaagtcttgatatttcctatgaagaagaacagtagtgcagtgacagacgaaatgggtgggcaggcagaggcaggatttctgagggagagaagtagctagctttttgcagagaagagttccggcacccaagagagcagctgagagtacaggcaggcaggcaggatgccggtagggcccggccgcacggcgccacagaatcctggagaaaggggcctcttcatggcctctgcattcagctgctgtcaccctccgcacaggccatggccaaaatttaattttcatagtggactctagtttttgagccttacttgctattattgaaataattttcttgtttctttttaaagatcttcggattatgcttcactgaccactgtaataagtttaaagttgagaaaatatggcttgttaatgaatgataggtcaattttagtatgttggtcattttaatattttgccaccagttggtttggatttgatgccaggaggagacagcctcatttctaaggactagtcttgcctttgtgggataagggtggtgtgttctgtgtccttctacatgtccgagcgatctctgtgcagctcaaatgtggtcactgtcttattgcgctgatttcctctccttccatctcacaattgaggcaaaatattgttactgttgaagtgttgtccaataggacttccagcagagacaggatgtctgcactgtctaatttagttgcctttagccacatgtggtgttctgtacctgaaatgtggctggtctgattggatagcttaatttataattttatttaattttaattaacttaaatttaaacagctctgtgtggatagtggctcctgtatgagacagtgcaggtctgttgagaagcagctttactggtgggagtggagggcttggagagggcacgtgggtttcctgctggtatcttttgaccttatttaatctgcccaacatttgcaagtaagttgtgtgtgtgtgtatatataaatgtgtgtttctgtcttcttgtttcctttgactgcatttatttgaaagacactaggtggcagaattactgtatttgattggtttcaagataagagttgaaataattcatctcgtgtttttatataagtaaggtgtgtttagcatgtaaaattggtaatatgtattcacgtactgcttaaacaaaggctatgaattccacccataaaccgaaaatgaagacctttaaatttgtccatttcaggcgtgggtacttcttaaataatacctggttcaggaactagtcagaatggcacccttgactttttgtttcctgcttttcctcttgttgggagaggagggtattcatcccaaagtggtttgcctatttcacattccatctaggataagcagaatagccaagaaagatagctgtcctcctgtttacaacatttggggtaaccagcatccctctcttttggtccaagatagactggtttagaaacagatgatggcaccagaggcccaggaggtggaaacatcagctttgtttgttgtccatgtggctgaattagagctgtctggccttgtagcctcaacacggccttccagctttgctcaccgtgattttcaaggacacatcttgtgctcttccctgcctgccatccagactatacccagtcagggtggcaggagctgctgccccttcctccctgagtcctggtcgtgggtggtggagatgtgccatgacgctcacggaggcatgctcaccccttcctctgtggcagaggggatggctgcacgacagctcttccctgtcctttccaaagcgtctgtggttccactttttggggcaaagcaggaatactggaagagagagaaagtggtcctttctatagtaataaagttgacattgattcaagttcatgcttggggaaaggacagggctactaacaattataatgctgggagcaatggaattttctcatgggtatgtggtaggtttaattttaattatcccagttaattcttagaactgctctgtgaagtatttcccgctttgtgcttaagttctaaaagatcctgtgccaaaaccaagaatgaaaacccaagcattctttcttgcccatcgatctttctctcatcaggccacttcttgggttgatagtggtgagtgtagccgctgccactttcagaatacccaccatgggccccagtcactgtgtggcgtggagaagagatggttctctctgtgtcatagctgaacaagcccagcccagagaggtttctgccctaggagctctcgatggtggaattgggatgcgatcccacatcctgcctgttttgaaaacagcattctttatttccaattcctgcttccattgttccttttaatatttctttgtttagctcacaaaaacacggcttgcggagctgctgcgtgcagctgtagctgtttctctgggtgcagcctgcatccgccttcctgcccgcctcctttcctgcactgccatcgtggtctccgggcacttggtccctttctcttcccctgagtccctttggctcccctgtgccacccttgtgatccacaggctctgccttctttctgtctcagactgctgctcatcactactcgggaccctaggaagggaggttccaccgagaagcatcttctcatctcagccacgttctcagtgccactgttgtctttgttaggtaatggtagctactgtaacaaataaaccaacatttccatggcttcacaccagagaaggttgtttcttggttttatgacaatgtattgagggtgttcttggttcacggatggttttcctccatgtgggaattcggggacccaggctcctttccttcttttggttctgttctccaggccttcacatcctctgtgtctggttggggacaaggagagggaaggtaaagaaggctttgtggccttggataagtgacaggcatgcctttgctggtgttctctcgtggtgacaggtcacagccccaccctgtaaaaggggactgagagacgtcgtcctgctgcttcccagcagcagcactgtggtctctgatgtgttttctgtgaggataaaaacaggtgattccaggatgaggaaagtcagggaaacccttggaaggaggggaccaggcgggtgtcaccatgggattagtggtggcttcagaatgagctgcagcgagtgccatgccttctaaagcttttgctattctgatatgcccacaccatgcccagcaggtgtctgccttgctctccgcagagagagtgatgaatccttctcatgagcctctgtccagttgttcctccctccacctggaagggaccctgggttcctcataacatcccagcggaacaggggaccttctatcctgtccccaagttcatcctcatcctcctgccggcttcctggcccctcttatgtctgcttcctgacgccacatccttctggattctctggaattgaattttgcctttgatgcttatttaaaaatatccattgcaggccaggtgtggtggctcacacctgtaatcctgtgcactttgggaagccaaggtgggcagattgcttgagcccaggagtttgagattagcctgagcaacatgttgaaatcctgtttctatagaaaatacaaaaattagctgggcatggtggcgcacacctatactcccagctactcaggaacctgagacaggaggatcaattgagccccggaggccaaagctacagtgggctgtgatcgtgccactgtactccagtctggtcaaacagagtgagaccctgtctgaaaaaaaaaaaaaaatccattgcatacttcaccgtagcgaaacatgtatgtcttacctttcctttcctgcctgtagctgctcttttacacttaacagccacactaagccagccttaaatgaaaaacaaaccagcacttcctgtgccctcctgcttccttcatgaggggtccctccctctgtgtacactccattctcattgcccatggtggtttgtttccctcttgtttctcaagccatggcagcctgcctcttgccctctttactaaaaaggcctttgcagaggctgcctgtgttctttctttctaggtctctctcatcctaggccctccagcttgattctgtggagctgccctcttgtcactcagtagcttgtggggtcttctctgtctagccacttaattgattgtgttcctcgagttgctgtccatggtctctcgttactgttttctctgtgtttctgcctctctccttggccttggtaggtccatcccctttgtgaccttggctgttgctctcatggacaactttctcttgctggtccttgtagtcctggcatccagcttctcgacacgggacttgtcctgccagtacctcagacttgcacttaaaattgaactagcaccactgtcactctccagggcctcttcttgttaattagatcattagggatgttcagaatcccagcatcatagtatgttcctcctcccgctaccccaggaaccctaaccttacctcctcctctctatctactaggaggtggccctcagagtccgtctcatcttccacctgaacttccctaataggctccagcagctgccaccccgggggctgagtacttcctccatgccttgtgcagtgctgagccctttacctgggttctcctgtttgctccttattacagccctgcgaacagatactgctcttaattccatcttacacctaaggaagctgaggccccaggtaaggtgcatccaaggtcacccaggtagtagacagtagagccacgatctgaaccaggcagtctgattcagagcctgtgttgacactcagccacctagaacacagcttggattgtgggtttctattacctgttcaaaacccctacatcccgggtctgtccctgcacgtgctctgtggcctggctgcatcttccttgaaggcagtgcatgcctcttcactcagggggcccatgcaggaacagagggccccacagaaggatgaggccagtgcagaatgggctggaggggacaatgctgaccaggaagcaagtgtagagaaatcccaggaaacctggaggagccagagacaaggcattagaactcctcgtcgtgacctggtctgcattctctgagtgtgctgcttctgttagctcgcttccttggtctcaggttatagtttaaggcattgtggagccctaaaaagcctgtactctgtttttacctgttttaggaccctttcactttggggatgtgttgattttttttttttttttttttttttttttgagatagagtctcgctccattgcccaggctagagtgcagtggcacgatcttggccactgctgcccctgcctcctgggttcaagcaattcttgtgctcccgcctcccaaatacctgggattacaggcacccgccaccacactcggccaatttttgtatttttagtggagacagggttttaccatgttggtcaggctggtctcgaactcctgacctcaagtgatctgcccaccttggcctcccaaagtgctgtgattataggcgtgagccaccacacccggcctgaaatttaaatcagaaataaaattttgatcccaacagtgatgccaggcagcccagatctgggggagagggtggccttggccagctgggcctttctctgtttcccaagtcttgctgcctctccctgctgggctttgcagcctgtgcatgtctctgtgcctttgaccttgtttatccaaaggagaggatagaatgaagtcatgattcctggagccctgagaaggatgctgtggagaaatttgccggtagaatctagctgagtgtgttgctgaggtgccagcattgtgtgtggggaggctgaccgcttggcctgcctaggcccaggatgctccatggccgggcacagaggccacttggctgtcaggtgtcaggagcctgcagagggcacacagagcctggaccgcaggggggtcctgctttctcacctggcctccttcagcatttctgtccctcagtccttagcaagcccaggagctgttgagtttggcaggtgccgagtgctgttcctgcctgtgtagctgtggctcagtcctgtgggggccccgctgtggcccgagtgcagtgattcgaggcgctgagtgttccctgactccttctccaggagctgtgttcagactttcgcagctcttggcttggagctcctggagggcttggcattgccgaccaatgtggaggtcgacagtgagagaggaggaatgctagctttcttgaccagtccattaaataagtgggatattggccaggcacggcggctcacgccttaatcccagcactttgggaggctgaggcgggtggatcacgagctcaggagttcaagaccagcctggccaacatggtgaaaccccctctatactaaaaatacaaatattagctgggcgtggtggcaggcgcctgtaatcctagctacttgggaggctgaggcaggagaacagcttgaaaccggaaggtggagtttgcagtgagccaagattgcgccactgcactccaacctgggcaacaagagcaaaactctatctcaaaaaaaaaaaaaaaagtaggatatctgtttctgcttagaaaaatcagaattttctaaatgccaggtgttctgaatacgtaagtatgggagacgactcagcctgtttcatttttatgtaaaatcttcgcgtagccatgtggcactggaccgagatgaaagcaaagacatttctccttaactttgtttctaggaatgttccggagaatcacagcagctgccactaggctgttccgcagtgatggctgtggcggcagtttctacaccctggacagcttgaacttgcgggctcgttccatgatcaccacccacccggccctggtgctgctctggtgtcagatactgctgcttgtcaaccacaccgactaccgctggtgggcagaagtgcagcagaccccgaagtaggttcataatgccccacagcccagggcgccagcccagcaccctgtcctgagactcccagtaacctgagctttggccaccgttaaagcattttcattttccattttttgtgagggcttgtgaaatttctgctgcatattaatattcctttcatggacagcatattattgggacaaacatgcggtccagctaaaggcattcaaaatagcagttgctttctaaatgcgattttctttggcaggttctttgacaccattgcatcttgtgggatatgcttgtcatgctctgtggctcctactaagttctagtccttaaattggttccatagccagacatgttgcaatgtcttaacctcattataaagtaaatgtggttctggttatccttagataatgaagtaacagtgtagcaaatttcaaaacctcttggaaatgttattttaccattcaaaaaggcttactaaggttctcgttatgggtggccctctttttgcaaaaggttttcaggcttaagctccatttctaggtgctccaacactccattatttgtatatgtatggaaataaaagctgtgaccacccccaaccctggcccccgcccagctgaatcctcagcacagtatttctggaaggctcaagatcccacgctggggaaaagaagttctggagacaaaagagggcaggtgctgccgtgcctctctgctcagtatggatactggaccttgtgctgccagggctcccagtagggccagttcatggcactcagctggaaagtccactgttgggaggcattcttaaccatccactctgtgccgtatgtagtggggtctggtcattctgttggaggagacagaccagtgacgacatttgaaatgcttggtggatgtcttaggcctgttacgatgactgagcactgtgggggcaggagacagaaagtcagtgtctcctagttctgtgctgctttaacgtgcatagaaatcagctgcggattcagcagatcactccttttctgacagatgggcctgcttactctgatgttatatcagaaagctctgaatctgggaattgtgtcccctgaattggagtaacagaaatgcttagatgatgagtgtttaaaagaaataaaccaaaggtaaatttagtttggaattcagcaagcgtcttcattcagccctctgagggcaaactacagctttttgtaaatgtaggtaaattctgtgactgtttcgtgaccccctctgatccagttttcctttataaccttctgtattgttccttctattatcctgaaataacattaatagattaggctgggcgtggtggctcatgcctataatcccagcaccttgggaagccaaggcgggcagatcacctgaggccaggacttcgagaccagcctggccaacatgatgaaatgctgtctctactgaaaataacaaaaattagccgagcatggtgacaggtgcctgtagtccctgctactcagaaggctgaggcgggagaatcgcttgaacctaggaggaaaaggttgcagtgagctgagatcgcgccactgcactctagcctgggtgacagagtgagactccatctcaaaaaaaaaaaaaaaaaaaaaaaattaatggatcaatggatttttaacctaataattaaatttcaaaaaatatcgttctttaatggtaatgtaaaggtaaaattaagataatatgtaacaagcatgtgagtgtctaaggtgtccccgtggtggaaggaaaaaataaatccccataagtgtccaagatgcccatagagagcagagctgttctggtttaaacccctgctcttagcactgtgtttttccagctgtgggtggtgggggatgagtatctttttatttccatgagatgagaaaaatgaattactagaagtgtgaaatacaaaacacagctgctctttttttagccatagactcagcagccataaaattgctgtatccagttgcagaaattcctgctgcttactcttgaccctctctcggtttgtgtgcatctcctctcaggctggctcccagatgggagctggctccaggcgacactgggtgctctgctccaggaggtccttatgtgggtcctgccctagcctagcccctctcttatggactctgtcactgtgggtttatgattcactctcaatctgtcttacctcttggtgaactgttagagtcctgcctatactttggcgcttgtgggtgtgttgtggtacacatgatgtgttggtcacttcccagctcatcttgttctgagtcaccctagatttgggacattcattcgccaccagtaccgggcggtgtatggcctgagatttgggggggcttgtgctgctacaaattggggctgaatttgagttgacagtggaccttctttatgtctactgctcatatttgaattgcaaatactgcctcttctctttcagaggctcattaccctatagctgtattattgcaaagtgcacaattacagcttgagtgtaagtcacactgcgctggcaggacggcccactgagaaagggcacgtttcctgttcgttagttttcacattgacacataatttacaatacagtaaaatgtacttttctatcaactgtagtcagtaacagcccccctcccccaaccacatcaagatatagaggagtgctgtcacttcaaacagttccctcttcctctgccacatcctgcccctccccaggtctaaccaccaatccgtgctctgtccctctgttcagcccattgcagaaggccatagaaatagaatctataggctaggtgtggtggctcatgcctgtaatcccagtattttgagaggctgaagtgggaggatgacttgaggctgggagttcaagactagcctgggctgcctagcaagaccccatctccagaaaaaaaaaatttaaaaattacaatcacgtccctgtagttcagctgcttgggaggctgaggcaggaggatcacttgagctcaggagttagaggttacagtgagctatgatcgtgccactgtgctccagcctaggtgacacagcaagacgttgtctctggggaaaaaagaaagaaacggaaccacgcggtgtgcagccttctgagtctggcccctttcggtgagcagtgtctaaagttctgtcgcgtgttgcccacgcgtcggtggctcgctccttgcaactgctgagcattgtatggctaggctgtagtttgttttcacttcaccagttgggaaacagagaaaaggcactttttaaaaagtttaaatctgtagaattttggtttttaccagttctcttctaaatcctgagggattacaggaaaagttgttgtatttcagaatattcttagcttgatgtgacctctgtccccgttaaggccctttgccgcaatgggaaggacgtcgctcggtcagaccctgaaggtcagaggggcagtttgggagtgtgtcaacattttaactgtatggactagagccaagagtctcaaggtttataattcccacgtattcaaaaagaaaaaaacaataaagtgagaagtcagtgtagagtgaaataacctgtgttagtggggaagaagtgtttttaaacaggatttccataacgtataacatcaacatgtttagagtggtgatgtttcattgggaaacgaacagtaaaacatgaaagcagggaggttttcattctggcagttggcaactttcacggcagatggagaatttcaaaagcaattgctcaattatcaaacatagccagtgtgagttctgaaataaaggtgctgattgaatgtgcagctttatggtggattttgctattcaggcaagcattttaattttctgcctgttaaattctgttttctttagtttttcatatgtggtttattgtagcttaggaatagataactgagagtatatattacacatacaacattctgatatggcaatatttaaaacaacttgtctgttttagaactagaattaaacataatcatcttcagtattttgcaaataagctcactgccatccagaaacattgtcaatgcatctgttgctccttctagaagacacagtctgtccagcacaaagttacttagtccccagatgtctggagaagaggaggattctgacttggcagccaaacttggaatgtgcaatagagaaatagtacgaagaggggctctcattctcttctgtgattatgtcgtaagtttgaaatgcctgtaaacggggttgagggaggtggggaccaggagaacatcctgtgtagatgacacttgcatggaccctctggaacccagaccgcccggtgtcctgccaagctccatcgaaactaaatctagaatgaatgtttacttctgctgtgacatataattggagaccaggcctggccttccagtcactggattctaagttggactgtgagagtttttgcagctgactcatttatcaaatgcccggctattggctcacgcctacatgatgctgggtatgtttgttaatttgagggaagcaatggaataataataactaatgatttaaaaaacaaagtaagtgcattgactgtagtggggttctgattttaaatttttttaaaaattaataccaggagcagtggcttatgcctaaattccagcaactcgagaggctgaggtaggaagatcacttgagcccaggagtttgagacaagcctgggctatggtgtgagacacccatctctaaaaaaataaaaaataaaaaattatccaagtgtggtggctcgtgcctgtaatcacagctctttgagaagctgagggcggaggatggcttgagcctgggagttcgagaccagcctggcaacacagagaaaccctgcctctaccaaaaaaagaaagagaggaagaaagaaaaattagcctggcgtggtggtgcatgcctgtggtcccagccacctgagagactgagaagggaggattgcttgagcccagaagtttgaggctgcagtgagctgtgactgtgtcactgcactccggcctgggtgacaaggcgagacccctgctctaaaataatttttttaagttaatttgtagaaaaggtgttagatgttctttgtcacattttatgatggattcctgtttaaatgccgttctctttaaagaaaaaaaaataacttgtgggagtttttaaccataaaactagcatcacatatttaccatggagaatttacaaaaaaacaaataaacggaggaaaataaaacctcctgtaatcatactactcagagataacttgctgttagattttggtctagatttaatactttttctatatttatattaaaaatatttaaaacatatgcatttctttgtcacaaacatggtatcttatagatactactgtcacatagcaaaacagtgttaaatattctgaatcagaaaaggaagccgactctccaactgaaagaggtgttatcctagagactttttctggtgatgacaatttattaatagtcactttttgctttactttctctattgaagtagtttttctattttgttctacttttaaggataatataatttataatgctgtttttcacagaaatataagaaaaaagatactaattttataagttaataaagtttgatcatcccaaatccaaaaatctgaaatccaaaatgctccaaattctgaagctttttgagtgctgacattatgttcaaaggaaatgttcattggaaggtttcagattttcggatttagggagctcaacaaataagtataatgcacatatttcaaaacctgaaaaaaatcctaaattcagaatacttctgatcccaaacatttcagataagggttattcaacctgtactgtcagatgatcccaaatgaaaaatattaatcgttaaccaaatatcaaggaattgatcacattttacagtttctgcctaggattatgaatcaagatgaaaaggctctgcatgtttaaaaatatatatttttattttcttataaatcttaaatatctacacttaagatttatttgatatgtgggatccattcatattttggattcaacagttctgtcaaaactgtggcagtgataggggattctttttttcccactgaactatcacaaaattggaaaaagagtaattggagaaccccactggcttagccggcccgaagcccgggagagggcaggcagtgctgtggatggggtcatcccagcgcaacgctgcccctgctacctgcggatctcgctgaggcctgcctttgtcctttgacccttggccatttgttagtgtctctgagagctggactgctgtaccctacttccccagggggcctaacttcacacagcctctgccgcagtgcgtggttggaggtgacggccttggtaaatcgagtttcctacctcctcaattatttgtgctcatacactgtatatttttagtgaggtttatatttgggatgtgttttctccttcttaccctttctggcctttctatggcattaatacctggtctcttcttgtgtacttgaaaatgaatctctcatcatatttttccttagtgtcagaacctccatgactccgagcacttaacgtggctcattgtaaatcacattcaagatctgatcagcctttcccacgagcctccagtacaggacttcatcagtgccgttcatcggaactctgctgccagcggcctgttcatccaggcaattcagtctcgttgtgaaaacctttcaactgtacgtcttcatcctgccgactattgccagttgcagttttccctgccttaaaaatggagtattgaaatttttaactttaatttctgatttgcaaaatagtcatcttttgttcttttccttcttgctgttagccaaccatgctgaagaaaactcttcagtgcttggaggggatccatctcagccagtcgggagctgtgctcacgctgtatgtggacaggcttctgtgcacccctttccgtgtgctggctcgcatggtcgacatccttgcttgtcgccgggtagaaatgcttctggctgcaaatttacaggtattgggaagagaaaccctgatattgatttatattgaaaatttagcaggccaagcaaaacaggtggctggctttttcctccgtaagtatggtcttgacatggtcaccgatagaaacatggaaacatctgcaaacttgccgttactcgtgtgtccgatctgactgtttcttgtatttttttctagtctgcccttactaggatgaactgtacacatcagttcatcctttttaaatgagcatgaggttattttgggttgttaggtgttacaaacacactaatgtgtttttgtctattagagcagcatggcccagttgccaatggaagaactcaacagaatccaggaataccttcagagcagcgggctcgctcagaggtaatgctggaaacacaggtcgtccttgtgttaggacaacccaggatataaaggatatagatttgtacgggaataaattcacaggacaagaaatcgatgtgccttataggtgggtttactgcagaagtgccataatagaaccttcctacttttaaaacaaccagatctcactttctaaagagtaaaggatgaccggcaggatcacgtctgtgacgtgagtggaggcagtttgcactcctggtggctgtttgagaggtagcatttagaatgcctgtattcactgtcctgtgatgagtgggaaaataggttatcaggtttatcttagcaaaatcaaagcatgtcatctaattgctaaacaagagttggcaaatctgagagacattactcaatccttggcatgcaggacttacatctgcatcctgttgccattttatgtcttcaaagcatttaatcatttagttgtgtttgcaaagtctttgagaagcctttgtcagaaatccctacatctcctatgtgagtgtatttccatgactgcagaataagttaaacttttacctttttccttcccttgcggggcggggtggggggcagggattgtgtgtgtgagagggagagagagacagcagagaaggagaatataattatcatgctgtgtactttgagctgaaactgcaaaaaaggaaaaacacacaaaaattattatgcttttcagtctttagagtaccttgtctattatgcttttcagtctttagagtaccttgttgatggtgtttttaaatgggattgggcacaattaggtggacagtttgggatgatttttcagtctgtagggccaagctcttttgtaatttgcattatgaagttgtcactctcatagcagatggcgggagataaactattattactttttgaccctagacttagtcttcagtccagatgagggagattaaaagattataaatatcttgtgccagatgaggtgattttattttgaaatgaccatgaattcctatcagttgtcttactgggatatttgatagtggaatttgtgcatttgagtcttagatgatctgttttacatttattaagaaagcctttattagcttttatactgtgtattgcctgttgcagtgtttgagtataaatgaaatttctggaaaatattaatggagtacaaactgtgatacttaaaagtaaactagggcctgcatttgtatcatgacctgtttgagtattgatgagaagatagctgtgaagaaaaaggtttaaacaagtgtattttcctttaagaagccactaatagtgcatctccttagagtgtatatttctagaatcctagtgtgcagagtttagactaagactaaaaaaaaaaaaaaacaaattatactgtaatttcatttttatttgtattttagacaccaaaggctctattccctgctggacaggtttcgtctctccaccatgcaagactcacttagtccctctcctccagtctcttcccacccgctggacggggatgggcacgtgtcactggaaacagtgagtccggacaaagtaagtgtccagcgtgtctgcatgggaggcacagggcgctgagtgcctctgtcacctgtggcagatacagagagtgcagaggaggtgccgtggacccaaggagttctggcgctcggctcggctcagtgaagctgtggttagagacgtggggggccatcaaggtctgagggagccaagcagtgctgatgtgggacccttttggtaggagtgtggggtgagtagttagtgggtgaatcaaggaatagtcggccgtggcctgcaggcccctgactgcacaggccttcaagcacatgtcaatgccgttagcctccctccatctcctcataccttctggccacctgtgagttgcactgccactgccagccattctggtatgttgtcagcacctccactgctcatacctcatggttagggaccacctggagccttggtagagccttggtagagccttggtactctactttcctggacaaagttcagcttatgaatatgaatttagatttcaaaaaccagcagcccaagtataagaaagcgaaggttcagtcctgccttcttaggctctattcgctaagcacctgccctgccctggttgctggggagagatgagtaaagcagacaacccaggagaggatggcaaaggggccgctaacccttagtggtttagctatatttggaaggcctattggaagttcaccaggtgaagggggaggctgtgagggtgcccaggcaggtaacagaagtccaaaggggaaaacctgtggtgtggtgagccgtatagccacagcctgccggccggcagccctctcagcctagtgcggtgttcccaagcactggcctaggcctgtagctccagggatgtgaagtccccttgaacgccgcccatcatgttccccttatccatttttttcttcccaggactggtacgttcatcttgtcaaatcccagtgttggaccaggtcagattctgcactgctggaaggtgcagagctggtgaatcggattcctgctgaagatatgaatgccttcatgatgaactcggtacggggggagcagtggaggcaaggaatcctcagcttttcttgtgacttccaagtgggatttgtctcatcatcatgtgacccacttgttgacaacacatgttggggactccagtctgggcagggacgggatgtcggagagactccactctgaatggggccgggaagtggggaggactccatttcagatggggtcgggacatgggggttatgctgatcgagacagaaaagcacattgtttcagccacattagaatccacggaggtgttgttttgaaatccagctggccccaaggctgggtgtatggtttgggatgagaactatctggcctccactggaggaacaaacacaggatgttatcatctaagctccatggccaagacagaatggaagtcaaggttgcgtatttgccgtagacttcaacacagtgtcgtaatgcgtgacgtcaataacttgtttctagtgtcttggaagttgatctttagtcgtaaaagagacccttggatgcagcgagatttcctctactcacacctctgttagatgtagtgaggttcttcaccccccaaccccagatgtcagagggcaccctgcgcagagctaggaggccatgcaaagccttggtgtccctgtccctcacccgtgggcaggtcctgtgagcagtgggggggccacctcttgggtatggtgcagccatggcccaagcagggcttcttctcagacctactaggacgggagaaacctcctggtgctttagccctgcgttgatatgcagcaaatgggagggaagtgggcacctgggaggacaaatgcctgtagaggccgggagtgacggcaggtgttcatgaaaagagaccttgtggggagggcaacacaacagtgtgttctgatgtactgaagagctcaactgaaaacaacaggagaattagcccaaaatccatttactaaaattgtttatctttttttttttttttgagacaaagtctcgctgttgtcccccaggctggagtgcaatggcgctatcttggctcactgcaacctccgcctcctgggttcatacgattctcctgcctcagcctcccaaatagctggtattaacaggcatgcaccaccacgcccggctaatttttgtatttttagtagagacgggatttcaccatgttggccaggctggtctcaaactcctgacctcaggtgatccgcccacctcggcctcccaaagtgctgggattataggcctgagccaccacgcccggcctaaaattgtttatcttaagattcatgcagtgaaagctaacttactgagtgataaatttgcttagtgatctgtttattaggttttccaaatttgctaattgggctttgaacagctgtaaaagttctgactgtaaaagaaagcttcaacttttggcattcatgatgcttttctgagtattaaactaagatagatgttttacctgaaggatcggccaccaatctttaaatggctaaacaaaagggttgctaaaacataatccaaattgacataagaaataccatttttccaaccaaaattttggcattcatatggctacttttacgtatttcagctgcatttgaacatctttttcaaactttagggtggttggtgtatcactgaggtcttggatgacactttagctttgattttgtttttatgaattaaaattgtcataccaaaatttttatttcaagcaaatccaagagcataaaaaattaaaatattacttaaaatactaagagagaacagatatatattttactaagcatatgttgaatgaaattgttcaaatatttataacaggcatagagtagaattttcttaaaaatatttttgatggtataccaatttgtattttctcagaaacatttgccttattcttttttctgttgtgtttttcttacctgattgaaagctcataatctgttgttattgtttgttaacctttaatgctctgatttcaggagttcaacctaagcctgctagctccatgcttaagcctagggatgagtgaaatttctggtggccagaagagtgccctttttgaagcagcccgtgaggtgactctggcccgtgtgagcggcaccgtgcagcagctccctgctgtccatcatgtcttccagcccgagctgcctgcagagccggcggcctactggagcaagttgaatgatctgtttggtaattaaaattaaaatttatcttatttttaaaaagcattccagggccagtatagtactttgcaccaagtaaatgtacaataaaggcagtggatctaatacattgaaagcgtttacagaggtagctaaagagcagcacgggtgtcctcggctcagaatttcttcctgtgtgtttgccactttgccattcattgacatggtcatggacatagggctctaagcccttgaggaaggctgggccagacctcaggggagatgcagccccaaaccacgtgcagtcctgtggacggatgtgtagatgtgccactgaggaacaatgtcttgagctttcatcagattctcagagaattgcttgactgcctttcgaagttgatgcatctgtgctcacgtttgcacccacccacgaggtccttctgtttcaggggatgctgcactgtatcagtccctgcccactctggcccgggccctggcacagtacctggtggtggtctccaaactgcccagtcatttgcaccttcctcctgagaaagagaaggacattgtgaaattcgtggtggcaacccttgaggtaagaggcagctcgggagctcagtgttgctgtggggagggggcatggggctgacactgaagagggtaaagcagttttatttgaaaagcaagatctctgaccagtccagtcacttttccatctcagcctggcagtaagtcttgtcaccgtcaagttattgtagccatccttcaccctcacctcgccactcctcatggtggcctgtgaggtcagccaggtccccttctcatctgcacctaccatgttaggtggatcctaattttagagacatgaaaaataatcatctggaagtactttatgtcttaagttggcctggacatgtcagccaaggaatacttacttggtttgtgttagtgcttgtaattcgcccccagaatgtgtacacgttctggatgcattaaagtctggcctgtatccttaaagggccatcgctgtgctgcctgccctcagcaaggacacactttgcagacccacagaggctccgcctccacctcacaccaaagaaagggaggagtccaaagggcatcagtgccattactcacaaaatgataaatacacccttattctgaaccacgtggagtcatatggtttgtgatccctgtccttcaggtttcagcttagtggggaagtgggaaagtcagcgtgtgatcacagcacagggtgattgctgctgattatattatgtgcctgctgtatgcaggatgaaatactttatatgcgtcatcttatttgactctcacaaccccctgtgagataggctctgttactcccatttgacaggtgaggaaagcaaggcttagagaatttcagtgacttgcccaggtcctctgagctaggaagtagccattctggcatttgaacccaaggcctgctatccctagaacccacgctctcaaattcaacctatgacagaggcaagccctggtgctgtgggagccccaaggaagagcctctggcctggtggccacgtagcccaggagagatttctacaggagcccacagcgctgaaggagagagaggcagcagagtaagggggctttgtggcagagaggggactggcactttggggaataggtgggtcaggactgaatgtaatggagccatgtcagagctgtccttctggaagggcaagggcacctggacgcgctgcccctcagtgctttggacggttccacaactgtgattcacacggcttccccaaacgaaggtacacgagtgggcattctgtgactcggtacttccctttaggccctgtcctggcatttgatccatgagcagatcccgctgagtctggatctccaggcagggctggactgctgctgcctggccctgcagctgcctggcctctggagcgtggtctcctccacagagtttgtgacccacgcctgctccctcatctactgtgtgcacttcatcctggaggccggtgagtccccgtccatgaacggtgggttcctatcatagttcctgtctgcttcaccatgtttttattttgtgctgcctgtttgccaggtactaagctaggaattggggatggagaggtagataaaatatgcatcaggaagggctgggccccatctcttactctccaatatattggagtctacactggaatttaactggaatttgcttttttagtcattttatttagattttgaagtttcagctttcatcaaaaatacctctaaactttatgtctctgtgatctttggtcttagctgttttatgtatttagtcttatatgatcataagattaataacattacattcagaagattatttgttttctgtcagagttaaaatgtttgtttttatactgcattgtaatattaacgtactgtaaaataaaagtggcttgttcttttcaaggaacagtatcctcaacaagggtcattagccacaatttttaaaaaattggacgtcatagtttacatgttagagggcgttttgaagctttgtatttttaaattaaatgttatagagtgatgttttcatgtttcataattgttttcatctgtgcatttgtagccaacttgaaaacaaagatccagggattactacttaaaagccagacttcttggaggttatagtgatgattttgatagtatcttgagccgtctcataataacctcagggtgagagatggccaacaggagacagtcgagggacttagaaatctgaatgaaatctgaagttcaaatcttcagacatataccactaaccaagagattggtacctcagtctagtattgtctgtttgtctaaaattggttctaaggaatctaggctagtctgtctatccctttcaacttttgtgaggctgcacaaatgtaaaatgttgaataaaaagcactgatggaagtgtgtagaaattcttctctttgttctgttgtaattttagttgcagtgcagcctggagagcagcttcttagtccagaaagaaggacaaataccccaaaagccatcagcgaggaggaggaggaagtagatccaaacacacagagtaagtctcaggacccatttttttcttacatgttgttcctccaggacttaaaaatcattcacagagacgtgcaccgcggtgagtgtggactcctggaagcgcaccgtagctccgctgtgtcctgctgctcctccctagctgtcagggaggctgtagtccattgctttgccagctcttttgtttccgagtgaacaccttatccgtacacatgcggctgtctctgaccctacagaccagctgggatgccactgggggagcgctcccttccccccgcacttcccacactctgcagttattctgagatccttgagggcagggaacaggtttgtcttctttgtgttctcagaaattaatgctcggcctctggtcagcaagcaacaaccttttgttgagtgataatgaataaataaatgtttcccacatgagtattcagtaacctcagtgtcaggttcagccatctgttttggtggatatttaaaagaaaattccgcttttcctacagaaaaaaaaaaaaatccaaatcccagtgatttaagccagttatagacttagacatatactacggcttttcatgcactttcctcccaattctagagtaggtattttactaggaaaatggtggcagtgcctgttgggaggaagattctttggccaagtgtcttttgttcttgccagggcccctaggctgctggggtgcttcagcttctttagcccagtgtctggtggggaatggcccctgttgcctgtcccacagaggtgggggtgcctcacctggagcctgtccacacattttacacagcacgcttacctggagcatcaggcatcttttccatgctctgtggctcaggaaacacgccttttcaatcatgagtgcaccagtgcttttgggctttttctccccgcttttgtgcaatcctggttgtggatggagttttcctgtctttagtcttctgcatagtacttttctcttctggttcccggttcaaggttttgtaattagagaatgacccagaagcaatggcattttaatgcacagccaaggacttctctgaatttgtatctcaaacctctgtgggtccttcaggcttcagtttgtgatttcatgatttcttgttgctacctaaggaatatgaaaacacccacctccctactctgcatcttccagccgagtggcacctcaggctgtggatcctgtgcttctgtggtgaggataagaatagtgccaaccgtgtggattgaaatcaatcagttaatccctccatgtaaagcacctggaacggatgacagtcttgttatgaatactcaacaaatgctatcatgatttttagttagatttccattgctttaaaacagttgagacatcttggcggtttgagttagagcaacgggccctgaagtgggttctgtttgggtgaagatgattatgcttattccccatggccctctttaggcaagagtgggaagctttctttgtttttttaatcacctcgataggacgttacttcttaaaggtcatccaataaatattaataggccgggcgcggtggctcacgcctgtaatcccagcactttgggaggccgaggcgggcggatcacgaggtcaggagatcgagaccatcccagctaaaacggtgaaaccccgtctctactaaaaatacaaaaaattagccgggcgtagtggcgggcgcctgtagtcccagctacttgggaggctgaggcaggagaatggcgtgaacccgggaggcggagcttgcagtgagccgagatcccgccactgcactccagcctgggcgacagagcaagactccgtctcaaaaaaaaaaaaaaatattaataaagccaactcgttagcgtggggcttaattgcttaagtccaatgagaagtccttctctatcctaggaagttgcccaaactgtagaatctcgtggcctgtgggtaatagccacgtaatacacactcactgcctcaacaaatcatattttagtaggtatgatattctagactcaagacaccattctgtggatcttcccaagggtgtgaagtgtccacagcgtctgccttgggagtttccatgcccaccagaaccatgccccaagcccctcaagcactctgacctaggaaagccagtgaagcaaggatgacaacatggccctttgatactagctgagggacagacacaggtcctgggagaccagagaaagacgaggggcagaggaggtgtcctaaaggaagtctgaggctgaggagccacaggatggcttccagctgtcacaggctgctgctggccttatcacagagagtgggccagagggctgggaaccaaggccagagctcaggttcaggaccattccagcaatcccagcagaaaatggggagaattgtatggtataggcggatatgaaggtagaatctgcaggccttcagtggccaactcagagtctaagtggattccacagttacagcttgagcagctggttgtaggtcatgctttctacactgggcatataggatgtgttttttaaaaagtcctctcttaaccgttgcttgtttagatcctaagtatatcactgcagcctgtgagatggtggcagaaatggtggagtctctgcagtcggtgttggccttgggtcataaaaggaatagcggcgtgccggcgtttctcacgccattgctaaggaacatcatcatcagcctggcccgcctgccccttgtcaacagctacacacgtgtgcccccactggtgagtctgctcgttccttgcagaagaccaagtacggtgaaaggcaccggtaggccctgggctgggcacacgtgagagggcgggacagaatccccgcagcccagaggctgcctgctgtggttctggtgcccactgtggttctggtgccaggctgctttcctcaggcaccacgtgtggaggtcgctagtagaaatactgggttttctaaaatgaactgaggccctacatccctaagagattagtgttagacctgattctagagcaactagaccactttgcttaatagcagaccagaaaccacaccccctcgagtgagtgagattttcctttggagataattcatgtttttctacacagttttgcagttgtcttcagaattggtttaaagtaggtgttattgccaggcgcagtagctcatgcctgtaatcccagcactttgggaagccaaggtgggcggatcacttgaggtcaggatttcgagaccagcctggccaacatggtgaaaccccatctctactaaaaatataaaaattagccaggtgtggtggtgtacgcctgtaatcccagctactcaggagactgagacaggagaatcgcttgaacccaggaggcgaaggttgcagtaagccgagatcgcgccactgcactctagcctgggcaacagagcaagactccgtctcaaaaaaaaaaaaggtaggtgttattgatcagaacccttgtttcagataacatgaggagcttagcttgaggagagtgagggttgatggagggggactgacttctgcccagtgaaatggcatcatctcccaccagcccgctgaaataagatgatggggcctgttccttagggcctgcagcatcctcaggcaggaaagaaaggccgacctggcagggtgtgagccagcaggtgtaggtcagggagaatggagccaggtcccagggaagaggcttgtggctgcctgagaagggtgcgtgcctgcctgtgtgtgtgtgtgcacgtgtgtgtatgtatgctggagagtctagggaggcttgctccaaggacgcagtattgtttgatcctgagagataaggattctgccgcagggaatgaaggtattccagatggcgggcttattccgaagaagaggccagtgcctggcggtgctggaagcagttgcagaacagggagttgtaggctttcctgggaagagagcagcaggggtgctggagaagcaggccacacttgctgcatggggttgctctcggccccactcttggtgcacagcgagtcactgtgggttcattagcatctggttatgagacagtaactgctcctttggaggggctcgtggagaccatgcaggagggcacggtcttgaggtcatgccgtccagagcacacctgaggataggccaggacgggctgcacgctgtaggtaaaattcctccagcaagctcttcactggcattgaggagttccctgagtgcggtcatctggaaggcagctgtaacaggcactgcagtctctccctgggtgggtaccagagaggagcataggggagcataaccgatttaaagagagggctttcctgtggtgaggtaagagattagctggtcattatcatagagccccctctgcctttgtgcagatgggctgtgggaatcctggggttccgttgggtcctttgtcacctcactgaaggcatgtaagctgagctggccagaccgtgagctgatcctgccacttgaacagcatcaagcctgcctctggattcttctgtgcatggcacttgtctgagcacctcacgcacagagaactggacttcagagtttacagaaataagctgtatggttcattttcatgcctgcttgccaataaacatatctgagctgaacctcattgaacgcctgcctttattctagcacagcacctgctgtttgtgggcgaggggtgctgtctctaactcctgcctgcttctcccagcactccctgagtggggtgtgccagcagcctcaggatgaggacaggaagtgggagggcagagcagatttgggagggccacttgatggggaaggaagtcccaggaagcagttggagctgttttctgggggagaaggtgccagctctgggacagtgttggggtagtgaggagggagcccagtggagagaagtcgggcttcctgcttcctcacagtatgtctgtcctgactcaactcggatgatgtcacttccttttcatcttctcaggtgtggaagcttggatggtcacccaaaccgggaggggattttggcacagcattccctgagatccccgtggagttcctccaggaaaaggaagtctttaaggagttcatctaccgcatcaacacactaggtactcttggggcctctccttcaggtcaccattgtcggacatctaccgggaggaaatccagagcccccagtactgggatcttctcatttgactccagaaaagatttaagcatgataataatacaaacctatgtgaatacattttgcagtgttggcaaaactccttttatactgagaaaatagatcccagttcctgtgttttgtggcttgaatcccagctttgtgtattccgggcttgtttgaagtcaggaaaggttcatgtgtagtggacaacgtgagaccaaattctgccttagattttgcatttaggctaaacagtggcagcacttgtctcagaatgttttcttgtgttcaccagtctgatcctgttgtgtctcagtggtccattttctcatatgggaacaagcagacgggagcagatggagtcaggtttcttggcactcgccttccccagagcctagaggcagcatggggagaaagcaggcttggggctcagacagtcctggtctgcttccagccctcctacctgagcagcgcagggcaagtccgtctaacctctagagaccctcagttttgtcatatgtaaaatgggggtcgtgtctatttcatagaattgttgcagatttagaaattacatttctaaacaaatgttaccccttatttctaaataagtgtctaaatgaataagtcaccacttttgcccctatttgatggcaagaggtgtgatcttgtggtgggactgtaatcagtcagttctcagtgactgtgccctgctgtggtgtttcctggaatgttcctgtcttgtcctagaaagtctggcaggggcaccctgactccactgtccagtcctctccccagtccctcgggcttctgcagatttgaggcttgtttggatcccagaaggttgtggcaggagacaccttgcctctactttcccctttataattcaatgtccaaagagagccctgagcaggtacctcacgccagctgcctcacggagctcctcctcttcctggctgtgaggatcggtatcagtggcctcctgctctctcccccttgcctaacacgagcacctttgcttacttgggtgcccttgctcttgaactgcccatcggacgtgcgtgacccaagactgtgccgcagtccttgccttgtctgtgctcattttctttgttcatttttttccctgtaacgtaaattgttatatttgtctgtatctgtgtctgaatcagtcctgcacgctctccttctctctgtctcttgttctttctttaccccgtttatcacggggaccccgatgtccattgctctagttctcctgtcctaagcaccccatcccgtctctctggccttaccacaagtggcgtggctgcctcagacatcatgatggggacatgaagcacagctgtcagaaacaactgttcgttagatacactcgaatgcagctcatcaatagggatggagggtctgtcggatgtattttcactgaatccccgttcctaccttgatacactctttttaatctattcttctagacaggtcagaggaaccattactttgacttttaaatttttagcagctttattgaggtagaattcacatactacagatttcacccactctaagcggacagcttggtggccattagttttatccacagagttgtgcagccagctgcacagtctcagggctggactccagggaagattttagcccatttagtgagtggggcagaagtggccctggccctgcacgaggttgcctgcatgggcgtccctgccctgtccctgtgtctgctccactgggggttgaccaggctgccagggccgacttgggcctgtgccacctgcctctcatgtgtctcggacagtgcagccgatgtctatacttcggtttcctcaatgatgaaatggaggggatagtgttccccgcatcatagaactgtgtgaggtttaagggactcactgcccttggcgtggagccttctccaggggccgtgctgtgtcggcgtagctgtcagctctccgttacaggcttgagaagggttgacactctctcatgtaacatttatatttctaggctggaccagtcgtactcagtttgaagaaacttgggccaccctccttggtgtcctggtgacgcagcccctcgtgatggagcaggaggagagcccaccagaagtaaggccacaccctgtgctggttggcacatgggcagttatggccgcttgcaggcctttggtggggaataaaataaggcagcaagctggtgttctttttttctcttaccttatttttgaaagagtagctgaatggtgtcttgactgatattccagagcagggacaaagcctgctgaggtctgggggctgcgattaccaatggctggaatgcattttattacggtgcattccatgttaaggatcaatacgattgtgccctttctggaaaatatcttttagtttatcaatattcagaggagtgtaggttgaattaaaatgaaaaggcactttataaaggccatgagtagtacctggtttcatttttctaatgtcttgcagagattttatcaggcttcttgaagtgttcacgtacattacgctaacacgatattaataataactgtgctctggtacagcggagccagcagaatgggaagttgtggaatgcaggcccttgattctgatagaaggtgtggtttgaactcacagaaatgacagtttggagggtagacatatgtcacaagtcatcaagattgtctttaaattcatgcatagaagctaacagggtgtcataagcaaggcctgtaaaatgtatgagggaattcaaagataatttattaaaaagtaattcatgtttggagttttgtgcccaaaggagtccttgatttgaaaaatgggcttttgcccatcagattgtttcagggcccgtgtgtgcggaggccctgccttgtgccccgtgagctcagcctgacagaaatcctttggtagcacttaaggctcctcttcctcccattgaggcagggaagactctgggttctgcaggcagaggtggttgtgggtgtcttgctgctcttgttgacatgtgggctctccttccaggaagacacagagaggacccagatcaacgtcctggccgtgcaggccatcacctcactggtgctcagtgcaatgactgtgcctgtggccggcaacccagctgtaagctgcttggagcagcagccccggaacaagcctctgaaagctctcgacaccaggtttgcttgagttcccacgtgtctctgggacatagcaggtgctggggacagtgggttccccgctgaagcgtccagcagcttcaaccaggccgttttccttcattgctagaattgaaaacaccgtccgtgtggcctgtgcaggagatgcagacccaaaggtggcctcctggtcagtgagaagctggaaacgtgacaggaactgacgtggggttattgagcatttaggggaagacgttagcagagcaggaatgagcaggcaactagtagaacacccacttaagggctcacggacaggtgctcacttaggaagtgagtttcatttggtattacaccaggttcctttaggcaaagcggagggaaagttctggtgtttttcacttgtaagattttgaaggaaacaaaacactctttaccttttttctaaaatgtaggtttgggaggaagctgagcattatcagagggattgtggagcaagagattcaagcaatggtttcaaagagagagaatattgccacccatcatttatatcaggcatgggatcctgtcccttctctgtctccggctactacaggtacctgagggaaagggtgcgggggagcggttgtacttgggctagaatgagagaagactggcatgctcaccacaccagtgatgcgggaagacctgagtgtggtctgagttggaggctgtggtgctaaatacgctgcccctttcataagcaggagtcttagtcaggcccagggaggaagtaaaatctggaaatgaatgagaagcattctctcctgccagtcaagaaatgagaagcgaaagaattctcacgggctgtaagaccagcaggatttaaaagttgaattagttgcttatgttaagaactcaaccaagttcatctacacaagctgaatctccagcttttcctaagaaaccatgtgtggcagtggctgcagggcagggcacagctgggcctgagcaccccgctccctgcacctctcccctccctgggccctgcctgtcactgcccactctcccaccaagccttccggttgtgtgcctgccctatcacaggcatcggagcttgtcacctggtttaaaagaagagagttgtgtggggatttgggatgcacgtttttcactcaaaagtattttagcgtagagctctgtgattccgtagctatttaggagtttaagcaccttgaaggctttaattgcagaaagttctatgtggacgtgcaatgtgttatacgcagtgtctatgagactcaaatgtttattagggcgttgaagtaaactgagcacttggagggccatggatccagccttcaaggagctcataagtcaggaggacccaggagcaatgacctgtcatagaaggcagaaaagaggggcacagaggtgggtgggaggcatacacaggcagctcctggagctccaaggggagcaagtgcttccagggaagggggcgtggaggcccctttggaggaggcaagttgatctggggtctggcagagggttagctggggacatttagcgggaggctggtgcccgggaattggggggatgcccagcagaaagacatgaggaggctggcctggggcgtgggggggtgtgaaaggttaagtgggggcattatcctgctcccgctcctgccggctgtatctggtcagcctgggcaccgaggtggggttctggaaggcactgttcaccaaaatgcttatctgggtcccccagagagcttgcctgcctggactgtcggctcgcctgcaactgctgactcctaagcttttgcagctcagcccacaaccagttcctattcacagaggtgggagctgaggggtgacaagtgactgctgcagtcttatttgtcatagagaaaaagtgacagagtccagcttgcccactggccctgccagcttaactggttataaagtgacaaatccccaagacccacagggctctgcacaacctgggccctcctgccagtggcggcgagggcaggtggctcacggctgggtgcctgtctgggcaggagctgggctggtatggggtgggcctgcggccctgcccccctgtgcagatcaagactcagggtgctggtgttcacaggtgccctcatcagccacgagaagctgctgctacagatcaaccccgagcgggagctggggagcatgagctacaaactcggccaggtcagtctcgcgcccccgccgcctggcctctgtccgtttctgtcctcagactttggcgcttgacacacccaggagaaaagctcagtgcactttttaaatgaaaggaagttttccttttttttaaaaaaaaatttaatgttcattgtttttatctgttttattcctaggtcccgcaagcagaggaagcattagttttgtttttatttatgttctgtattccagaaagtagttaagagacctcacatgtagcgatagagatgtgtgtaagagacagtgagagggcgtgacttggacttaagcaaggaccgtgagacacaaaaaggggggtgaggacagagtggagtcagctgaaatgctcaggaggaagtagacgccatgaagggccatggtatggggggccgcaggcgtggccgtgagtgtccctggggccagctcttggggggctccctgagtgtccctgtccctgtggccagttctgggtgggagccccgtgtgcaggcagacagctcggccacttcctagcaggtcacattggtctgtgcttctgtttcctcctcagataagtgaagggattcaagggtctgggtgtggtggctaacacctgtaatctataacattttaggaggctgaggcaggaggcttacctgagctcaggaggttgaggctgcagtgagccatgattgcaccactgcactccagcctgggcaacagaccagtactctgtcccttaaaaaaaaatgtaaacagaaacgtagggccatttgcatatgatggcacatggcgtggagccctacaggtgtatgctgggcggggcccggctgtgctggccgacttgcacctttccctccaccccggtgctgtgtctttcgctcaccgggttcctgatttagtgaaagcagttgtgcaggacagttctctttgtagcttttgtttctgtggaaatgggtcagaatatggtgtttagaaacacttatgagctctgagagtttcctcttctgagttcctggcctgcagccttcacagcagaaaccctgtgatgtcacaagcctgtttctgttccctgctctctgcctgtactgtcctgttttgtgcctgccggtttcagtgacaggaagcagggagctactggaccagcctgtatttttctagacatagttggaaaaagaagtcccactcttctgtcctttcacctttgacagatgtttccaccccaagataagtgaaaatgaccaataggatgcactgtatttttcatgaaagtgtttctgaagggcaggctgagagtgagaggcctggggctcactgggtgcctctggccttgtcctgggcccagggacactggtctgtgcccgaggtattccctatccccccaaccccgctgcatttggccacatccttcaatgtttgcgttgtgtccagcgtccgcaaaccaactgtcatgggatcatactggggctgaagtacggtcccacccctgccctgtctggggctgaagtacagtgccacccctgccctgtctggggctgaaggacagtgccacccctgccctgtctggggctgaagtacagtgccacccctgccctgtctggggctgaaggacagtgccaccccttccctgtctggggctgaaggacagtgccacccctgccctgtctggggctgaaggacagtgccacccctgccctgtctggggctgaaggacagtgccacccctgccctgtctggggctgaaggacagtgccacccctgccctgtctggggctgaaggacagtgccacccctgccctgtctggggctgaaggacagtgccacccctgccctgtctggggctgaaggacagtgccacccctgccctgtctggggctgaaggacagtgccacccctgccctgtctggggctgaaggacagtgccacccctgccctgtctggggctgaaggacagtgccacccctgccctgtctggggctgaaggacagtgccacccctgccctgtctggggctgaaggacagtgccacccctgccctgtctggggctgaaggacagtgccacccctgccctgtctggggctgaaggacagtgccacccctgccctgtctgggatgtttagcccctagatgccactggactgagccgctacttgcttttgggaaagaggggtgggggttaggggtctgggcgaggggagtgcaggggctcctccttggcctgagagctgttcatacagactcctcgcccactccctgcagggtgctgggtcccaggggggaaatggcccttggtgccaagaacgtgagttggggctagtgccagtgatgatggagaacagctttttatgggcacacagcccacagcactgtgccaagtgctcgaggcttcccgagaaccaggcagaaaggaggacagtcgaggtgtgctgactgcgtggtggctgcgtgatctagagcgcgggtcacaaaggcgcgagggagctctggccttgggtttaccgcaatgactgccagtgcgggagactggaaaaggaatctcacgtattggttccgtgttttggggactccattcagatgtcacttaggagtgaaagcatcccttcgtagagcctctttctgtgtcaccctcctcagctgctcctggggttgactggcccctgattcatgcctttagcatgtgctggagcttcccagcagctgtccagcccctgccccaccctctctgtgggctcccttgcccgtaacctggggtgtctgaacgacccttgctaaggggcagactgttagacggtaggcatgtgctgagtcccagtggccacacccacccaccaggagcctggcactgtggccgcagcactgagcagtgccccgtttctgtggcaggtgtccatacactccgtgtggctggggaacagcatcacacccctgagggaggaggaatgggacgaggaagaggaggaggaggccgacgcccctgcaccttcgtcaccacccacgtctccagtcaactccaggttttccaatggcctttttctttttaacagaaatttgaaatttcttatcagtcatttgatttgtttgaggtgcttcttgaaatgagcctctcatctcatgtacttggaaaatacccatctcgcatattccacaggaaacaccgggctggagttgacatccactcctgttcgcagtttttgcttgagttgtacagccgctggatcctgccgtccagctcagccaggaggaccccggccatcctgatcagtgaggtggtcagatccgtaagtgagccttcccattcccctcacacctgcacgtgccacacgcaccacacacgccacacaccccacacacacacaccgcccacacacatgccacttgcacacacacccctcatgcatgcaacacacacacaggccacacgcaccatagacaccacacacacatgccacatgcacacacatacacggcatgcaccatacacacaacacacacagcacacatgccacacacacacgccacaccacatgcaccacacacatgccacatgcacacacactccacatgcatgcaccacacacacacacacacaccacacacaccacatgcaccacaccacacaggttacatgcacacaacacacacatgccacgtgcacacaccccacacaccacatgtatgtgccacacacagcacacaaccacacacatgcaccacacacatgccacatgtgcatgcaccagacacatggcacacactacacacacgccacgtgcacacaccccacacacatgtacgcaccacacacatgccacacacacatgcaccacacacatgccacatgtacacacatgtatatacacaccccacaccacacacacaccacttgcacaccacgcacacacaccacatgcgcacacacacaccacatacgccacatgtacacaccatacacacaccatacatgcaccacgtgtaccacgcacccacacagacacagcacacgcatacaccacacacacacgcacacatgcgtcccgcacagtaatgtctcttgggtgtaagaacacgacttgccagtagtagcgttctggatgcgttgcctggattctaacagcgcgattctccccttgccctcctggttttccacatctccagcttctagtggtctcagacttgttcaccgagcgcaaccagtttgagctgatgtatgtgacgctgacagaactgcgaagggtgcacccttcagaagacgagatcctcgctcagtacctggtgcctgccacctgcaaggcagctgccgtccttgggatggtaagtgacaggtggcacagaggtttctgtgctgaagccacgggggcccatctgccttgggacctggtgttggccagaggtgccgggtgcggctgcctccttccaagagttgacccgaaccggactccacggcccacgtgagctgcagtgcttctcagatggagggggttcagcgacggtcagtgccattcacaggtcactgtgatgtgggttgtggcggccaagccatggtttggggtcccgtatccctgggcttatgacatcattgtagtagcccatccccacagaaccacggtgtgtggtggcgctgaggcatcgtagatggtggaaatgctactggcttccccatgctctgccctgaggcctgactgcctcactccccttctcagttatgttccaggccccccgagcttcctggctggacagcttctctcctgggggccgttttgtcacagtgaccctgtgtttctagtcccaaatctgggtgctatagtctctttttagcgtggtggttgtcttagtcttttttggctgctaccacaagttaccttagactgggtaatttataaacagtggaaatttacttctcaccgttctgggggctggaagttttcatggtcaaggtgccagcagatttggtgtgtgatgagggctgctctctgcttcatagatggcatcttctggctgggtcctcacggtggaaggagtgaacaagctccctcaggccttttagaagggccccaatccacaagggctctcccatcatgacctcatcacctcccaaggccccaccttcttgtactgtggcactgcaaattaggtgtcagtgtaggagtttcaggagggatagaaacattcagaccatcccagcggtcaagtgttcatcctcttgagttcctccttattctgcttctggtttatcaggattcagccagtgcagcatggtacctgtattctgtggcacatcaccacatggtatttgccaagtatccatcacctgcacacgtgaaatcattgcccgtgggtcccgacatctggcgaagcatattcaaggatggcagaactgtcagagctggcacctctggttccttgtcatgtggcattacctagtaatccattttatgatagcaatggaaactcatttcttcaacaaacacctgagtggctgccgtgtgccagccgtctggggcccttggtgagaatggcatggtggtgcccatcagggcctgcctagcccgtgctctggacgggctcctgtgtgtcaggaacgacaatgctgtcatgacggtgaatgatttttttttttgccatcactccagccgctaacatttgcggagctcttcctcccgcacccccacctgacaaggccaagggtgaccttggccccaccctaggcggccaaggtcagaggttagctggcttgtctgggtcacacaaaatgcagcagaggttgaggtgagcacatgtccgtgacctggagcctgactccctctctgcgagtcttgactgctcttgcctagactctgtcctccccgagcccaaacgccagtcatcttcccttgtgggtgtccttcagcctggtgccatgctggtgactcagcagccgtccagggagtggaaacaattgagtgtgtgggttccctgtgtgggcatctctcttcacggcgaacaccctctgggtgttgcccacacgatgtcaaagcggctcttggaaggggtccttctcctttgtgggaagtttcagctgctgggctaacttgaattgtaactgtggttttgtgctcaggcccagatccccctaggcaagtgttgtgccatcagtaatcaaatgagaaataatcattttgaaaagcagatcctaaggcaggatggtcatggacactcactcccagctctttgtgcactcatgctttctggaagatggccatcctctgtgaaggttttcagcgcgtcatgcttggtacccacgtatccagagcatgtcgttttgaggtatttgcccaccgttgtgaaatccgtgccacccgagagcaggtcctgatgtggggctttcagaagtgggacctggggccgtacgcagtccttagggaggggccgtgtggcgttgtgcgtgtgaggggatagcacagggtgaggtgggggcccaagaaggaagtgacccacaaagaacagcctcctcttttggtccttgttcctgggatggctgggagtggcttctgtgtcgtccggccatttcccctgcggagaggctcctaccactgccgagaacctcatcattccacaaaaacaagaggccgcctggccatccagcgctccatgggaattctgtgtccccatagtcttgggctgaaggagggtgacattccttgctgacttctgcaggggtctcctcactgttaaagagcagattgaaagtgaagaacgtgggctaagtgtttaggtcgatatttaaccctgctaggttttggatactaagtgaaattgaggccattttggttgaagttgacagaaaccactatcagggatccccaagactaccccaggcttttctagaaagactctcagctaagatgtgttatggtaaaagcacacaaaacaaaatcagcaaagaaaattagcaagggcagaggcccatggggcgatgtcccgaggacaccaggcttgagcttccagaatcctctcccagcggggtcgtgcaggacgcacttaactccccgcacagtgagccgtgacagcgcgtgtgcagtgtcgtcgccaggaaagcacactagagactcggtgccagggtttttactgggggctgggcacatgggcaccctctgcctgcctcgtgcccagactctggactcccggagggaaggcaagttctcagcaccaaccctggtgcccacacaagcagctgagcacagggagcccctcctcagtgaggatggtgggcaccgtcccaacaccagccaggggccagccttgcacacaggcctctcaggatggtctccggcctgctgtgtagtctcttctgcacacaagcgtgagggcagcgcccccgcctcggctgtggggaggagccactgggacgtgagctctggtggcatgcagcagcttttgtctgtgtgtgcctaggacaaggccgtggcggagcctgtcagccgcctgctggagagcacgctcaggagcagccacctgcccagcagggttggagccctgcacggcgtcctctatgtgctggagtgcgacctgctggacgacactgccaagcagctcatcccggtcatcagcgactatctcctctccaacctgaaagggatcgcccagtgagtgggagcctggctggggctggggcgggggtctcagaatgagctgtgaaggaagcagcatcaccctctccaagtgcccaggctcctggccagatggcaggccaggtatcagtgggaacccaggtgggtgccatggctgaggtcagtgagacgcaagagcacaggtgcgtcctagaggcttcctcgggcacctccagcgagctggagctctcgcctctgctgctgtctcatgtggcgcttagcacactctcccacgtgcccattcctgactctgctctcgaggccatcggctctcattctctgctcccagaaccctgttattacccaggctagcctcctctctgcaccttccccgccctggcccagtacctccctcttgtttccactgtgattccgacctcaccttatcttaaagctgctggacggcaggttctgtacacacgtgtccttgacaaagcacggctggtgccgcaacccctcagcgagcaagtcaagctcttcacagcgatgtcttacaagcgcagagggctctgtgacaccctggtctcaccgccactcttccaaagtcgcagaggctttagcagagatgggcccagcctctctgagtcataggcttctgcacacgggagctgtctttagagggagggtggaatttcatcagccacccacatgggggagttgagggcaagaattaggagcaaagatgggaaggggtctgggaggaatggccagtgatcccctttgacaagtgggcaggaaacgggggctaggtcaaagttgagtggaagacctggagggagacgggaaggtctctgtaggcacagttcagacaggagggaggtgtgagccagggcacatgccggtggccgtctggcaggatttgggacatgctggagcagggacagcggctcatcaggggccattgccctcatccaggccagagtgtcacaagcccgtggggaggcccttctcgcctgtcatccttgctgggcagtgggtgctgtgctagcaggacaggcggacggctggcaactgtctctgcatccctggagcctggcatagggccaagtcacacggggcacaggcctgcaaatcaggcacatatgttggtgcagtgacgtgattttggggggcagccccagaacaggccccagacacaggccaaagccctgcctgtgctggtgtgttgggctgttctatggctcttgctgtgggcatggaggactcagggaaggagagttgaggtggtccaggagttgcgtttgggatgcagagagcttgtggcatccaggtagaaatggtgcgtggggctgacctcagcaccatgggcagaggggccgtgtcacgtgcctccgaggtggaggtgggaccacgtggtgacagatatacgcatcactgggcacgtttttgtgggtgttggggggcatcgtattggctcctctgttcacagtggccactcattcagtccctggctaccaggtcctcactgtgccatggggaaggccggcgctgtcgggggatcacagaaggcagcacgtcatgatggcatgtgccatgaaggaaaagcacagggcactcaggaagtagaggggactggcctggggtgtgggaatctagggcctcgttgagggacagagagaggaagtgtgtggtggccagcatggaggtggccacaggggaggctgagttaggccgagagggcagggcgttggggaggtagacgggctcagccactcagggagtggtcaagcagaggctgaagggtcaggccaggttgcaggggcctgggggagccactcagggtaggcgctcccgggagcccgcctggcccatagctctacactcccgcgtggggccggacatgctgtgaagccctctccacgttggatgggggtggctgagcctggatgctgtctcccgttttcagctgcgtgaacattcacagccagcagcacgtactggtcatgtgtgccactgcgttttacctcattgagaactatcctctggacgtagggccggaattttcagcatcaataatacaggtgagtgggccctggctgtcttcctctgcacacggggagtgggcttcccttctcttttccttgcaggatcataccagtgggccagttttgacttggtcgggaggaggcatgaacacctgagactgtgcagcgattctttgacacagaggcctttctccctgtgcagatgtgtggggtgatgctgtctggaagtgaggagtccaccccctccatcatttaccactgtgccctcagaggcctggagcgcctcctgctctctgagcagctctcccgcctggatgcagaatcgctggtcaagctgagtgtggacagagtgaacgtgcacagcccgcaccgggccatggcggctctgggcctgatgctcacctgcatgtacacaggtgagcatgtacacggtgcccataaggccagcccaagtcctgttcaagggaggcaggagcatgctcactcaagggacctcgactaggtgccctctgatttcacacttctggtgttgccccaagccggccccatcaccttgcaagaaaggctctggagcccccagggctggagtacctggtcagggttgaccgtccctgtggtcactcatcccatgtggctgagctgggctgggtcctgggcaagcaaggggctgatatcacctgctttcagatctccagggactcactggacccctgtgtacaaagcactgtctacagagcctattgggttgtatagaggtaaccttcgtactgaacacttttgttacaggaaaggagaaagtcagtccgggtagaacttcagaccctaatcctgcagcccccgacagcgagtcagtgattgttgctatggagcgggtatctgttctttttgataggtaagaagcgaagccccatccctcagccgttagcttccctagaactttggcctgaagctgtgcttttgtgtgtgtctgctgatcccctggcgctgttgctggagtcctgccagtgattccccaccacagcctgaccatgggctgccttggctcagggttccactggcgagctggtggtccttggaccccagcactcaggtgtagcgttgaccagttccaaggttgtcccagtgcctgcccatctctcctgagggctcagggacagtacctggcagttgggggtgtggcagggggcaggaatgaccagcctctgggagggtggggcagaagcctgtacagtgaggaggagctggctcagcctggctgcctatcgtgagaggggagcccacggggctgtgggaggggggccgtggtgcctgtgagcagggtgaggagcagcggcaggaggatgaaggtggaacccacacatgcatctttgagacccgtgtggtcagtggcttctgccccccaccaccccccactgctgtgcgtgcatagaattggcttccctcacctgctctggaagtgggttaggagcttggtagggctttttctcaaggacaagggcccctgatttgctctcaggcctcagtcctggcgacatggtggatctggagccttgttgcactgccttgcctgtgctctccaatcagggtggccagtggggagccatttggcttttctcaagagcatactcaggtggaccttgctccactgtttgaccagatgaggcattctgaacagccaagcctgtgctggtctgttttcatgttgatttttttttttcttttctttttgagatggagtttttcccttgtcacccaggctggagtgcaatggtgtgatctcggctcactgcaacctccgcctcccgggttcaagtgattctcctgcctcagcctccctagtagctgggattacaggcacacaccaccatgcccagctaatttttgtgtttttagtagagacggggtttcaccgtgttggctgggctggtctcgaactcctgaactcaagtgatccaccctccttggcctcccaaagtgctgggattgcaggcgtgagccactgcgcccggcccccatgtcgatttttaaatgcacctctgcatcgttcttcagtccccatatgctcactgagcaccactgcgactggcagacgggcacagggaggcgccacgaccagtcctggccttcaaggggcttgtggtctagtgggcccaatgctaggtggcgagtgctccaaagagtgtggtgcacgccttccgcttgaccgctctccagacgccacagggaggcacctcgcagctgaccacagatttctctctgtggagcagtgtcttcagagcggctgccatgccactgctgggcgagggtctgcgggcgggtagagccaggagcacctgtgaggaagtgcactgccattttcgtagctgcttcccgtgtgtctcagttacacacggctggcatgtgtgcactgatgagacgggaacgtgatggttgcttttcagcactgaaagggatactgctcagggggcgtgtttcaggatctggttagggaagaagcagcgagagcacagatggggccctgtgtggtaacaagaaaaaagtcctggttgacaacagtgccacgaagcgttagaacacatagggatgtttgtggagcatttgcatgtggaaagcagcaaaaacataatgggaacgggttcttttgttatgatttttaaaaatctcttttgtaacatccttcccgctgcgccgtttctgcatattcctttatgtagctttcaaactcctcttaggagttctggtccctacagggcgtgggagcccaggctttacgtagctttcaaactcctcttaggagttctggtccctacagggtgtgggagcccagggcctgtgccgagcagcctgcctccacgagctagacagaggaagggctggggttttgcctttttagtctcaaaattcgtactccagttgcttaggctctgactttccccacttggaaagtccctcacggccgagggtccctcccagccctgatttcacatcggcattttccccagtattagagccaaggccctccgcgggcaggtggggcagctgtgggagctggtgccagtctctgacctgcgtccctcctcccaggatcaggaaaggctttccttgtgaagccagagtggtggccaggatcctgccccagtttctagacgacttcttcccaccccaggacatcatgaacaaagtcatcggagagtttctgtccaaccagcagccatacccccagttcatggccaccgtggtgtataaggtgaggttgcatgtgggatggggatggagtgggaaagcctggaggtggagttgcctccgacttcccagcagattcgccagcagagcccagctcctccgctttaaagcagcaatgcctctggcccccaccccacccccgccacccaggcgcagcaggtgcttcccgtccccccagccctgacactcaggcacctgcttgctccttgcaggtgtttcagactctgcacagcaccgggcagtcgtccatggtccgggactgggtcatgctgtccctctccaacttcacgcagagggccccggtcgccatggccacgtggagcctctcctgcttctttgtcagcgcgtccaccagcccgtgggtcgcggcgatgtatcctctctgggtccctggtgctggccccgtttcccttgtcaacaccgaggctcatgtttcatgataaggttttgaaacctaacctttgcaaaaaccccacagatgccagggtgacaggccctcagccccagggaagtaaaatgctgacaggggtacagaaaggagcacgtccagacatttgctgaccagggcctctcagaggggccggtgtatggcaggagggtcgcagctgaggggcctttctgtggagggcctgggtgaggggagcgagggtgggcggtggtctctgcagacgtcccgcccactcgcgggctctgtgtggctgggcttctcctgacactgcttctcattagctttggtcattgtgcctcgatcgccctctcggggaaaggcttaagtaaagatccagttcccacccccagatgctggctgccaggagtttccctttccacagcccttccccaagacagaccacaagagcctccaagcagcacagttgtcctggtgctgacagcacagccttgcccggcgtgcctggcacggctctgccctcactgcattggagcagggctagtggaggccagcggaagcaccggccaccagcgctgcacaggagccaggccaggtgagtgctgccgagtgggtgccctgcctgcagggcatccagccagccaagggttgcaggaatggaggtggaggcgctgatgcagctggaggcatccaggtggcccttccggggctctgctcgctctccaggctccctggacccctttgtagactgtttcaggagaggaactcccaggtgaggacagggaggcagcattcccctcatttgccggcctttttccttaactcctgcaccagcctcccacatgtcatcagcaggatgggcaagctggagcaggtggacgtgaaccttttctgcctggtcgccacagacttctacagacaccagatagaggaggagctcgaccgcagggccttccagtctgtgcttgaggtggttgcagccccaggaagcccatatcaccggctgctgacttgtttacgaaatgtccacaaggtcaccacctgctgagcgccatggtgggagagactgtgaggcggcagctggggccggagcctttggaagtctgcgcccttgtgccctgcctccaccgagccagcttggtccctatgggcttccgcacatgccgcgggcggccaggcaacgtgcgtgtctctgccatgtggcagaagtgctctttgtggcagtggccaggcagggagtgtctgcagtcctggtggggctgagcctgaggccttccagaaagcaggagcagctgtgctgcaccccatgtgggtgaccaggtcctttctcctgatagtcacctgctggttgttgccaggttgcagctgctcttgcatctgggccagaagtcctccctcctgcaggctggctgttggcccctctgctgtcctgcagtagaaggtgccgtgagcaggctttgggaacactggcctgggtctccctggtggggtgtgcatgccacgccccgtgtctggatgcacagatgccatggcctgtgctgggccagtggctgggggtgctagacacccggcaccattctcccttctctcttttcttctcaggatttaaaatttaattatatcagtaaagagattaattttaacgtaactctttctatgcccgtgtaaagtatgtgaatcgcaaggcctgtgctgcatgcgacagcgtccggggtggtggacagggcccccggccacgctccctctcctgtagccactggcatagccctcctgagcacccgctgacatttccgttgtacatgttcctgtttatgcattcacaaggtgactgggatgtagagaggcgttagtgggcaggtggccacagcaggactgaggacaggcccccattatcctaggggtgcgctcacctgcagcccctcctcctcgggcacagacgactgtcgttctccacccaccagtcagggacagcagcctccctgtcactcagctgagaaggccagccctccctggctgtgagcagcctccactgtgtccagagacatgggcctcccactcctgttccttgctagccctggggtggcgtctgcctaggagctggctggcaggtgttgggacctgctgctccatggatgcatgccctaagagtgtcactgagctgtgttttgtctgagcctctctcggtcaacagcaaagcttggtgtcttggcactgttagtgacagagcccagcatcccttctgcccccgttccagctgacatcttgcacggtgaccccttttagtcaggagagtgcagatctgtgctcatcggagactgccccacggccctgtcagagccgccactcctatccccaggccaggtccctggaccagcctcctgtttgcaggcccagaggagccaagtcattaaaatggaagtggattctggatggccgggctgctgctgatgtaggagctggatttgggagctctgcttgccgactggctgtgagacgaggcaggggctctgcttcctcagccctagaggcgagccaggcaaggttggcgactgtcatgtggcttggtttggtcatgcccgtcgatgttttgggtattgaatgtggtaagtggaggaaatgttggaactctgtgcaggtgctgccttgagacccccaagcttccacctgtccctctcctatgtggcagctggggagcagctgagatgtggacttgtatgctgcccacatacgtgagggggagctgaaagggagcccctcctctgagcagcctctgccaggcctgtatgaggcttttcccaccagctcccaacagaggcctcccccagccaggaccacctcgtcctcgtggcggggcagcaggagcggtagaaaggggtccgatgtttgaggaggcccttaagggaagctactgaattataacacgtaagaaaatcaccattccgtattggttgggggctcctgtttctcatcctagctttttcctggaaagcccgctagaaggtttgggaacgaggggaaagttctcagaactgttggctgctccccacccgcctcccgcctcccccgcaggttatgtcagcagctctgagacagcagtatcacaggccagatgttgttcctggctagatgtttacatttgtaagaaataacactgtgaatgtaaaacagagccattcccttggaatgcatatcgctgggctcaacatagagtttgtcttcctcttgtttacgacgtgatctaaaccagtccttagcaaggggctcagaacaccccgctctggcagtaggtgtcccccacccccaaagacctgcctgtgtgctccggagatgaatatgagctcattagtaaaaatgacttcacccacgcatatacataaagtatccatgcatgtgcatatagacacatctataattttacacacacacctctcaagacggagatgcatggcctctaagagtgcccgtgtcggttcttcctggaagttgactttccttagacccgccaggtcaagttagccgcgtgacggacatccaggcgtgggacgtggtcagggcagggctcattcattgcccactaggatcccactggcgaagatggtctccatatcagctctctgcagaagggaggaagactttatcatgttcctaaaaatctgtggcaagcacccatcgtattatccaaattttgttgcaaatgtgattaatttggttgtcaagttttgggggtgggctgtggggagattgcttttgttttcctgctggtaatatcgggaaagattttaatgaaaccagggtagaattgtttggcaatgcactgaagcgtgtttctttcccaaaatgtgcctcccttccgctgcgggcccagctgagtctatgtaggtgatgtttccagctgccaagtgctctttgttactgtccaccctcatttctgccagcgcatgtgtcctttcaaggggaaaatgtgaagctgaaccccctccagacacccagaatgtagcatctgagaaggccctgtgccctaaaggacacccctcgcccccatcttcatggagggggtcatttcagagccctcggagccaatgaacagctcctcctcttggagctgagatgagccccacgtggagctcgggacggatagtagacagcaataactcggtgtgtggccgcctggcaggtggaacttcctcccgttgcggggtggagtgaggttagttctgtgtgtctggtgggtggagtcaggcttctcttgctacctgtgagcatccttcccagcagacatcctcatcgggctttgtccctcccccgcttcctccctctgcggggaggacccgggaccacagctgctggccagggtagacttggagctgtcctccagaggggtcacgtgtaggagtgagaagaaggaagatcttgagagctgctgagggaccttggagagctcaggatggctcagacgaggacactcgcttgccgggcctgggcctcctgggaaggagggagctgctcagaatgccgcatgacaactgaaggcaacctggaaggttcaggggccgctcttcccccatgtgcctgtcacgctctggtgcagtcaaaggaacgccttcccctcagttgtttctaagagcagagtctcccgctgcaatctgggtggtaactgccagccttggaggatcgtggccaacgtggacctgcctacggagggtgggctctgacccaagtggggcctccttgtccaggtctcactgctttgcaccgtggtcagagggactgtcagctgagcttgagctcccctggagccagcagggctgtgatgggcgagtcccggagccccacccagacctgaatgcttctgagagcaaagggaaggactgacgagagatgtatatttaattttttaactgctgcaaacattgtacatccaaattaaaggaaaaaaatggaaaccatcagttgttgctgtgtgaggcttgctttgcttcatgagaacctagaccttgctgagctggagtcttaggaagcagtctcctaagtgcttctccagcaggggcagaaactgtcccaccagctaacatctggcattatggagggtcccccaggcagctgccagcagggacaggccccgtgttttctgtagccagggatgaggaagtggccccagggcatgggcctggctgggtgcttctgcaagggccttcccaaaccacagtacaggtggtcttcctgccctgcagatgggagctgtgggagctgctggagctgctggagccttcatggtcaagtgacatcataagcttatatgacatacacaagcctcaggacttggcccatggcactgaagcaggtcatcaggcccagcacagagactagagctgtgttctcacagggcccaccacccttccacctccttggccattgacacctgcgtccctggcccagctgctcccaggtaacccccaaagcagctggcacatcccacctctggtgtggccggggctgctgtgtgtccgcagggcctgccccgtctattctagcttgtttgtcctgtctgaaccagcgcctactccaagaagcctctgctcagcccagcggggatgcttctaagctccggacgagcctctcggaagccttggtgattggtggtgtagtcatcttgggatgcagatgtcttaccaacctgcaagaacaaaaaccctgtggcttcctctggtgcagggtatttagtcaatgtttgctgaggtcccgtctggttctggctaattggcaggggtcgtccacccattctttccctgctctgctgtctgtgccaggagagacgggggccagtcggccaaggggccagctcctgctgcctgctcctcttgggcacgtgcgggggccccctttctctgagcagggatagggatcagtctgccggagggatgtggtggacaggcctaaagcatttggggcggggcatgccacttgagctccctaaatctgtctcctcataggtgacaccgctccagggccccccagtggcctctcctttcagagctacctaaattctggtcacttcagagaaatggagcacccccttctccctggtccaggtgtggacagcctggcacactgagcacacctggcatggctggtaatttcagaaagaagaggggccggggtccagtgggaagcagcggtgaacccctcgtgagtgggctttgcagtccctccccatgccacggcagagctgccctcaacacagccttcctcttcctcatcggagagcacaccctgtccccttgccgagctgtgccctgtgccttcggtggtatttgattttggctgctactggctttgttgggatctggaagtcgcttcccctgcgtggtgcgtggagcactgtaagtcagatgagggaagtagccagggtgaggtgagtaccgggtggagccgccactgaagggactgggtaggggggccttgcctctacatgatgtgacacagccaaccgaggacagaggaagccccgttcctgggggtgtggggtgcacccctcagggaagcctgcagtggggcctgaggaaaggcatcctccgcgagcccacgagtctggtccatgagcaccgtgacagtgtctgtgggtagaggtggacccggccttgtgtcatcaccaggacctcttttgggaaaccatgtggacatcgcttgcgggtcccccaggctctgcagccccagcagcctggctgccttttgggcaagtggcttgagccacagaggacccagtcctgttgcagccacatcctctgggggggcccgccagtgtggccggctttctccaccctacaccaggcctccaggtgtcctggtcgggggtgtctgggccctgggtgggccctgtggacctgtgaggtcagggtcagggcatcactggaggcagagggctgaagttgtgggtctgggttccccttgtgtgcacaggcccctgccctccatgcttggtcaggcagctacccccaaaactgctaggacaggctggtcctgaggtggatcctggcccctgtaccctctggacagcccacccgcccaaccttctaccctgccccagcggcggcagtgttggccacatccttcccctcctggccccaattgctctggggaagtccaggctccggagcctgcccaggggccccccgtgatttgggcccaggactccacgtggttctctgccttcacccaagccctgaactcctcagctgccaaatccccacccatctgcacaggctgtgctcaccactgctgctcctggaaggtgcccctcagtgggacgcccacctcctctctgggcttctgtgtttgggagccctgctgcccccacccttggtcagtccccatgtcctgctggcctgtcaggcagggcagaaaatccacccagaaatgctgagcaggatgagagtctagttgggcccagcctcattatttagaagggatggaggcctagggagcatgcttctagcctgagcccagcagggccccgcccatgtcccaggtctgcaccagggacagctcctgccgaggcctgacctgccccttctccctcaggtgctgctggttgaccagcctctggccctaggagaccccgtagcgactgagggtcccagcaggccatgcagctttgccaaggtacgagcccctccccagcaggggacagatgtggggaccctcccaggcaggagcagctgggtgcctggtgctgccatctgctgcctgcctggttcttgtcctcacattggaggtcagtgtgagggctctgcctcgggaaaggccatggagcttgccctgtccagggcctcccatgtgcactgagcctgggaagagagggttggagttgagccttttaccctgggaatgctgcctggaggatggtgcgggtgtggggtggcaccctgccaggcagggccctgcctccctgcgcccactggaactcgggcaggcaggggtgtaggtgcctcctctagagccgtccggtgggggcccccggcagtggtggtggtgtccactggccagcagctgccccttcagccaggacagtaggcctgacgctgtccccagcagctccaaggtggatttgtggaagggggtagagggcacgtagaggccccatgacctccccagggttctgggagggctgtgcccccttagccagcaccatgctgggtgatatagtcagatcctgttacccctgttgtggaggtgaggaaacaggttagtggggaggacatgactaaggtccatgctgagtcgctagagctgcacccagaaccactgctgggaccccatgcctttctgcttaccccttgtgccgggagatgccaagagatgctgggagccagccccacctctgcccttggagtcatggctacggaaagggcattcggaccggtccctgacctcaccggggagggccgaaccctgttcctgaggagccagggcttcctagaggaggtaggccttctagtcactccttcatctgcaggcactccacagagctctctgtgccagcccccagcacggagggctgaccttagtcgagtggagatgccccagtgccaggcagtagggatgatgtctcctgaggcccagatggaagggactggactagtctcatggggctgatggtggggccaggccttgaccagggacccagtgtagggggtgcagagacccctctgagttcctcacacatccctggggccctccccatacacttcctatcctgactgcgggcaagagggagccccagttcgccttccctatgctgggcacccacagtggggctgggcacccccgccatgcccctgccctgtccttcccctgagagcctcggtcccacctccaaggtgcctcagaggacagcaggggcagcgggcagaggccgagatgcctcctcattccaggctcagctgcccttcttggggcagcccacacctgagagtctcctgcagttggtcaggcctgaggagggcaggggggtgcctgctgtccctctgctgaccacagtggcatttagcctgggcaccgcgcccagcacagtccatgctgcacaggtgccgtgggctccacagagccctgcctgacatgcatgtgttacgtttcgggtgccgatgcccttgggcggcacttctccgggcagaacccccaggccaccgctccggttccggttccgctgcatctggggctctcggcaggctgtggtcctccggccagcctgggggcatctcagtccctcagccccacaggggcctgccccgcagcctgggcctcgagccccgtctccgcacgctgtgccgaatctggctgcccatcagctccctgcgtacccagactgtgccctgccatgcccgtggctcttcccaggagtgccctgtggcctccccctggcttgctgggctgattccctcctgtgtctcaaacagagctcacctttgccatcactgctgtcctcaccggccggtgccagaggcccgtgtctgtgtaccctgtgtctgcacctctgggcagggcctggctctgaccaacccgggcttccagtgtccacagacctaaggcccagggcgcctgggggctggagcaagagaagcaaaaggagccaagggtgggggtttggggttcttgtgagggcccagccccaggaccccaggaccaggacacccaggagccccagggcccagccccagttcagaaggcaggggccttctgagggagcttaagggtcccacagcccaggacccccaccagggccagtggccagcgttgggggactcagcctcctcgtcgctcgtcctctctgtttctcccaccttttgccccctttctccttgcctgttcccacccgaggccccctcttggcctgcgtgagccggggcggcactgaactgggggccgatccgcctgggcggcggtgagaggcagggccgggagccgggccgctgggtttgggcctggcccgctcgccgcaatattgatggcccgtcagtgcagccctgattcctgtgctttcagttaaaaggtttctgttgttgtagcttatgcagttgctctgttgctatggaaacgtgacatcaaaatgacgtttcccgtttaaaagcttttaactaaattcctgcctgtcagatgtaggccccattttgagcgtggagctgccttcgagcgagcgtgagcggcgcctcccgcccatggtgcgtggggccgggccggggccctcgctgagcgcgctctctcaccccacaggcgcctccggcatggcggcggccgaggggcccggctacctcgtgtctccccaggcggagaagcaccggcgggcccgcaactggacggacgccgagatgcgcggcctcatgctggtctgggaggagttcttcgacgagctcaagcagaccaagcgcaacgccaaggtgtacgagaagatggccagcaagctcttcgagatgaccggcgagcgcaggctgggcgaggagatcaagatcaagatcaccaacatgaccttccagtacaggtgggcgagcgggcagtgtgggccccaccaggacgggcgggcccgggcgtggcgggccgctcctgactttcttggagctctgagtcgggacgatgtgtgggtcgtggcctgcctgtcggtctcctctggccgggtatgggcagaaccccacggggtgagacggggcccacggaaaccgtgtgtgcagccttccattggggaagtggggaaactgaggcccagcaagggcaggaaaccagtctaagagctgaggggtagcaggggtggggctggtgctgggcagaggccaggatggctcccaggacgtatgggcggtctgggcactgtccctcggaggcagcaacactcatggtggtgcccactgacctcacaccctgctcccccatagggaggcggcggctgccagtgccctccccaccaccaagctcccaagctcagcaggggtttcaggggcctactgcgtcattggggaaattgagactgcaagtgagaaggaggctcagtgctctgcgacttggagcatccactgagcctctgccatgagccggtgagccccactggggctggccctagggtcacggtggggtatttccagaaatcaccaggtgaggtgcaggaccagccagcgcatgggtggggcttacggtgcgaagaagaaagaggtggaggcctgccctggcccaggactcccagcgtgggggctcccggcctggccccacctctgctcctgctacatggcaggtgggcccttcctgccctggcaacctgcagggaaggccggaggggaccacccagccagggagatgttggcgtctaggaggggacaggtgtggtcccacacacccagcatcttaaagtgcgtgggtccccagcccattaggacagggtcccgggtgggcaggggtcatggtggggtgaaggtctcaggcacaggcaaggtcacaggtgcggtgagggtcttgcagggtgtgaaggtcataggtgtgcggtgaaggtcacaggtgtggggtgatggttttgggtgtggggagggtcttgcacggagcgagggtggcagcaagagctggaagctgcagggggagaatggcagcagagagcacccggccctgtgggcggcctggacagggctgggcctggggctgccggagagcctgtcagcttccaggatgggagtggcctcactcagctgctccacctccgggtcaggcaggtgagcctggggcagagaggctgagagcacctgagccacttgtgggagaggccacccccactgcccccctcaggcgaggagccggcctccagcacagcagaagggaacccccagtccccagccctagtgggagtggggaagaggcccagcaaggccccggacagaccgccagcctgtgaggtctccgctttcagttgcgttgatttgattttttctgagccttgaaggaggggtccggggcctggccctgcccaaaggcccctaggcaggccccaaagccgggacctagggtgctgagcatgacggatgttgggtttgagcggctggcttgcgacgtgagggctgaggtgtgagcctgggtatcttcagaggttcggtggacacaggcagctgcccgcggccccactgttcccgtggcctcctagtcctgctcaggcacctggtgaggaagggacgcagagggcagtgggaggtggccacgactgttccagcaggctcccctctgactcaggaattcacgggcaccacctccctggctggctctggttggtgtctggccaggttattcattatttatgctgaaagcctcttcagagtcccaggggagggtttctgtctccattcctggaggctgagagatgagggtgcagcagagtgggggcctccactccagaccctgcagtctgggctggccaagggctgcaccggtgcactgcacgtcatggctgatgaagcacttccacaccgcagcccctcagagctgccacagtcagccttagttcaccgagggggaagctgaggcccagagcatgagagggacttgcccagggccacatagtccttagcagaggaagctgtggctgggtgactcgatctttgtcctttttctttatacccgcagtctccccatagcagaggcttttcttttttttttctttttcttttttttttttttacaagaactctttatatattaaggctgttgggctgaagaagcctgagagggtggctggttctgtggagcatggtttgttgaagtacagtttgggggcctcctacactgagaataggccttttctcgtttctccaaagagtgggctggctcaagtagggcagagagagaagcctggggcagaggttagggatgggcacccagcgcctgccctcacacgctctgtgctggtgtcttcacagccacgtgccaccctgggcagcatcccctgctcaccatctggctgtgcctgtttgctgggggcacctcattcagaatccagcttattgtttccaacggccaatggccacaccctggcaggtagcaagagtaggagagaggagacacccactccgagcacaggttgggtttggagcccggccttggggcactctgtcactcaaaggcagagtggggagtgggcactgggccttaggaggtactgggtccagtgaggcagagatgcccctgccccacccccaccttgtggcttcttccctggcctggccagagctgtctggccgccatggggccctgtgtctcctgccttgacctcccagagggcagccgaggcccaggggaggcctggggacttagcctctcagggcaggacctgtctgcaggagtaggtgggtgctgggggtcccagtggtaatgaggcatcaggcagtgtgggaaggggcccatccggcccaccccagggcctctgggcaggttgcaggttgtagcgctggatctaggctcctgcccagactgtaggttcaaccaagaatggcatgggagcccagcctgctgtttgctttattaaatctgccctgtagctgggggaggggcttactttgatcatcactatgtcattgatataaaaatagaggctcagagaggtgaatgaacctgcccaaagtcacacagcaaagtgtggagatgagatactgactcagggctgtggacactgaagcctgtgctctaacgccagtggctgtcgctccctgaggcattctctcccgaacaacacagttattatattacaaaatattatcactatatttatatatcttataataccttattattacaataaaaccttattactctacctttcaaaatgaattatttaaaaagcagtatttgctcattgcagagagtctagaaactatagaaaagcaagggaaaagcaataggaccagccccaaggtcccagcatgcacagataaccttagtaatactgggacgtgtgcttcctttttaacatctgagcccgtgtaggtcctgaagcccagcttctttctaagtccattgtcatcttgaccctggagcctggccgattttgctggggaggcccttgccagccgagagcggctcctgcctgtgccggcgtggcgcgcccctctgctgaggctgggcaggacaggggctgggccagctctgtttctcacccttggctcttgtgtctctcgtttcaggaaattaaaatgcatgacagatagcgagtccgccccgcccgactggccctattacctagccattgatgggattctggccaaggtccccgagtcctgtgatggcaaactgccggacagccagccgccggggccctccacgtcccagaccgaggcgtccctgtcgccgcccgctaagtccacccctctgtacttcccgtataaccagtgctcctacgaaggccgcttcgaggatgatcgctccgacagctcctccagcttactgtcccttaagttcaggtagtgtgtctgcttgtccttcccctgccctggggtatctcagcccccaccatttagagaaagggactgggagtggcaaggccggcggcggcggccacagtggttgcagaggccgtggctgcgggcagcgcctccagggacaggcggcctcagaccagggagggctttagtgtccacaggcagaccgagtttgtctcccagctccatcacttttgagctgcacggaaagttccttgacttctctggcctcagtctccctcctataaaatgggggtaaatcagtacctttctcagagggtggctgggagcatcacaggagagaagacgcagcatggggcccggcacacggagggagaccaagccccagaccccagaatgcgccccctggcctcccttagcccacacagaccccaccctcacaggctagctgccctctcagcactggggagggtgtcgggctgcacctcatcacgtgttgccgtgggcatgacccgtcccctctgccatccatcccacacctcagacccgtcccgtgctggccacgtgactgtgcctgcaagatgctcacagggcagccgggagccaggcagcatgcaggacagacacctgcggggtgggcctggggagcccagagaaggtgcttttgaggaggggacatttggggtgggctttcaaggtaaaatagaagttggccatttggaggcaagaacaggaagattgtggatttgagtcacagcttctcccctgccctggtcttcaagtctttctgacaggaggtgtcagaaaagtatctttagtagagaaggcgtctccgaggagggtccctctcatgccgggggccgctgcttgactcaggatttctcattgaagacctgagacaaaaacgcttttgctggcagctagaaggaaccagcaggaggcctgagatttgtggctgttgttcccgtggactgagcccagttctcagactcagctgcctggggccttgcacaggactggggcgtgggggctgccctccctgatcaggcccaaagcgcggatctcacgcccctgaggttggctgtaccctctcagctcagagcagagtgtgggccagggatgagcaggcactggagcagggccctggggtctgtgggttttggcagctccctgcccttcagggaggtctgctgagaccacgggtggcccctaccccagcagcagagctctcaggaggcgcccacagggctggactgcctttactcaccacctctaccagagctctgaggtcctggggagagagcccaggcctcttgtgggccccacaccctctaggtgcctgtccttctgcctctctaccaaggtgtgccggccccatttctaggccgccgggagataagggggctcacatctcaggcccttccttctgggacctcagtttccccatctgcctaaggccgggtggggctggtggtcttggcttccctacaggggtcctgagtactctgcactacccagcaccccccacccctgccttcatctctccctgggggtggtctctccacccctggcccccaactggggctgagcccccacctgcccagtttggtgggtgaagggtgctccctggcaggatatgcccctctgcagcccagaacatcccaccctttccagaccgaaggggtgtggattgtcctgggaccctggtcattggggtcatccgctagtcgcaaaggacggcaatgcctgtggcctctctttctttctttttctttttttttttttttgagacggagtctcgctcttgtgcagagagcagtggcgcgatcttggctcactgcaacctccgcctcgtgggttcaagcgattctcctgcctcagcctcccgagtagctgggattacaggcacccgccacaacgcctggctaatttttgtatttttagtagagatggggtttcaccatgttggccaggctggtcttgaactcctgacctcaggtgatccacctgcctctgcctcccaaagtgctgggattacaggcataagcctccacacccggccacccctgttactttctgtcaaaggcggtgggttctggcccctcctttgcacatggaatatgagaccctgagtaagtgacctgactccctggggcctcagtttccccatttgcccagtaggattgtcgggagggtccggtgaggcccctggtgtgcccaggctctgtggccagcacgtccacagccggcactgtccttccaggtcggaggagcggccggtgaagaagcgcaaggtgcagagctgccacctgcagaagaagcagctgcggctgctggaggccatggtggaggagcagcgccggctgagccgcgccgtggaggagacctgccgcgaggtgcgccgcgtgctggaccagcagcacatcctgcaggtgcagagcctgcagctgcaggagcgcatgatgagtctgctggagaggatcatcaccaagtccagcgtctaggccagcaggcggcggcggcggcggggccgggcggctggtggtactgctcaggccacccagggcaggccactcaggccaggcgggcaagggggccgccccgcgagcggagaccgccttccacctggcctctggcaggatgtcccttctgaggggtattttgaggaacccccaggccctggggaccgtgaggctccagtctccagcatgaatgcccttcctcggacacaggccagggcctctggggttcactccgagtaagaacgtcctagagccactctccagtgtcgttactatcaatgatacttgacgtggctttgatattaaacgtatactttttcattcttgcctggaacgcacagtttgctgttgctggcttggtgaggatgccctgattgatggatcccgaaaatgaaagcagatggaaacgggttggggcaggctggagctgggggagctctctcctgaagggaaccctgtgtcctccctcaccaggacctctgcgtctctccttaaatggcctctgacgcctgatgaaaaccccagcgaccttccaggaggcttttattcagctctgtttggagcatcaggtgtttccactgcctccttagcaatgacactaataaaagtcgtaacacctgttcacatgcacagccctgttgagtgttctgggtgctggagatatcatggtggatgacacaaaggccctggcctcttggagcttatgctcccatgcggggaagacacatgggtcagtagagaaatggttgcaggttgtgataagtgctggaagggaggggttggcctgaggacacggaggcagacatacgtggagctgggaacagtggccacacagggaacggccagtgcgaaggcccagaggcagaggacactggagcaagcccaggagcagctaggaggctggtggccagcagccaggccacggaagcccgtgcagcccgtggggaggagtgttcatgcttttcaagcttagtgggagtcttttggccagtgcagctctgggtctgacatcggtgggggacagaggggtggtggagcggccacagctgcaagctcacctcactgccggcccttccaccagtttcaaactctttctagaagctccagctttcccaaagctgaattctctatgagcctccttggccgggactcgggcgtctggttgccctggctgcaaaggaggctggggccaggtgtgtttgagtcacctcctggaattaggcaagttgctgcccaaatagaaggttgttggcaggtgggtcagcaggtgaacagcatggtttgactcagggttcagaaaaatctccctctggctgccaagcgagcaggccgtggagacaggtgcagaggcaggtgtggcagcaggcatcctgccaggcagtgctgcagtcatcctgcgacaagcagcagcagctcatcctaccctctagggggtcttgaggtcagccaggcaagagagcagcttggactccactgggtgtgggaccagcctgtggaccatggtggtgtggagggtgccctcggcctgcctgtgtgaaggagaggccggcgtgttctgtggagcccaaaggggagctgggcaagcaggattcacttcactctgagggtcctggagctcccaccctcctcagccatctccccagagcctgtgtgccgaggactcggcccatgttgctgtgggatgagaggcagagtgtcgtgagggtgtaaggagcggcggcagtggtgggaggagggagcagcagccagcgctacggtgccagtttccagctgccagatgacgccgctgaccctgtggttgagaagagatgcacagagccagctcttgcaagccagtgtggctgccatagcacctgccgagaagcagaaggaagggtggccccaggaggacagaggatgcgggcacatctgatgcgggcctgagttttgggagcttttgctctagccagtttccagctccgggacccacccgcctcgtaggcaagacaccacccaagaaatcatttgcttaacaaacacactgggctccaactggacacctgtgccaccctagatgctgggaacccagccatgacacaggcacctgcccccagctgctgaccactgaggctggctagcagctcccatggggccagtgtggggttccccagcctcctaacagggagccagtcacaagccctcgagagggaagggtgcccgcggccctggcaggaaggttaggctggacgctcccacaagacataacagatggaggttctaaatgatgtagcaacttcttcaccctgaaactgctgtagagtcagccatgacgcaccggtacttcagtaactgccaggcatccgggacagcacaccgcgagtcgctgctgtgcttgggttagaagtggtttggtctgttttcttctcgccctctctaatcagagtcagtgattcatgcccttccatcaccttagagaaggggcaggcgctgcccgaccttctccaggctggagcagcatcgcctcatgtcagcagaactcagctgtagaatatcgtggggttggtgcctttcatcagcagcatgtccttaacaactttctgatttcttccttagttgttggtccattaaggagaaaaaaaatgatctcagccattgctaaaatatttgataagattcagcaaagcagcatgttaacattgaaaactagaatcaggagccaggcagatgtgcttgcttttcacctgtagtatttcatgttgttttgacgtttttagctaatgcattaagataaataaacaaaagccgggcacggtggttcacgcctgtaatcccagcactttgggaggctgaggcgggaggatcctctgaggtcaggagttcaagaccagcctgaccaacatggagaaacctcgtcattactaaaaatacaaaattagctgggcgtggtggtgcatgcctgtaatcccagctacttgggaggctgaggcaggagaatcgcttgaacccgggaggcggaggttgcagtgagctgagattgcaccactgcactccagcctgggtgacagtgaaactcggtctcaaaaaaaaaaaaaaattaaaaaaagataaataaaataagcaggataagaaatgaagaaagtagagttacctttgttttcagatttcatttttgtatacccagaaagccaaatgtacaaaagactgggagctctttaaaccagcttaaacttgttgaaaatgaggatgaagaaatatcccattcagagttggaatgaatttaacccagaaggaacaggacctctactgaagagaactatgcagtcttactgaaaaatctaaataatacctgagcgctggagaaacttcgcacactcctgaaagctccaaagtcaatgtcatcattttattaatgtcattccaaacatagtctcaataatatcacttcttggttttgacatggacgcgatgatgtttaaattcatatgaaaaaagaacggggccaaaagtccaaggccagtcagcgtgagaagaccgctcggcctccctcggagtcggggagttggaaccgcagactgagatcatgtggctgctggaggccaggacgaacgtcgggaaatggagactcctgcgttgctggtgggatgtggtgcagccgcttccaggagcaatttggtgtcccgtcctaaagctgaagaaacgcatttcctctggtcagtgccactcctagacaggccaccctgcggcagccgtcctcaaactggtctgaggacccctcaacgctcttaaaaatcattaaaagtgggccaggtgcggtggctcacacctgtaatcccagcactttgggaggccaagacaggcggatcacgaggtcaggacattgagatcatcctggctaacacggtgaaaccccgtctctactaaaaatacaaaaaattagccgggcgtggtggcgggcgcctgtagtcccagctacttgggaggctgagccaggagaatggcgtgaacccaggaggtggagcttgcagtgagctgagatcactccactgcactccagcctgggcagcagagcgagactctgtctcaaaaaaaaataataaataaataaataaaaataaaataaaataaaattcattaaaagtgccaaagaacttttgcttatgtgagttctaatgaccaatattaatacacattagaatatcttattagaaattaaacctgagacctttagaaaacatgtattcatttcaaaatagcaataaacccatgacatattaacataaataacaattgtatgaaaaatatattttccaaaacaaaaagttttcgggagaagtgtggcatagttttacatggtcgtaaatctctggcttaagagaagcccactggcctctcagcaggctctgggtccgtccactttgggggtgttttggttgtgaagtataggagtgaatggagaagctcattcttacccagatgtgtatttgaaaagaaaaggaacattttaataacctttgcaaataatcggtatattcttccgtgatcctattccaacactggacaggtggtggtttgttttttttttttggagacggagtcccgctctgtcactcaggctggagtgcagtggcgcgatttcagctcactgcaagctccgcctcc

SEQ ID NO: 2 - DNA, 13481 bp, Homo sapiens
  CDS (146)...(9580): Synthetic oligonucleotide
gctgccgggacgggtccaagatggacggccgctcaggttctgcttttacctgcggcccagagccccattcattgccccggtgctgagcggcgccgcgagtcggcccgaggcctccggggactgccgtgccgggcgggagaccgccatggcgaccctggaaaagctgatgaaggccttcgagtccctcaagtccttccagcagcagcagcagcagcagcagcagcagcagcagcagcagcagcagcagcagcagcagcagcaacagccgccaccgccgccgccgccgccgccgcctcctcagcttcctcagccgccgccgcaggcacagccgctgctgcctcagccgcagccgcccccgccgccgcccccgccgccacccggcccggctgtggctgaggagccgctgcaccgaccaaagaaagaactttcagctaccaagaaagaccgtgtgaatcattgtctgacaatatgtgaaaacatagtggcacagtctgtcagaaattctccagaatttcagaaacttctgggcatcgctatggaactttttctgctgtgcagtgatgacgcagagtcagatgtcaggatggtggctgacgaatgcctcaacaaagttatcaaagctttgatggattctaatcttccaaggttacagctcgagctctataaggaaattaaaaagaatggtgcccctcggagtttgcgtgctgccctgtggaggtttgctgagctggctcacctggttcggcctcagaaatgcaggccttacctggtgaaccttctgccgtgcctgactcgaacaagcaagagacccgaagaatcagtccaggagaccttggctgcagctgttcccaaaattatggcttcttttggcaattttgcaaatgacaatgaaattaaggttttgttaaaggccttcatagcgaacctgaagtcaagctcccccaccattcggcggacagcggctggatcagcagtgagcatctgccagcactcaagaaggacacaatatttctatagttggctactaaatgtgctcttaggcttactcgttcctgtcgaggatgaacactccactctgctgattcttggcgtgctgctcaccctgaggtatttggtgcccttgctgcagcagcaggtcaaggacacaagcctgaaaggcagcttcggagtgacaaggaaagaaatggaagtctctccttctgcagagcagcttgtccaggtttatgaactgacgttacatcatacacagcaccaagaccacaatgttgtgaccggagccctggagctgttgcagcagctcttcagaacgcctccacccgagcttctgcaaaccctgaccgcagtcgggggcattgggcagctcaccgctgctaaggaggagtctggtggccgaagccgtagtgggagtattgtggaacttatagctggagggggttcctcatgcagccctgtcctttcaagaaaacaaaaaggcaaagtgctcttaggagaagaagaagccttggaggatgactctgaatcgagatcggatgtcagcagctctgccttaacagcctcagtgaaggatgagatcagtggagagctggctgcttcttcaggggtttccactccagggtcagcaggtcatgacatcatcacagaacagccacggtcacagcacacactgcaggcggactcagtggatctggccagctgtgacttgacaagctctgccactgatggggatgaggaggatatcttgagccacagctccagccaggtcagcgccgtcccatctgaccctgccatggacctgaatgatgggacccaggcctcgtcgcccatcagcgacagctcccagaccaccaccgaagggcctgattcagctgttaccccttcagacagttctgaaattgtgttagacggtaccgacaaccagtatttgggcctgcagattggacagccccaggatgaagatgaggaagccacaggtattcttcctgatgaagcctcggaggccttcaggaactcttccatggcccttcaacaggcacatttattgaaaaacatgagtcactgcaggcagccttctgacagcagtgttgataaatttgtgttgagagatgaagctactgaaccgggtgatcaagaaaacaagccttgccgcatcaaaggtgacattggacagtccactgatgatgactctgcacctcttgtccattgtgtccgccttttatctgcttcgtttttgctaacagggggaaaaaatgtgctggttccggacagggatgtgagggtcagcgtgaaggccctggccctcagctgtgtgggagcagctgtggccctccacccggaatctttcttcagcaaactctataaagttcctcttgacaccacggaataccctgaggaacagtatgtctcagacatcttgaactacatcgatcatggagacccacaggttcgaggagccactgccattctctgtgggaccctcatctgctccatcctcagcaggtcccgcttccacgtgggagattggatgggcaccattagaaccctcacaggaaatacattttctttggcggattgcattcctttgctgcggaaaacactgaaggatgagtcttctgttacttgcaagttagcttgtacagctgtgaggaactgtgtcatgagtctctgcagcagcagctacagtgagttaggactgcagctgatcatcgatgtgctgactctgaggaacagttcctattggctggtgaggacagagcttctggaaacccttgcagagattgacttcaggctggtgagctttttggaggcaaaagcagaaaacttacacagaggggctcatcattatacagggcttttaaaactgcaagaacgagtgctcaataatgttgtcatccatttgcttggagatgaagaccccagggtgcgacatgttgccgcagcatcactaattaggcttgtcccaaagctgttttataaatgtgaccaaggacaagctgatccagtagtggccgtggcaagagatcaaagcagtgtttacctgaaacttctcatgcatgagacgcagcctccatctcatttctccgtcagcacaataaccagaatatatagaggctataacctactaccaagcataacagacgtcactatggaaaataacctttcaagagttattgcagcagtttctcatgaactaatcacatcaaccaccagagcactcacatttggatgctgtgaagctttgtgtcttctttccactgccttcccagtttgcatttggagtttaggttggcactgtggagtgcctccactgagtgcctcagatgagtctaggaagagctgtaccgttgggatggccacaatgattctgaccctgctctcgtcagcttggttcccattggatctctcagcccatcaagatgctttgattttggccggaaacttgcttgcagccagtgctcccaaatctctgagaagttcatgggcctctgaagaagaagccaacccagcagccaccaagcaagaggaggtctggccagccctgggggaccgggccctggtgcccatggtggagcagctcttctctcacctgctgaaggtgattaacatttgtgcccacgtcctggatgacgtggctcctggacccgcaataaaggcagccttgccttctctaacaaaccccccttctctaagtcccatccgacgaaaggggaaggagaaagaaccaggagaacaagcatctgtaccgttgagtcccaagaaaggcagtgaggccagtgcagcttctagacaatctgatacctcaggtcctgttacaacaagtaaatcctcatcactggggagtttctatcatcttccttcatacctcaaactgcatgatgtcctgaaagctacacacgctaactacaaggtcacgctggatcttcagaacagcacggaaaagtttggagggtttctccgctcagccttggatgttctttctcagatactagagctggccacactgcaggacattgggaagtgtgttgaagagatcctaggatacctgaaatcctgctttagtcgagaaccaatgatggcaactgtttgtgttcaacaattgttgaagactctctttggcacaaacttggcctcccagtttgatggcttatcttccaaccccagcaagtcacaaggccgagcacagcgccttggctcctccagtgtgaggccaggcttgtaccactactgcttcatggccccgtacacccacttcacccaggccctcgctgacgccagcctgaggaacatggtgcaggcggagcaggagaacgacacctcgggatggtttgatgtcctccagaaagtgtctacccagttgaagacaaacctcacgagtgtcacaaagaaccgtgcagataagaatgctattcataatcacattcgtttgtttgaacctcttgttataaaagctttaaaacagtacacgactacaacatgtgtgcagttacagaagcaggttttagatttgctggcgcagctggttcagttacgggttaattactgtcttctggattcagatcaggtgtttattggctttgtattgaaacagtttgaatacattgaagtgggccagttcagggaatcagaggcaatcattccaaacatctttttcttcttggtattactatcttatgaacgctatcattcaaaacagatcattggaattcctaaaatcattcagctctgtgatggcatcatggccagtggaaggaaggctgtgacacatgccataccggctctgcagcccatagtccacgacctctttgtattaagaggaacaaataaagctgatgcaggaaaagagcttgaaacccaaaaagaggtggtggtgtcaatgttactgagactcatccagtaccatcaggtgttggagatgttcattcttgtcctgcagcagtgccacaaggagaatgaagacaagtggaagcgactgtctcgacagatagctgacatcatcctcccaatgttagccaaacagcagatgcacattgactctcatgaagcccttggagtgttaaatacattatttgagattttggccccttcctccctccgtccggtagacatgcttttacggagtatgttcgtcactccaaacacaatggcgtccgtgagcactgttcaactgtggatatcgggaattctggccattttgagggttctgatttcccagtcaactgaagatattgttctttctcgtattcaggagctctccttctctccgtatttaatctcctgtacagtaattaataggttaagagatggggacagtacttcaacgctagaagaacacagtgaagggaaacaaataaagaatttgccagaagaaacattttcaaggtttctattacaactggttggtattcttttagaagacattgttacaaaacagctgaaggtggaaatgagtgagcagcaacatactttctattgccaggaactaggcacactgctaatgtgtctgatccacatcttcaagtctggaatgttccggagaatcacagcagctgccactaggctgttccgcagtgatggctgtggcggcagtttctacaccctggacagcttgaacttgcgggctcgttccatgatcaccacccacccggccctggtgctgctctggtgtcagatactgctgcttgtcaaccacaccgactaccgctggtgggcagaagtgcagcagaccccgaaaagacacagtctgtccagcacaaagttacttagtccccagatgtctggagaagaggaggattctgacttggcagccaaacttggaatgtgcaatagagaaatagtacgaagaggggctctcattctcttctgtgattatgtctgtcagaacctccatgactccgagcacttaacgtggctcattgtaaatcacattcaagatctgatcagcctttcccacgagcctccagtacaggacttcatcagtgccgttcatcggaactctgctgccagcggcctgttcatccaggcaattcagtctcgttgtgaaaacctttcaactccaaccatgctgaagaaaactcttcagtgcttggaggggatccatctcagccagtcgggagctgtgctcacgctgtatgtggacaggcttctgtgcacccctttccgtgtgctggctcgcatggtcgacatccttgcttgtcgccgggtagaaatgcttctggctgcaaatttacagagcagcatggcccagttgccaatggaagaactcaacagaatccaggaataccttcagagcagcgggctcgctcagagacaccaaaggctctattccctgctggacaggtttcgtctctccaccatgcaagactcacttagtccctctcctccagtctcttcccacccgctggacggggatgggcacgtgtcactggaaacagtgagtccggacaaagactggtacgttcatcttgtcaaatcccagtgttggaccaggtcagattctgcactgctggaaggtgcagagctggtgaatcggattcctgctgaagatatgaatgccttcatgatgaactcggagttcaacctaagcctgctagctccatgcttaagcctagggatgagtgaaatttctggtggccagaagagtgccctttttgaagcagcccgtgaggtgactctggcccgtgtgagcggcaccgtgcagcagctccctgctgtccatcatgtcttccagcccgagctgcctgcagagccggcggcctactggagcaagttgaatgatctgtttggggatgctgcactgtatcagtccctgcccactctggcccgggccctggcacagtacctggtggtggtctccaaactgcccagtcatttgcaccttcctcctgagaaagagaaggacattgtgaaattcgtggtggcaacccttgaggccctgtcctggcatttgatccatgagcagatcccgctgagtctggatctccaggcagggctggactgctgctgcctggccctgcagctgcctggcctctggagcgtggtctcctccacagagtttgtgacccacgcctgctccctcatctactgtgtgcacttcatcctggaggccgttgcagtgcagcctggagagcagcttcttagtccagaaagaaggacaaataccccaaaagccatcagcgaggaggaggaggaagtagatccaaacacacagaatcctaagtatatcactgcagcctgtgagatggtggcagaaatggtggagtctctgcagtcggtgttggccttgggtcataaaaggaatagcggcgtgccggcgtttctcacgccattgctaaggaacatcatcatcagcctggcccgcctgccccttgtcaacagctacacacgtgtgcccccactggtgtggaagcttggatggtcacccaaaccgggaggggattttggcacagcattccctgagatccccgtggagttcctccaggaaaaggaagtctttaaggagttcatctaccgcatcaacacactaggctggaccagtcgtactcagtttgaagaaacttgggccaccctccttggtgtcctggtgacgcagcccctcgtgatggagcaggaggagagcccaccagaagaagacacagagaggacccagatcaacgtcctggccgtgcaggccatcacctcactggtgctcagtgcaatgactgtgcctgtggccggcaacccagctgtaagctgcttggagcagcagccccggaacaagcctctgaaagctctcgacaccaggtttgggaggaagctgagcattatcagagggattgtggagcaagagattcaagcaatggtttcaaagagagagaatattgccacccatcatttatatcaggcatgggatcctgtcccttctctgtctccggctactacaggtgccctcatcagccacgagaagctgctgctacagatcaaccccgagcgggagctggggagcatgagctacaaactcggccaggtgtccatacactccgtgtggctggggaacagcatcacacccctgagggaggaggaatgggacgaggaagaggaggaggaggccgacgcccctgcaccttcgtcaccacccacgtctccagtcaactccaggaaacaccgggctggagttgacatccactcctgttcgcagtttttgcttgagttgtacagccgctggatcctgccgtccagctcagccaggaggaccccggccatcctgatcagtgaggtggtcagatcccttctagtggtctcagacttgttcaccgagcgcaaccagtttgagctgatgtatgtgacgctgacagaactgcgaagggtgcacccttcagaagacgagatcctcgctcagtacctggtgcctgccacctgcaaggcagctgccgtccttgggatggacaaggccgtggcggagcctgtcagccgcctgctggagagcacgctcaggagcagccacctgcccagcagggttggagccctgcacggcgtcctctatgtgctggagtgcgacctgctggacgacactgccaagcagctcatcccggtcatcagcgactatctcctctccaacctgaaagggatcgcccactgcgtgaacattcacagccagcagcacgtactggtcatgtgtgccactgcgttttacctcattgagaactatcctctggacgtagggccggaattttcagcatcaataatacagatgtgtggggtgatgctgtctggaagtgaggagtccaccccctccatcatttaccactgtgccctcagaggcctggagcgcctcctgctctctgagcagctctcccgcctggatgcagaatcgctggtcaagctgagtgtggacagagtgaacgtgcacagcccgcaccgggccatggcggctctgggcctgatgctcacctgcatgtacacaggaaaggagaaagtcagtccgggtagaacttcagaccctaatcctgcagcccccgacagcgagtcagtgattgttgctatggagcgggtatctgttctttttgataggatcaggaaaggctttccttgtgaagccagagtggtggccaggatcctgccccagtttctagacgacttcttcccaccccaggacatcatgaacaaagtcatcggagagtttctgtccaaccagcagccatacccccagttcatggccaccgtggtgtataaggtgtttcagactctgcacagcaccgggcagtcgtccatggtccgggactgggtcatgctgtccctctccaacttcacgcagagggccccggtcgccatggccacgtggagcctctcctgcttctttgtcagcgcgtccaccagcccgtgggtcgcggcgatcctcccacatgtcatcagcaggatgggcaagctggagcaggtggacgtgaaccttttctgcctggtcgccacagacttctacagacaccagatagaggaggagctcgaccgcagggccttccagtctgtgcttgaggtggttgcagccccaggaagcccatatcaccggctgctgacttgtttacgaaatgtccacaaggtcaccacctgctgagcgccatggtgggagagactgtgaggcggcagctggggccggagcctttggaagtctgcgcccttgtgccctgcctccaccgagccagcttggtccctatgggcttccgcacatgccgcgggcggccaggcaacgtgcgtgtctctgccatgtggcagaagtgctctttgtggcagtggccaggcagggagtgtctgcagtcctggtggggctgagcctgaggccttccagaaagcaggagcagctgtgctgcaccccatgtgggtgaccaggtcctttctcctgatagtcacctgctggttgttgccaggttgcagctgctcttgcatctgggccagaagtcctccctcctgcaggctggctgttggcccctctgctgtcctgcagtagaaggtgccgtgagcaggctttgggaacactggcctgggtctccctggtggggtgtgcatgccacgccccgtgtctggatgcacagatgccatggcctgtgctgggccagtggctgggggtgctagacacccggcaccattctcccttctctcttttcttctcaggatttaaaatttaattatatcagtaaagagattaattttaacgtaactctttctatgcccgtgtaaagtatgtgaatcgcaaggcctgtgctgcatgcgacagcgtccggggtggtggacagggcccccggccacgctccctctcctgtagccactggcatagccctcctgagcacccgctgacatttccgttgtacatgttcctgtttatgcattcacaaggtgactgggatgtagagaggcgttagtgggcaggtggccacagcaggactgaggacaggcccccattatcctaggggtgcgctcacctgcagcccctcctcctcgggcacagacgactgtcgttctccacccaccagtcagggacagcagcctccctgtcactcagctgagaaggccagccctccctggctgtgagcagcctccactgtgtccagagacatgggcctcccactcctgttccttgctagccctggggtggcgtctgcctaggagctggctggcaggtgttgggacctgctgctccatggatgcatgccctaagagtgtcactgagctgtgttttgtctgagcctctctcggtcaacagcaaagcttggtgtcttggcactgttagtgacagagcccagcatcccttctgcccccgttccagctgacatcttgcacggtgaccccttttagtcaggagagtgcagatctgtgctcatcggagactgccccacggccctgtcagagccgccactcctatccccaggccaggtccctggaccagcctcctgtttgcaggcccagaggagccaagtcattaaaatggaagtggattctggatggccgggctgctgctgatgtaggagctggatttgggagctctgcttgccgactggctgtgagacgaggcaggggctctgcttcctcagccctagaggcgagccaggcaaggttggcgactgtcatgtggcttggtttggtcatgcccgtcgatgttttgggtattgaatgtggtaagtggaggaaatgttggaactctgtgcaggtgctgccttgagacccccaagcttccacctgtccctctcctatgtggcagctggggagcagctgagatgtggacttgtatgctgcccacatacgtgagggggagctgaaagggagcccctcctctgagcagcctctgccaggcctgtatgaggcttttcccaccagctcccaacagaggcctcccccagccaggaccacctcgtcctcgtggcggggcagcaggagcggtagaaaggggtccgatgtttgaggaggcccttaagggaagctactgaattataacacgtaagaaaatcaccattccgtattggttgggggctcctgtttctcatcctagctttttcctggaaagcccgctagaaggtttgggaacgaggggaaagttctcagaactgttggctgctccccacccgcctcccgcctcccccgcaggttatgtcagcagctctgagacagcagtatcacaggccagatgttgttcctggctagatgtttacatttgtaagaaataacactgtgaatgtaaaacagagccattcccttggaatgcatatcgctgggctcaacatagagtttgtcttcctcttgtttacgacgtgatctaaaccagtccttagcaaggggctcagaacaccccgctctggcagtaggtgtcccccacccccaaagacctgcctgtgtgctccggagatgaatatgagctcattagtaaaaatgacttcacccacgcatatacataaagtatccatgcatgtgcatatagacacatctataattttacacacacacctctcaagacggagatgcatggcctctaagagtgcccgtgtcggttcttcctggaagttgactttccttagacccgccaggtcaagttagccgcgtgacggacatccaggcgtgggacgtggtcagggcagggctcattcattgcccactaggatcccactggcgaagatggtctccatatcagctctctgcagaagggaggaagactttatcatgttcctaaaaatctgtggcaagcacccatcgtattatccaaattttgttgcaaatgtgattaatttggttgtcaagttttgggggtgggctgtggggagattgcttttgttttcctgctggtaatatcgggaaagattttaatgaaaccagggtagaattgtttggcaatgcactgaagcgtgtttctttcccaaaatgtgcctcccttccgctgcgggcccagctgagtctatgtaggtgatgtttccagctgccaagtgctctttgttactgtccaccctcatttctgccagcgcatgtgtcctttcaaggggaaaatgtgaagctgaaccccctccagacacccagaatgtagcatctgagaaggccctgtgccctaaaggacacccctcgcccccatcttcatggagggggtcatttcagagccctcggagccaatgaacagctcctcctcttggagctgagatgagccccacgtggagctcgggacggatagtagacagcaataactcggtgtgtggccgcctggcaggtggaacttcctcccgttgcggggtggagtgaggttagttctgtgtgtctggtgggtggagtcaggcttctcttgctacctgtgagcatccttcccagcagacatcctcatcgggctttgtccctcccccgcttcctccctctgcggggaggacccgggaccacagctgctggccagggtagacttggagctgtcctccagaggggtcacgtgtaggagtgagaagaaggaagatcttgagagctgctgagggaccttggagagctcaggatggctcagacgaggacactcgcttgccgggcctgggcctcctgggaaggagggagctgctcagaatgccgcatgacaactgaaggcaacctggaaggttcaggggccgctcttcccccatgtgcctgtcacgctctggtgcagtcaaaggaacgccttcccctcagttgtttctaagagcagagtctcccgctgcaatctgggtggtaactgccagccttggaggatcgtggccaacgtggacctgcctacggagggtgggctctgacccaagtggggcctccttgtccaggtctcactgctttgcaccgtggtcagagggactgtcagctgagcttgagctcccctggagccagcagggctgtgatgggcgagtcccggagccccacccagacctgaatgcttctgagagcaaagggaaggactgacgagagatgtatatttaattttttaactgctgcaaacattgtacatccaaattaaaggaaaaaaatggaaaccatca

SEQ ID NO: 3 - DNA, 20 bp, Artificial Sequence
  Primer
gggaccctgatcaacaccat

SEQ ID NO: 4 - DNA, 24 bp, Artificial Sequence
  Primer
ccagttcttgattttgtcgaaaca

SEQ ID NO: 5 - DNA, 18 bp, Artificial Sequence
  Probe
tgggtggtctccgcggcc

SEQ ID NO: 6 - DNA, 16 bp, Artificial Sequence
  Synthetic oligonucleotide
  misc_feature (1)...(16): n = A,T,C or G
nnnnnnnnnnnnnnnn

SEQ ID NO: 7 - DNA, 14 bp, Artificial Sequence
  Synthetic oligonucleotide
  misc_feature (1)...(14): n = A,T,C or G
nnnnnnnnnnnnnn

SEQ ID NO: 8 - DNA, 20 bp, Artificial Sequence
  Synthetic oligonucleotide
  misc_feature (1)...(20): n = A,T,C or G
nnnnnnnnnnnnnnnnnnnn

SEQ ID NO: 9 - DNA, 20 bp, Artificial Sequence
  Synthetic oligonucleotide
ccttccctgaaggttcctcc

SEQ ID NO: 10 - DNA, 15 bp, Artificial Sequence
  Synthetic oligonucleotide
taaattgtcatcacc

SEQ ID NO: 11 - DNA, 15 bp, Artificial Sequence
  Synthetic oligonucleotide
taaattgucatcacc

SEQ ID NO: 12 - DNA, 15 bp, Artificial Sequence
  Synthetic oligonucleotide
  misc_feature 8: n = A,T,C or G
taaattgncatcacc

SEQ ID NO: 13 - DNA, 15 bp, Artificial Sequence
  Synthetic oligonucleotide
taaautgtcatcacc

SEQ ID NO: 14 - DNA, 16 bp, Artificial Sequence
  Synthetic oligonucleotide
taaattgtcatcacca

SEQ ID NO: 15 - DNA, 18 bp, Artificial Sequence
  Synthetic oligonucleotide
taaattgtcatcacctta

SEQ ID NO: 16 - DNA, 20 bp, Artificial Sequence
  Synthetic oligonucleotide
taaattgtcatcaccattta

SEQ ID NO: 17 - DNA, 17 bp, Artificial Sequence
  Synthetic oligonucleotide
taaattgtcatcaccta

SEQ ID NO: 18 - DNA, 19 bp, Artificial Sequence
  Synthetic oligonucleotide
taaattgtcatcaccttta

SEQ ID NO: 19 - DNA, 16 bp, Artificial Sequence
  Synthetic oligonucleotide
gtaaattgtcatcacc

SEQ ID NO: 20 - DNA, 17 bp, Artificial Sequence
  Synthetic oligonucleotide
ggtaaattgtcatcacc

SEQ ID NO: 21 - DNA, 18 bp, Artificial Sequence
  Synthetic oligonucleotide
ggttaaattgtcatcacc

SEQ ID NO: 22 - DNA, 19 bp, Artificial Sequence
  Synthetic oligonucleotide
ggtgtaaattgtcatcacc

SEQ ID NO: 23 - DNA, 20 bp, Artificial Sequence
  Synthetic oligonucleotide
ggtgataaattgtcatcacc

SEQ ID NO: 24 - DNA, 21 bp, Artificial Sequence
  Synthetic oligonucleotide
ggctaaattgtcatcaccgcc

SEQ ID NO: 25 - DNA, 19 bp, Artificial Sequence
  Synthetic oligonucleotide
gctaaattgtcatcaccgc

SEQ ID NO: 26 - DNA, 21 bp, Artificial Sequence
  Synthetic oligonucleotide
taataaattgtcatcacctta

SEQ ID NO: 27 - DNA, 19 bp, Artificial Sequence
  Synthetic oligonucleotide
aataaattgtcatcacctt

SEQ ID NO: 28 - DNA, 21 bp, Artificial Sequence
  Synthetic oligonucleotide
tcttaaattgtcatcaccaga

SEQ ID NO: 29 - DNA, 19 bp, Artificial Sequence
  Synthetic oligonucleotide
cttaaattgtcatcaccag

SEQ ID NO: 30 - DNA, 18 bp, Artificial Sequence
  Synthetic oligonucleotide
taataaattgtcatcacc

SEQ ID NO: 31 - DNA, 17 bp, Artificial Sequence
  Synthetic oligonucleotide
aataaattgtcatcacc

SEQ ID NO: 32 - DNA, 17 bp, Artificial Sequence
  Synthetic oligonucleotide
ataaattgtcatcacca

SEQ ID NO: 33 - DNA, 17 bp, Artificial Sequence
  Synthetic oligonucleotide
ataaattctcatcacca

SEQ ID NO: 34 - DNA, 17 bp, Artificial Sequence
  Synthetic oligonucleotide
ataaatagtcatcacca

SEQ ID NO: 35 - DNA, 17 bp, Artificial Sequence
  Synthetic oligonucleotide
ataaattgtgatcacca

SEQ ID NO: 36 - DNA, 17 bp, Artificial Sequence
  Synthetic oligonucleotide
ataaattgtcttcacca

SEQ ID NO: 37 - DNA, 17 bp, Artificial Sequence
  Synthetic oligonucleotide
ataaattgtcaacacca

SEQ ID NO: 38 - DNA, 15 bp, Artificial Sequence
  Synthetic oligonucleotide
taaattctcatcacc

SEQ ID NO: 39 - DNA, 15 bp, Artificial Sequence
  Synthetic oligonucleotide
taaaatgtcatcacc

SEQ ID NO: 40 - DNA, 15 bp, Artificial Sequence
  Synthetic oligonucleotide
taaattgtgatcacc

SEQ ID NO: 41 - DNA, 15 bp, Artificial Sequence
  Synthetic oligonucleotide
taaattgtcttcacc

SEQ ID NO: 42 - DNA, 15 bp, Artificial Sequence
  Synthetic oligonucleotide
taaattgtcaacacc

SEQ ID NO: 43 - DNA, 17 bp, Artificial Sequence
  Synthetic oligonucleotide
ttaaattgtcatcacca

SEQ ID NO: 44 - DNA, 17 bp, Artificial Sequence
  Synthetic oligonucleotide
aaaaattgtcatcacca

SEQ ID NO: 45 - DNA, 17 bp, Artificial Sequence
  Synthetic oligonucleotide
attaattgtcatcacca

SEQ ID NO: 46 - DNA, 17 bp, Artificial Sequence
  Synthetic oligonucleotide
atatattgtcatcacca

SEQ ID NO: 47 - DNA, 17 bp, Artificial Sequence
  Synthetic oligonucleotide
ataatttgtcatcacca

SEQ ID NO: 48 - DNA, 17 bp, Artificial Sequence
  Synthetic oligonucleotide
ataaattgtcatgacca

SEQ ID NO: 49 - DNA, 17 bp, Artificial Sequence
  Synthetic oligonucleotide
ataaattgtcatctcca

SEQ ID NO: 50 - DNA, 17 bp, Artificial Sequence
  Synthetic oligonucleotide
ataaattgtcatcagca

SEQ ID NO: 51 - DNA, 17 bp, Artificial Sequence
  Synthetic oligonucleotide
ataaattgtcatcacga

SEQ ID NO: 52 - DNA, 17 bp, Artificial Sequence
  Synthetic oligonucleotide
ataaattgtcatcacct

SEQ ID NO: 53 - DNA, 15 bp, Artificial Sequence
  Synthetic oligonucleotide
taagttgtcatcacc

SEQ ID NO: 54 - DNA, 15 bp, Artificial Sequence
  Synthetic oligonucleotide
taaagtgtcatcacc

SEQ ID NO: 55 - DNA, 15 bp, Artificial Sequence
  Synthetic oligonucleotide
taaatggtcatcacc

SEQ ID NO: 56 - DNA, 20 bp, Artificial Sequence
  Synthetic oligonucleotide
tctctattgcacattccaag

SEQ ID NO: 57 - DNA, 20 bp, Artificial Sequence
  Synthetic oligonucleotide
ccttccctgaaggttcctcc

SEQ ID NO: 58 - DNA, 17 bp, Artificial Sequence
  Synthetic oligonucleotide
aattgtcatcaccagaa

SEQ ID NO: 59 - DNA, 17 bp, Artificial Sequence
  Synthetic oligonucleotide
aattgtcatcaccagaa

SEQ ID NO: 60 - DNA, 17 bp, Artificial Sequence
  Synthetic oligonucleotide
aaattgtcatcaccaga

SEQ ID NO: 61 - DNA, 17 bp, Artificial Sequence
  Synthetic oligonucleotide
taaattgtcatcaccag

SEQ ID NO: 62 - DNA, 17 bp, Artificial Sequence
  Synthetic oligonucleotide
aataaattgtcatcacc

SEQ ID NO: 63 - DNA, 17 bp, Artificial Sequence
  Synthetic oligonucleotide
taataaattgtcatcac

SEQ ID NO: 64 - DNA, 17 bp, Artificial Sequence
  Synthetic oligonucleotide
ttaataaattgtcatca

SEQ ID NO: 65 - DNA, 15 bp, Artificial Sequence
  Synthetic oligonucleotide
attgtcatcaccaga

SEQ ID NO: 66 - DNA, 15 bp, Artificial Sequence
  Synthetic oligonucleotide
ttaataaattgtcat

SEQ ID NO: 67 - DNA, 15 bp, Artificial Sequence
  Synthetic oligonucleotide
ttgtcatcaccagaa

SEQ ID NO: 68 - DNA, 15 bp, Artificial Sequence
  Synthetic oligonucleotide
aattgtcatcaccag

SEQ ID NO: 69 - DNA, 15 bp, Artificial Sequence
  Synthetic oligonucleotide
aaattgtcatcacca

SEQ ID NO: 70 - DNA, 15 bp, Artificial Sequence
  Synthetic oligonucleotide
aataaattgtcatca

SEQ ID NO: 71 - DNA, 15 bp, Artificial Sequence
  Synthetic oligonucleotide
attaataaattgtca

SEQ ID NO: 72 - DNA, 15 bp, Artificial Sequence
  Synthetic oligonucleotide
tattaataaattgtc

SEQ ID NO: 73 - DNA, 15 bp, Artificial Sequence
  Synthetic oligonucleotide
gtcatcaccagaaaa

SEQ ID NO: 74 - DNA, 15 bp, Artificial Sequence
  Synthetic oligonucleotide
tgtcatcaccagaaa

SEQ ID NO: 75 - DNA, 15 bp, Artificial Sequence
  Synthetic oligonucleotide
ataaattgtcatcac

SEQ ID NO: 76 - DNA, 15 bp, Artificial Sequence
  Synthetic oligonucleotide
taataaattgtcatc

SEQ ID NO: 77 - DNA, 17 bp, Artificial Sequence
  Synthetic oligonucleotide
ataaaatgtcatcacca

SEQ ID NO: 78 - DNA, 15 bp, Artificial Sequence
  Synthetic oligonucleotide
taaatagtcatcacc

SEQ ID NO: 79 - DNA, 20 bp, Artificial Sequence
  Synthetic oligonucleotide
ctcgactaaagcaggatttc

SEQ ID NO: 80 - DNA, 19 bp, Artificial Sequence
  Synthetic oligonucleotide
aataaattgtcatcaccag

SEQ ID NO: 81 - DNA, 19 bp, Artificial Sequence
  Synthetic oligonucleotide
cacagtgctacccaacctt

SEQ ID NO: 82 - DNA, 19 bp, Artificial Sequence
  Synthetic oligonucleotide
tcacagctatcttctcatc

SEQ ID NO: 83 - DNA, 20 bp, Artificial Sequence
  Synthetic oligonucleotide
tcccatttcaggagacctgg

SEQ ID NO: 84 - DNA, 20 bp, Artificial Sequence
  Synthetic oligonucleotide
gctgattagagagaggtccc

SEQ ID NO: 85 - DNA, 16 bp, Artificial Sequence
  Synthetic oligonucleotide
atcatggctgcagctt

SEQ ID NO: 86 - DNA, 16 bp, Artificial Sequence
  Synthetic oligonucleotide
ttcagtcatgacttcc

SEQ ID NO: 87 - DNA, 16 bp, Artificial Sequence
  Synthetic oligonucleotide
tggctgcagcttccga

SEQ ID NO: 88 - DNA, 16 bp, Artificial Sequence
  Synthetic oligonucleotide
atggctgcagcttccg

SEQ ID NO: 89 - DNA, 16 bp, Artificial Sequence
  Synthetic oligonucleotide
catggctgcagcttcc

SEQ ID NO: 90 - DNA, 16 bp, Artificial Sequence
  Synthetic oligonucleotide
tcatggctgcagcttc

SEQ ID NO: 91 - DNA, 16 bp, Artificial Sequence
  Synthetic oligonucleotide
catcatggctgcagct

SEQ ID NO: 92 - DNA, 16 bp, Artificial Sequence
  Synthetic oligonucleotide
ccatcatggctgcagc

SEQ ID NO: 93 - DNA, 16 bp, Artificial Sequence
  Synthetic oligonucleotide
tccatcatggctgcag

SEQ ID NO: 94 - DNA, 16 bp, Artificial Sequence
  Synthetic oligonucleotide
ttccatcatggctgca

SEQ ID NO: 95 - protein, 3144 aa, Homo sapiens
MATLEKLMKAFESLKSFQQQQQQQQQQQQQQQQQQQQQQQPPPPPPPPPPPQLPQPPPQAQPLLPQPQPPPPPPPPPPGPAVAEEPLHRPKKELSATKKDRVNHCLTICENIVAQSVRNSPEFQKLLGIAMELFLLCSDDAESDVRMVADECLNKVIKALMDSNLPRLQLELYKEIKKNGAPRSLRAALWRFAELAHLVRPQKCRPYLVNLLPCLTRTSKRPEESVQETLAAAVPKIMASFGNFANDNEIKVLLKAFIANLKSSSPTIRRTAAGSAVSICQHSRRTQYFYSWLLNVLLGLLVPVEDEHSTLLILGVLLTLRYLVPLLQQQVKDTSLKGSFGVTRKEMEVSPSAEQLVQVYELTLHHTQHQDHNVVTGALELLQQLFRTPPPELLQTLTAVGGIGQLTAAKEESGGRSRSGSIVELIAGGGSSCSPVLSRKQKGKVLLGEEEALEDDSESRSDVSSSALTASVKDEISGELAASSGVSTPGSAGHDIITEQPRSQHTLQADSVDLASCDLTSSATDGDEEDILSHSSSQVSAVPSDPAMDLNDGTQASSPISDSSQTTTEGPDSAVTPSDSSEIVLDGTDNQYLGLQIGQPQDEDEEATGILPDEASEAFRNSSMALQQAHLLKNMSHCRQPSDSSVDKFVLRDEATEPGDQENKPCRIKGDIGQSTDDDSAPLVHCVRLLSASFLLTGGKNVLVPDRDVRVSVKALALSCVGAAVALHPESFFSKLYKVPLDTTEYPEEQYVSDILNYIDHGDPQVRGATAILCGTLICSILSRSRFHVGDWMGTIRTLTGNTFSLADCIPLLRKTLKDESSVTCKLACTAVRNCVMSLCSSSYSELGLQLIIDVLTLRNSSYWLVRTELLETLAEIDFRLVSFLEAKAENLHRGAHHYTGLLKLQERVLNNVVIHLLGDEDPRVRHVAAASLIRLVPKLFYKCDQGQADPVVAVARDQSSVYLKLLMHETQPPSHFSVSTITRIYRGYNLLPSITDVTMENNLSRVIAAVSHELITSTTRALTFGCCEALCLLSTAFPVCIWSLGWHCGVPPLSASDESRKSCTVGMATMILTLLSSAWFPLDLSAHQDALILAGNLLAASAPKSLRSSWASEEEANPAATKQEEVWPALGDRALVPMVEQLFSHLLKVINICAHVLDDVAPGPAIKAALPSLTNPPSLSPIRRKGKEKEPGEQASVPLSPKKGSEASAASRQSDTSGPVTTSKSSSLGSFYHLPSYLKLHDVLKATHANYKVTLDLQNSTEKFGGFLRSALDVLSQILELATLQDIGKCVEEILGYLKSCFSREPMMATVCVQQLLKTLFGTNLASQFDGLSSNPSKSQGRAQRLGSSSVRPGLYHYCFMAPYTHFTQALADASLRNMVQAEQENDTSGWFDVLQKVSTQLKTNLTSVTKNRADKNAIHNHIRLFEPLVIKALKQYTTTTCVQLQKQVLDLLAQLVQLRVNYCLLDSDQVFIGFVLKQFEYIEVGQFRESEAIIPNIFFFLVLLSYERYHSKQIIGIPKIIQLCDGIMASGRKAVTHAIPALQPIVHDLFVLRGTNKADAGKELETQKEVVVSMLLRLIQYHQVLEMFILVLQQCHKENEDKWKRLSRQIADIILPMLAKQQMHIDSHEALGVLNTLFEILAPSSLRPVDMLLRSMFVTPNTMASVSTVQLWISGILAILRVLISQSTEDIVLSRIQELSFSPYLISCTVINRLRDGDSTSTLEEHSEGKQIKNLPEETFSRFLLQLVGILLEDIVTKQLKVEMSEQQHTFYCQELGTLLMCLIHIFKSGMFRRITAAATRLFRSDGCGGSFYTLDSLNLRARSMITTHPALVLLWCQILLLVNHTDYRWWAEVQQTPKRHSLSSTKLLSPQMSGEEEDSDLAAKLGMCNREIVRRGALILFCDYVCQNLHDSEHLTWLIVNHIQDLISLSHEPPVQDFISAVHRNSAASGLFIQAIQSRCENLSTPTMLKKTLQCLEGIHLSQSGAVLTLYVDRLLCTPFRVLARMVDILACRRVEMLLAANLQSSMAQLPMEELNRIQEYLQSSGLAQRHQRLYSLLDRFRLSTMQDSLSPSPPVSSHPLDGDGHVSLETVSPDKDWYVHLVKSQCWTRSDSALLEGAELVNRIPAEDMNAFMMNSEFNLSLLAPCLSLGMSEISGGQKSALFEAAREVTLARVSGTVQQLPAVHHVFQPELPAEPAAYWSKLNDLFGDAALYQSLPTLARALAQYLVVVSKLPSHLHLPPEKEKDIVKFVVATLEALSWHLIHEQIPLSLDLQAGLDCCCLALQLPGLWSVVSSTEFVTHACSLIYCVHFILEAVAVQPGEQLLSPERRTNTPKAISEEEEEVDPNTQNPKYITAACEMVAEMVESLQSVLALGHKRNSGVPAFLTPLLRNIIISLARLPLVNSYTRVPPLVWKLGWSPKPGGDFGTAFPEIPVEFLQEKEVFKEFIYRINTLGWTSRTQFEETWATLLGVLVTQPLVMEQEESPPEEDTERTQINVLAVQAITSLVLSAMTVPVAGNPAVSCLEQQPRNKPLKALDTRFGRKLSIIRGIVEQEIQAMVSKRENIATHHLYQAWDPVPSLSPATTGALISHEKLLLQINPERELGSMSYKLGQVSIHSVWLGNSITPLREEEWDEEEEEEADAPAPSSPPTSPVNSRKHRAGVDIHSCSQFLLELYSRWILPSSSARRTPAILISEVVRSLLVVSDLFTERNQFELMYVTLTELRRVHPSEDEILAQYLVPATCKAAAVLGMDKAVAEPVSRLLESTLRSSHLPSRVGALHGVLYVLECDLLDDTAKQLIPVISDYLLSNLKGIAHCVNIHSQQHVLVMCATAFYLIENYPLDVGPEFSASIIQMCGVMLSGSEESTPSIIYHCALRGLERLLLSEQLSRLDAESLVKLSVDRVNVHSPHRAMAALGLMLTCMYTGKEKVSPGRTSDPNPAAPDSESVIVAMERVSVLFDRIRKGFPCEARVVARILPQFLDDFFPPQDIMNKVIGEFLSNQQPYPQFMATVVYKVFQTLHSTGQSSMVRDWVMLSLSNFTQRAPVAMATWSLSCFFVSASTSPWVAAILPHVISRMGKLEQVDVNLFCLVATDFYRHQIEEELDRRAFQSVLEVVAAPGSPYHRLLTCLRNVHKVTTC